European Patent Application EP 4 726 035 A1, published April 15, 2026. Title: Cas酶及其系统和应用. Applicant: 益杰立科（上海）生物科技有限公司. Application CN. The sequence listing filed with the application follows.

SEQUENCE LISTING (127 sequences)

SEQ ID NO: 1 - protein, 1270 aa, synthetic construct
  REGION 1..1270: note = EpiCas001
  SITE 1270: note = misc_feature - Xaa =
MNNNGETKCYGNNLDRFIGLREVNKTLRNELIPTDSTRENIEKNGIISEDELRAEMGHELKAIMDDYYRNMIEETLSRKCNINWSTLFAAMDSVARSANKKDADKILEKVQKEKREEIHKLFKEQGNFEKLFKAELVSDVLPDFIGKYEGYSDEERISKLGTIKLFKKFMTSFKAYFDNRKNVFSKENISTSICHRVVNDNAFIFWDNLNAFKKIDKYAHDAVETIEGEISGKLGEWKISQIYSVDFFGMVIPQSGITFYNEVSGEINKYMNIYCQKEKQNSRQFKLKRLHKQILCIGETSFEIPEKYESDEEVYQSVNDFIGMIKNNDIISRLEHLAENVNKYDADKIYINSKSYENVSKCIGGTWNTIKDCLRLWYNENIRGSGKNKEKKVGKAVEEDKYKSIAMLNQLLENYSDGDGRIYNVQLYVEHITKIIGDYKPEELVYDANIRVIEQDEKAEEIKSVLDIYIAILHWIKAFIIEDAVEKDTDFYYEIEEIFDKVQSIIPLYNMVRNYTTQKPYKQEKIKLKFNTPTLAEGWHKSKEYSNNAIILQRDGKYYLGIFNAKNKPDKKIIEGCSQKKNKADYAKMVYYLLPKPHMNLPHIFIKSKEAVKNYGLSNYIVEGYDKDKHIKSSNGFDIKYCRDLIDYFKDCISKHPEWKNFNFSFTDTALYNDIGEFYNEIKRQGYKIEWTYISEEEINRLDENGQIYLFQIYNKDFAEGSKGTPNLHTLYLKNLFSEDNLKDPVFMLNGNTEVFFRKSSIKKPVVHKKGSVLVNRNYIDLNGNRITIPEKEYKEIYEYCNGIGNVNLSESAMKYYDMAKHYTATMDIVKDYRYTVDKFFIHMPMTINFNAESNNNINELALNFVAKNDNIHIIGVDRGERNLIYISVIDSKGNIIKQKSYNVVNDYDYKSKLKEREYDRGDARKNWKRINNIKELKEGYLSQVVHEIAQLVIQYNAIIAMEDLNYGFKRGRFKVERQVYQKFENMLINKLNYLVDKRKNADEAGGVLKGYQLTYIPERLKNMGRQCGIIFYVPAAYTSKIDPTTGFVNLFNFNAITSQEGRRKFINKFKHIRYNLNMNLFEFEFDYNDFITHNTQIAKTEWSVYTNGPRIKKERVNGKWNDGYEADITEVMKQKLSDNGIDYADGGDILTRIAEADDKLVSGIFEIFRLTVQLRNSKSESCGEDYDRIISPVLNESNRFYDSDEYSGENEILPVDADANGAYCIALKGLYEVKQIRENWVEGDKLSGDLLKISNADWFDFIQNKRYEX

SEQ ID NO: 2 - protein, 1265 aa, synthetic construct
  REGION 1..1265: note = EpiCas002
  SITE 1265: note = misc_feature - Xaa =
MNIKFNKFTGVKPVSKTLRNALIPTEFTMVNLERNGIISADELRAEKRQELKKIMDDYYRDLIERTLAENHSINWHILFELMKSKMHGDEKDTAKKLENEQKSKREEIHRLFAEQEEFGKIFSAKLVSDILPGFVASYAMYNDEDRTEKAEVVKLFNKFMSSFTEFFENRKNVFSKENISTSLCHRIVNDNALIFLNNMDSYKRIMENFKSESELVSKGLETMLGEWKISQIYSEDFFGMTMTQSGIEFYNDICGELNLVLNLYCQKSKKNSARFKMKRLHKQILCTEKSSFEISYKYDNDKDVYTSVNGFIKNIKNNNIIERLLKLGTETEQYDLNKIYISSQSYETVSIAIGGTWETIRNCLTSWYDDNIKGSGKAKENKIKAVVKADKYQSIARVDYLTETYNASGTDLQKAESYLSHIVQIIGDYEPEELYFDESIHLIENGDKISEIKKILDIYIDVVHWIKTFEISESVEKEPEFYYELDDIYDKILDAVPLYNKVRNYVTQKPYNQEKFKLNFDSPTLANGWSKSKERDNNAIILSRDGKYYLGVFNVRNKPDKEILEGHSKPKNETDYAKMVYNLLPGASKMLPKVFLSKKGIDNFKPSDYILEGYIKKKHIKSSETFDIKYCRDLIDYFKNSISRHPEWKNFGFNFTETSKYNDISEFYKEVEKQGYKIEWTYITEEDINKLDEAGQIYLFQIFNKDFAVGSKGTPNLHTLYLKNLFSKENLDNVVLKLNGEAELFFRRSSIKTPVIHKKGSILVNRCYVDADDGKRKPIPEKEYMEIYNYCNGKRDTELSESARKYYNISQRYEATMDIVKDYRYSVDKLFIHLPITINFKATENKNVNDMVLEYIAKSDDIHIIGIDRGERNLIYVSVIDMHGHIVMQKSYNVVNEYDYKTKLKECEQGRDAARKNWKEIGKIKELKEGYLSMVIHEITQLIIEYNAIVMMEDLNFGFKRGRFKVERQVYQKFENMLINKLNYLVDKHKAVDEPGGLLNGYQLTYIPDRMSELGRQCGIIFYVPAAYTSKIDPTTGFFNAFRFNLLTSAESRRDFLNRFKCIKYNGSMNMFEFDFDYNDFITHNTTIARTQWKVFTNGGRIKNIISKSGWNGTKKIDDITALMKEIFDSRKIDFSDGGNLLPEILAYEGADKDKFIVELLDIFKLTVQLRNSMPDGSDIEYDRIISPVINENNTFYDSDMYTEPNSPLPIDADANGAYCIALKGLYEVNQIKENWKEGETFPKSVLKLNNANWFDFVQNKRYEX

SEQ ID NO: 3 - protein, 826 aa, synthetic construct
  REGION 1..826: note = EpiCas003
  SITE 826: note = misc_feature - Xaa =
MNLAFLNRGYNYGMINRIERGPFSELGDQQLLEQTRRLAANQRCLEVHILDHLDEIDRRGLALRRGFSSLFDYAVRELRFSDAAAQRRIQAMRLCRRHGCVRASLQSGELGMTSAAQLETTFAGAERAERKSHTGHRNVGQGRGPDQDQDSVGSTRQLGLPAAPGEADEQGERGHRSAPEGAPPAAECSGDARERGHRSAPEGAAPAGEYTGEVAARTTPAVAVAVASRSGAQPPGGVHAGALLPRPELNGNAAPVQAPSRAPVAAPGAPGAGAGAGPAAPASDEGPAAQLLPPTEFSASTPEPEPVTAPAELRHTASRAPEPPRDDPFAELVPGTVSAAPLLHPQRQRELIEQAAGMSTRQVASLLAAAAPEVLPPRDTLRAVAPDRYTLKVSIDQECEQGLRLLKDLMAHLDPRMSWGDLVARVVREAVARHDPRGGGRGQRRKGADSAGASPRRTPKETRAAGAAGGPARRVGESTGREPNRTGAAGAAGGPAQREDESSGRAQNRTRAAVAPVAAARRRGGATSAPQSAPAVLVDGARAGGGPAGAPAAPPAPPGDTAATERQNPIEVLTSAAPPSQSAPAAPSDGAHAGGAPAGASAATSAPQSAPAAQLDGARAGRVPSGAPAATSAPQFASGALLDGSNAGAGVPGAPVATAAPQPALGGSPDGGPSGASAGASAGAAGGASADGFSARAAGPGASVATSAPKSVLGGFPDGGPPDAAAGAAAHTSREPVHSRRQSPRRRHIPAAVRRHIWHRDGGRCCYRDPLTGRRCTSAHLLQIDHLVPVAEGGGPEPSNLALRCFAHHRMRHGYAPAASPQPPIX

SEQ ID NO: 4 - protein, 807 aa, synthetic construct
  REGION 1..807: note = EpiCas004
  SITE 807: note = misc_feature - Xaa =
MDGLARVDRAVTACLAAPAWALPEEALVEALDEAHRLGQRLAVLERVLVREVDGRGLARAQGATSTAGWLRDRLRVSIQSARRLVADAGWLDAADDPGTTDDPGTTGDPSGTTDDPGTTGDPSGTRTYASVEPGTGIGAAGAPSPADALPDAAGRTGLDGAVTTGPGPGAGGAGGAGGADRAGAPGLSAAAGCGTAAAGPVLREALATGRVNLEQARIIAGAVESVRKEAGPDTADKALYTLLADARRFEPRALRALADRILWHVAPDAAEEADRAALRRADDEAQRRRHLTLSATDDGRMRLRGLLDSETSATLLAALDPLTRPAGLGDDRTSGQRRHDALGDICRLALRTGELPDNGGEPAQIVVTTEYAALTARLTAVGLPAARQPGATSGTRSSIARPSPEPAPAERGPTEPTPAEQGSIESTPAERRPTEHTPAERRRTERMPAERGAARRTQSGIGRLRRTTHERGGCGPRPPQRAAHNCGQPGRTGRAPAAGSGQRRPERPVPRIRNGTAGTTGTATGRWQRPRGAPTETPTETAVSGGPPTPQSSPPADPSTLGTQRGSPTTDQRPASTDRAPATPVHEATAPAQDALAVQDAAATVQRSPRLDHGCATADQQQDPGRDQDPGRDRAPGRDRHSRGPDRDQWQARDRDHGRQGRGRLGPGRLDNDLRLTPATVRRLACDAAILPAVLGSQGQVLDLGRQRRLFTGPLRRALVLRDRGCAFPGCDRPPRWCDGHHIQHWADGGATALHNAVLLCRHHHRVIHQDDWTVRIAADGHPEFVPPAWIDPEQRPRRNRYHRRAX

SEQ ID NO: 5 - protein, 1596 aa, synthetic construct
  REGION 1..1596: note = EpiCas005
  SITE 1596: note = misc_feature - Xaa =
MVVIECTVPDCEFKTTDASEAVAIALLANHNLVHRNEAQPRRLPANTAPKGPKLDRPKIDVGVTMEEWNIFTRRWEVFRAGSGIDENSAPSQLFQCAGTELGDSILKANPNAVNESLTQLMEAMRSLAIIPIATCVLRTELLQMRQERDESFRSFTAKVRGKAETCAYNAKCSCSRPVDYTDHVIRDVIINGLYDNEIRREVLGIDGILEKPINQVIAVVESKEMARNALPPSPSLSAVSSFQRQKTNSPHPAPSPPQADQAKEATCPGCQKTFKLFTEGARGWNKKPHQLCIDCHRVNRRARRPQRQPQQRSPQAPTVHANQAEPIAQISSLHGETKQDTRPTTHATTAKRPVRLDHHIFSKGEWKRARFRDHPRVPITISLARKGRHRKETADTTPDIHAAVSAIADTGAQSDLWSLADFLACGFSREELQPIRPSLTAANNSPISIEGAFFAKLSATSYSGQSTTSFSMVYVSSSVRDMYLSYDSLLNLDLLPHCFPRHDDVTEASNERRPASQNKTRPNYTSPTTNAARIVNEGCTKPASEHDVTCSCPQRETTPPRPSELPFPCTPANNTKMKAWLLNRYASSTFNTCPHRALPCMEGPPVEIHLDPTAKPTACHTPANIPLHWQKRVYEDLLRDEALGVVERVPYGEPVTWCHRMVVTRKHDGSPRRTVDLSPLNKYCQRETYATESPFQLARRIPNDTWKTVTDAWNGYHSVPLRSSDRHLTTFITPFGRWRYTRAPQGFLSSGDRYNRRFDAILAEFERKERCVDDTVHYDHDLEQHWWRTIEFLTRVGQAGIVLNPDKFQFAGRSVDFAGFHVSDHTIEPLPKYLDGIREFPTPTSTTDIRSWFGLVNQVSNYAQLRDLMAPFKPFLSPRHKFLWSSELEEAFQASKEKIVKAIREGVEIFDIHKRTCLRPDWSKRGIRYFLLQQHCSCSSGMPDCCPGGWGITLAGSRFLSPAEQRYAAIEGEALAVAWGLEQTRYFTQGCDNLVIITDHKPLVKIFGDRTLDEISNSRLFRLKQRTLPWRFEIHHLPGKSNYAADATSRHPSQSNTEEKAPLCPANPPDAAEIALMTAIRDTAQELGAISWTLLAQETAADARMGNLLHSLEQGTQLNKDDPTLANLGPIYESIYQEEGVLMYQDRVVIPPSLRQRVLQSLHAAHQGTSSMEQRARSIVYWPGMSNDIRVTREKCHDCNRNAPSQARTPPLPTAPPSTPFEAVFADFFNYKGYHYLVVGDRLSGWVEVLSSPATTNLAGSTGLIRHLRTFFATFGVPEELSSDGGPEFTAKATEDFLRTWDVKQRLSSVSFPQSNGRAEVAVKTAKRLLLSNTGPTGSLDQDRFLRAILQLRNTPDPDCSLSPAQIIFGRPLRDTLAFVNRLEKFSNPHIRPLWRQAWAAKEDALRTRISRTTESLREHARPLRPLAIGTRVFLQNQQGPNPNKWDRSGVVVEAAGHDQYRVKVDGSGRVTLRNRRFLRAYTPALPAIPQAPSGAPAKTPSMAPDAPSSPSQTCHHTNRTATPATTPGVPTPDLATAALALQVSPEEPDAAEEKQGPSTPEAMTLPSPPNAAARPRRTIRRPKQFEPETGTWTEX

SEQ ID NO: 6 - protein, 932 aa, synthetic construct
  REGION 1..932: note = EpiCas006
  SITE 932: note = misc_feature - Xaa =
MASIASLAPDGWLERKELSDGVSDDGLSDDESLLEERDTLETIRDSLTATNPDEIDGLLGRPSLGSDGLPSPRTPSRRREFLGERKGSKTRLSPTPPAAVPAPTCAPASTKNLWRGFALFAMAMACAALSLQRSPELVEYGPSRRLQTSFGERVDEAADGATSRRLQNSNQFCAARDGWEAFVGTARAGEAFGGEVCLLASTSTESSTLYGSHAAYSPPMRVRAEFLAADDLTRQLGLVFGVPAWPDAANLPATGYACVLEHKVTRWSSKSRLVLRRANADYDKNPDWINFKRSRWFDSEPNAWYEATAAIDDTSAAIAGKVGADVSCEVRDDGGAVVASVRKEDRWVMAHPGKVGFYSERDDLGERFVRALEVDGERAPEEPSFCCYWSPTSDMCGDCPDPQTDGWCAASRARCEGCGGTFCDAPTPPKEVPGRCCYDGAGCGSCSASDDDGFCAKSESNCGSCGGFFCSLAPTPAPTRVPSPRPTTPSPTAAPTVAPGHPTAAPATYAPSSSEPSSKPTTSTPSAQQGCACEEGPYEYDGKTFEGCTSYGWSVPWCGTTNCGICDGLVSTGCWDECEETYAPSSSEPSPKPTTSTPSAAPQGFPAIPLPTSATSPPTPTVFLTNADFRYGTYLITNPGVYVLREDIVFAPETPKMMPPLDSETYPPDRGFWLGFFAAISVAADDVVVDLNGHEIRSSREFLLRQRFFSIIELADKPFKANSGPPQFGALDAPLVPARRVHVKSGTLGLSSHMGIHGNDNEDVTVTDVVIRDFETGGVQLNGASRVRLERVTVGPSLGHEHSAGPVPALATLSQATNLLRVAEGTRHERQEEMVLLSAAVERFVQETLAGEDTSASVFASEAAGYAGLPDGSATVWIPTTGLGGPHQTSELSSSVKSTSIRLIFGRIDCSRRVLEKQPKSLCRNRRIRENX

SEQ ID NO: 7 - protein, 771 aa, synthetic construct
  REGION 1..771: note = EpiCas007
  SITE 771: note = misc_feature - Xaa =
MAGNHFKGSDSGRPAVPPRPNGAGKAGTPGGAGQGGSGKRVSPGETAMFTALYEQSQKAKKTGRARGNVFAGGATFASQPSGAPSVPANNAGAANAANGAGNVNAGKADNNTPSAGGAGLTGNLGTIYTGASETGTFARLDDSGAEFAGSGSKEDYYDFGLNYGSDASSSSTSDGLVRHRHRKGERKKRHTGAIIAAVVAVLLVALGASGFMLLNSAKTVKSEAKEAVEIVGGLKDKVTSGDFSTLPDDAKKIDELCDSMKAETSSPLWAAASFIPVYGSDINAARTMIDALSDVSSNALVPMADNLSQATPGKLFQDGMINVSALQAVADSLSSSSKVFKSANEKVQGIGDTHISQVTELVDKVKDGFATLNGAVDAAEKVAPVLPQMLGANGQTRNYLMYAMNNVEIRACGGFGGSQGLISVTDGQMSIGEFVPRIGLSEDEAVESVDEEDEALFGNHSNLYNSGNTYSPDWPRNSQRVAALWKSQYGQDVDGVIGIDPVFLQYLLGLVGNVSLPDGTVVDGTNAAKVLMHDVYWNYPVEESDGIFASVASAAFDKILGGIGDVDVTKLVSAVERGAEEGRLIAWMRNDDEQNAIKETGIDASLPDPDDPSADPVAGVYFNNLSFSKLDWYLNADTQIGQGIKNGDGTCSYRITVTLTNIMTQEEAGKLPDYVAASAPDAARDDERLNVSLFAPTGGNISDLTVEGTQFGLGAATWHGIPFYSGTVDLHAGETTTITYTLTTSAEAGDKPLTLRQTPTCQAARDSASAX

SEQ ID NO: 8 - protein, 744 aa, synthetic construct
  REGION 1..744: note = EpiCas008
  SITE 744: note = misc_feature - Xaa =
MEAGRDFIAFGQDVQGTDCCRGAGGAGLAGPAGRSGAGAKNVRPPCQTVGMEAGRDFIPFGQVVEGTDRDCCSGAGGAGLADAGAAGVSGVGGVLAGVRQLCAGVVEDSALWDLGAASDFAGGVEEISRAVEYLQLVAASAVDRARTQSAAAAAPGMSWTTGWRDEDPASDENSGTTAPVPVEPPSAAATGSDDGYRNTVEFLRARLRIGAAEARGRLALGAGVLPRQGLAGRSEAAVHAELGAAVAAGAVGSRAAAVIEAALGRVRHVGDAAAAARMEHALTRTAAENDTDFLARVARSWAEAMDQDGAEPSEELLRQRQGAFIRRQRNGLHHLEIFATAEQFEQLVTVMNTATNPRTGTGSGTGAGHGAMNAPAADTPEDAGHGSEPATDGPAGPAAVQEPAQDWAPAATGGAGWETGPAAGAGWIVGPAAVSASDTRAGVVSTSAAGATGDEFVSDPGPGYGFGPVPDPGPGDHRAEAGDTGAGGLDRRTRAQKQLDGLVGACQISLAAGTLPASGGLRPQVMVTIDYRDLLARLGNGTGTTSDSAAPAGTATDCPVHMAGTVDVAGTVDMAGTVDMAGTVGAAGSGRRTGGLPGTGSLLFTGPVTDSTIRKIACDADIIPVLLGTADRVLDIGRASRIFPPHIRKALIARDQGCAFPGCTIPASWCEAHHIDYWSRGGSTGTENGTLLCSHHHHLIHKEHWTIRVRAGIPWFIPPPHIDPAQTPRRNNYFHPARLDPAAX

SEQ ID NO: 9 - protein, 967 aa, synthetic construct
  REGION 1..967: note = EpiCas009
  SITE 967: note = misc_feature - Xaa =
MPNRKVTLTAFSRMDHRVEALEEGLNEVRASIAGVQATMRESYANIVALLEKHLGKSIATEGGTSEKKDKPESSEVKNNVTLEFRQSAKKVELPSFDGDDPAGWISRAEVYFRVQGTTPAVKVSLAQLCMDGLTIHFFNSILRENEDLSWEELKEALLERYGGHGEGDVYEQLTDLKQEAIDDYITEFEYLVAEIPRLPEKQYRGYFLHGLKPEIKGRVRSFAALSEMRRTKLLQVARVVEREVEGGSELKPNRGPRFGFGSGSHKNGSQSDWVMVRRREGSRNEGVKSNTDGPKGDRKRIGPRDRGYTQLTYNELMDYKQKGLCFKCKNPFGPMHRCPAKELRVLIVDDVENEEDEERILAVEVGEEEDEKGEMSILNLHHITHETHHTMKFQGTIRGVEVLILVDSGAIHNFISQKLVHQMDWPIEPTAEMNVKLGNGFQISTQGVCRGLEMCIGDLKMNPEMHLFELGGIDVVLGIDWLKTLGDTITNWKQQTMSFWKDKSWVTLKGHEGCRRQTVALQSILNRPKPTSQGLLWEMDNVKHKGKGVNELSIQQQAEMEVLFNKFEHVFQTPTGLPPKRNRDHAITLTDGHGPVNVRPYRYPHHHKNEIEKQVKEMLTAGIIRHSTSSFSSPVILVKKKDGTWRMCIDYRALNKATIPDKFPISVIEELLDELHGARYFSKLDLKSGYHQVRVKDSDVGKTAFRTHEGHYEFLVMPFGLTNAPATFQGLMNDIFRPLLRKNVLVFFDNILVCSKDWETHLHHLEEVLRLLAAHSLVANQKKCYFGQRSIEYLGHMITEEGVAVDSRKVDSVLSWPQPKNVKRVRGFLGLTGYYRKFIRDYGKIAKPLTELTKKDGFKWGVEAQKAFDELKKRLTTAPVLTLPNFSKEFVIECDASGSGIGAILMQDKKPIAYFSKALGVRNLTKSAYEKELMVVVLAIQHWRPYLLGRKFVVSTNQKSLKQLLQX

SEQ ID NO: 10 - protein, 1214 aa, synthetic construct
  REGION 1..1214: note = EpiCas010
  SITE 1214: note = misc_feature - Xaa =
MIKDFASLPPSHQHKLSLQCQLSTIDDHQTHVIPVLIDSGCTDSIIDEAFVRQHNISTKPLPTRVIVSNADGTKNRTGPLTEYVTLRLTVAGRTELMDFLVTGQREARILLGHDWLRRTNPNINWQTNTITYPSDDTEYHPEDGDRVIAVDLQSRIDKISVESNVSQTKSQQIAEESERAKSTLTFRDVVPPFYHHFEPVFTKASFDKLPPRRVWDHAIELLPEAKGLDCKTYPLNRDEQIHLDEFLKENLETGRIRVSKSPYASPFFFIKKKDGSLRPVQDYRKLNALTIKNRYTLPLISELINRLKGARFFTKLDVRWGYNNVRIKEGDEHKAAFRTNRGLFEPLVMFFGLTNSPATFQTMMDRLLRDLINEGSVIVYLDDIMIFTDSLEEHRKIVSKVLQILADNQLYLKPEKCEFEKKEDEYLGMIISHDTIRMDPLKVQAVAEWPIPRTKKELQSFLGFSNFYRRFIRDYGKIAKPLTILTGKVDWEWAEDQQRAFDVLKKTITTSPTLAIPNDEDPFKVECDASNYATGAVLSQQQEEKWRPVAFLSKSMNPAERNYAIWDKEMLAVMHALEEWRHLLMGAKHQFTIFTDHQNLTYFRDPQKVNRRQARWMDTLARYDFKLEHVKGSANTKADLLSRRVDHPRGERDNEGQVLLPQLAEANIYTMEDVLEEHYLDELLASQHKLDDYVVRKLKEDPKVWKKRDGIVWIGNEKEDELTLGSFENKIYVPQDPKLRARIIEEEHDTSLSGHPGERKTHEGVNRSFWWPSLRRDIRKYVAGCEICQRTKSHRQKPHAPLHPNPIPDRPWQIITTDLIGALPESNGYDAIQVFVDRFSKMAHFVPTHVTLDLLGYAKQLRDSVIRLHGIPEKIISDRGPQFMSNFTKDFYQTLGIEPGLSTGYHPQTDGQSERINQDLEHYLRTFINHRQDDWADWLAIAEFTYNNHLHSATNQTPFFVNYGSHPRKGTGQKPSGRSQAAEDFATSMTKLHEQTRQSLLLANQNLKKYYDRKRTEAREYHKGDKVWLEGTHISTDRPMKKLDDKRFGPFTVKAKVGPSAYLLDVPRSWKAIHPVFNEILLSPYHTPEFPNQPRTSKPPPIQVDGAVEYEAKEIIASRPTKLKGAKLDYFVHWKGYPITERTWEPDHHLKNSPSLITTFHRKHPAAPRVIASAALRFRPYENFTTTTEKPRLFDWITNRFTDCGAKILGTRIX

SEQ ID NO: 11 - protein, 977 aa, synthetic construct
  REGION 1..977: note = EpiCas011
  SITE 977: note = misc_feature - Xaa =
MSITDEYFQLTTKYRAQYGERTIVLLQVGAFFEVYGLKNPRTKVVTGSQIAEFAQICQLSVSEKNVCVEQDHVVMAGFRDYTLEKYLQKLSENDYTAVVYTQTKEGKNVTRQLHAIYSAGTYISYDNDSSQQITNHIMCIWIEKYQALDKSARLSCGVATANIFTGKSEIFEYQTAYYMNPTTFDELERCVSTYCPSEVLVLSTTLPQDVVQTIVQYVGITHPSRHIFCASNMTDAVKNCTQQKYIHHMLTTFFGEESQQLCAEFSNNEIATQAFCYLLHFVQEHNPDLVRKIEIPRFSSQSKTMLLANHTLRQLNIIDDLSASGKQAGQYSSVLSFLNKCASPMGRRLFQQQLIAPTFDQEWLQKEYNMTELMLQPDTEPMIPMLRKQLATIRDIEKICRQIVLHKIYPDSIAHLYDSLQTIQQIHVCFAELPKVLEYLHHSTEKIDQVLHTMQTYLLIDRCRGIQSVQSFPHSIIQPGVSSSLDKIIQTYEENLQHFREIHAFFNKIMRAKEGGDAEYIKIHTTDKSGVSLQITKKRATVLKSLLKGLADPKIQLSGGLYFCVEDIKFSSASTSADEIEIPCLKNICKALLTSEESMNQEIAKSFQDFLTTFENLHLENLEKCALFVAKLDVLHCKAYLASNYNYCKPTIVADHQKSFVDARDLRHVLIEHIQINETYVPNDFCLNLPDQPLGVLLYGTNAVGKTSLIRALGIAVIMAQAGLYVPCSAFTYQPYQSIFSRILGNDNLFKGLSTFAVEMSELRMILRMADESSLILGDELCSGTETESALSIFTAGLLHLHAKGASFVFATHFHEILKFEEMQQMPKLALKHMAVHYDPQRDCLVYDRKLQDGPGNRMYGLEVCKSLYLPDDFLQSALAIRNKYYPTSRGELTHHTSTYNTQKIRGICEMCKTNMGEEIHHLQPQKEANDKGFIGTIHKNHPANLMTLCEACHLKQHKSSITQKRKKTTAGYAVLX

SEQ ID NO: 12 - protein, 1028 aa, synthetic construct
  REGION 1..1028: note = EpiCas012
  SITE 1028: note = misc_feature - Xaa =
MEIFISDNTLNMSKKEDVEPVETNKIMKEYLDLTKQYTKIYGEKTIVLLQVGAFFELYGLRDDKGTILESQIEDICIICQLNYADKKLMYNSKQVIMAGFREYMLDKNIPKIIEAGYTAVVYVQEKDGKNIKRVLHSVCSQSTYLSCETDSSPVMTNNIMCIWLDTFKPMDRNVSTVSKTRDTIVYGVSTINIFTGKSSMFEYQTPFILNPTTFDELERYVSVFSPSEILFVSSLEKEINRTILQYIGVKCPSIHIYDSRDMENKTIIACSKQVYVQHMLSTFFGEEAMNVCREFQMNTMATQAFCYLLNYIQEHDKNIVRKISIPEFNNTSDRLLLANHTLKQLNIIDDSSIDGKKTGNLSSVLSLLNKCCSPIGKRNFKMMLLNPSTNETWLQQEYDMIEYMLQSENIYFIDMFRKQLSQIRDIEKICRQLLVLKVYPSSIYQLYKTIGVIHNLHICLAENKKITDYLCKDISKEQINSYHYINDLCLQINEFLENHFVLDDCKNIQSLTSFENNIIKKGISQPLDDLIKHHYEKIAIFEFVKKQLNEFMYSNGQNRDIEFIKTHETEKSGLFLQITKTRANILKNYIKAKLEKDADYSFHNKELQFSFYLKDIKFGVASSANEEIHIPILQKICKELITIKDEIDVVIRETYLEILKKIEDKWLPSLEQLANYVANVDILQCKTYIAKNYKYCKPEIVKSEKSFVSAQELRHCLIEHIQQNEIYVANDICLGNEKSGMLLYGTNAVGKTSFIRALGISIIMAQSGMYVPCSRFQFKPYTAIFSRILGNDNIFKGLSTFAVEMSELRIILKMADKRSLILGDELCSGTETESALSIFVAGLMDLHDKDASFIFATHFHEIINYDEIKMMNKLSLNHMSVIYDREKDALVYDRKLKDGPGTKTYGLEVCKSLYLTDEFLDKAYAIRNKYFPETRGELNFKSSTYNVNKIRSICEVCKNEIAEETHHLEEQHTADTDGFIGHFHKNHKANLVSICKNCHDKIHHDNSGKNTLNGKQRKKTTKGYDFMX

SEQ ID NO: 13 - protein, 856 aa, synthetic construct
  REGION 1..856: note = EpiCas013
  SITE 856: note = misc_feature - Xaa =
MLLTEEYLEEQKKLELKYGKNVVLFMELGSFYEIYEANGIGKVKEISNILNILQTKKNKNKPESQRNPLMCGVPSVSLDKHLNRLAQEEKWTIAIMSQTATDNGFERKITEIISPGTNVRNNIKDDTNSYLASLILDKNTKGIYSCGLSLIDVTTGNIKVYEGYGVHNDKEKILDEVNLILENYNIKELILLDNLDSNKLYYKFPSINMKTSNKSIHYKIQLITETFNKDFSELGLEQSPYIIDSLVGLLEFLIDHNKSLVVKLNSITFINNKEFMYLGNNPLKQLNIIGDDFSVEKLINKGISAIGRRYIREQILNPIINADEINNRYKYSLSLSKSNKLPTIEKSLKNIYDIERLSRKLELKTIKPFELGNLVTSLYASSDIIKNIKMLDTLTTFESYINLDLIKDYNSIHWNFFKDEQLMTLKTELELIMDLSNYEFDSFIKYSDKDGYYYEFTNKKYENLSFTSTIEHTRKLKNSIKLFTSELSSINTRRLVIESKMMEISNVLFKDVLDIFDITIINIEINKIQRIEFYLNNTKLLAKKYCIPTILDDVENIFDVTNLRHPLVEHLEQEVFVPNSIKFNKENKGYLLYGQNSSGKTVLSKSIGIAIILAQSGFFVPAESLAFTIKDSLFTRIIGADNINKGLSTFAVEMLELKNILNRSTPDSMIIGDEISHGTETTSGVSIVASAILHFNAPFIIATHLHQLDSINDIKEKPFIHFIHLALTFDTSTNSLIYNRTIQKGKGSSIYGLEFAKSLDMPFDFLDKAYAIRKEIADDISGLEQLTISKPSSYNSKLFLGTCYLCDNKGEEVHHIKHQHLADDDGFIDTLRKNHKSNLMVLCSSCHNKQHEKKIX

SEQ ID NO: 14 - protein, 984 aa, synthetic construct
  REGION 1..984: note = EpiCas014
  SITE 984: note = misc_feature - Xaa =
MSAKKGFSMIDEYFNIYNEKIKEYGKDIAVLIECGSFMEIYQIDNNEEKIGNAYEISKILNICYANKNGDLSNNNRSYPNFVGFTTNSMSKYLPILLENNYTVILVNQLETNGNKKGKLIQRGVTAVYSKCLQPLEMDTNADNQLLYISLDVKLIHSNVLKRNKTTMYELNTSICCVNNFTNSIEIYENNYTFTKDCIENCLNDFDHLLYKFFSKDINIHLVGENIINFESELLKFFNSRYDNMRFHNFDKQKHKEYIKTDYQNEYFKKVYNHINFGLLTPIEYLNITTMPSLSIVNLMYTIDFIGRHDLKYIRNLSIPKMMNDSDHLFLALDTLNQLNIDKGVFDIVNCTKTAIGKRYLKSLLCKPLKNPNEIEYRYKLTDELESIINTNNEIDQLLSCIIDFEKLHRKMSLEVLHPFEFEKLHTCYKNVNKLINVLSNYPLFHQIIPNNVKLNVFNEYINSYMETFDFDKLKKYNLNTSKDEISNYFLKGVIVELDEIQLKIDNITEEIERMRVKYNTICENNCKTKNPDYIKIAYTETEGYSFSCTKIKYQTLINAIKESSNFKIKQTNNIVKFFTPELVDLSNKLLTFKDLLKNKINLHYISTLKLYYYNYHDLFTSMTTFIQILDVVNSNLKCKNKYNYCRPIIDDNENDSSFFKAVGLRHPIIEVITQSNKYIPNDIVLDDNNIGILLYGLNSSGKSSLLRAIGIAVILAQCGLFVPCNSFIYKPFHTVISQVDLSDNMYIGKSSFITEMAGLKKILDLSGKNTLVLADELCRGTETYSAISIVCSTMIKLIQSNTKFFFTTHLHQIPQLKRINTLKSIDICHLSVTIKNSNIIFNRKIEKTSGDPLYGLEVCKTIINDNDFINDAFEIRNELTRNNTQILSHKKSNYNKKKITSYCEICNSCNSLETHHITEQYLADKNGIMPDGNHKNNLYNLVTLCHDCHLKVTLGKIKTRGYIQTINGRILDYNFTEDTTEKVX

SEQ ID NO: 15 - protein, 1018 aa, synthetic construct
  REGION 1..1018: note = EpiCas015
  SITE 1018: note = misc_feature - Xaa =
MTTEHKKYEYLKFNKSLNEEYLLLQEKYEKIYNKDFTVVLMQVGSFHEIYATNDRGYDLHKLSNILNIIVSKKNKKNPEVSEKNPYMIGFPILATPKFINILVDNGFHVIKIDQVTPPPNPKRAITQIYSPGSYIEGISSYDSNYILSIYIEEIKQMNNSYILFAGLSIIDLSVGKCIIHETFSTKDDEKYSLDEVLKFIYNFNPKEIIVYYKNLITYSENELLTYLELNDKKYLISEFSDNEYTKIIYQNNFLKEIYNLETCMTHIEELDLERINNGRLSFILLLNYCKKMNSTILNNIYKPEFYLNTKYLHYGNNALKQLNVQTYNSNEKSLFDVINYTSTSMGKRYLNFNICNPISDINILNDRYDKISELKEKNIDLSNKLKKILDIERLHRKISLQNLNPHNFVDLHISYSTILSLYEDIKKTKLNKIYNEKVKMNLENYISYYSRLFNLDEMEKYNLNDITNSFYNENINEKIDILQKSIKKEYKLIENLRDELEKFIDCKKKDYFNSFNEDKSPIQINYNEKDKYHFSTTSKRGSILKNNIKNNSKYNYDSYKFKDQSNTMKITCTYVDNISDKLVILNDKIRPLIKNTYLNDLKEMYEKYNDLYLKINNIIAEIDFINSGSICSIRNKYCKPKIILKDKSFMNVKSIRHPIIEQICSNKYVPHNLNLDDNQIGILLYGLNSAGKSSLMKSIGLNVILAQIGYFVSASEFVFSPYKSLFTRISNIDNIYKGLSSFALELVELNAILKRSGSNTLVLSDEVCKGTEYNSALIIVSAMIKMLVESNTSFISATHLHELTKLDAIKCISKIGIYHISVKYINNNIIFNRLLKKGNGTEEYGLDFAKYMIKNNKFIDICNNMKKDINNITANKSKYNKKLIVDKCQICKSIKNLETHHIEFQKNTDEYGFIIKKTLNHIHKDHISNLVILCSECHDDIHNNKIIMKGYEDTIKGSILKYKRSKCIEEKKYNDDEIKFIINKPNISQKKVKDLFEKQFKKNITIKNISKIINNKYX

SEQ ID NO: 16 - protein, 949 aa, synthetic construct
  REGION 1..949: note = EpiCas016
  SITE 949: note = misc_feature - Xaa =
MYNIIYLKINIVMTLIEEYFEFQDKYTKIYGEDTIVLMEVGSFFEIYQVGDLGKAKEIASVLNMILTKKNKNINEVTFKNPLMTGFPTVSLEKNVSRINAQSKYTVVLVKQRGQSPNITREVDEILSPGIQYRINTFKNNFLANIYVEYYRKNMFGIGISVVDITTGENYLMDSVSLEGFPDNPLSEIQQMVTKYGPSEVIVSMVDFESAESEATRIRVLLDEMIGKYSWKSCDSANYKVSFLNEMFSEIYKVKSILTPIEYLGLEHNQLAGNALIDSIGFIQKNNPCILDKMPRPEYINCAKYLTLNNDALSQLNVVDNNKKANRKGSLFELLNTTVTAAGGRLYGRRLSNPISSKEDLNAIYAEIDLFISDSKFAEVRREIAPILDINRIWRRLVMRKGDPMDIWNLYTSIKILADMKNDFSWIPNLENLSNSAQSANKYIESIFDISRIEDSYLSNLEDNIFKKENPILDKLEAELAEIKYKSQIIAEMFANHSFFTEKTKLVYTDKEGFYIETTPSRYKQYLGLNTAPKSDILAGFDVYKNKSKVRLTNDDLRKLSESKVIKIQKMSILIKEMFVKEVDEMYSAIGDDVESISAFISHIDVMAANAYNSVNLSLFKPELIDNEEGYSSVECHALRHPIVERLTHSEYIQNDVLFSNNKYGKVIFGVNSTGKSTLLKATGLAIIMAQAGMHVPSKMKLSPYQSLYTRITSGDDLFSNKSTFTVEMLELKQILEKADHNSMVLADELSHGTETNSGVSILAATINTLSKRKATFLFTTHLHQITGVRSIMDNKSIDLSHLSVNINPITGVIEYDRKLKDGAGESVYGILVAKGLGLADDFINDATSILNEVKSNRTQLDAITENNTNKYNSNKVNKNCEICGFQSSETHHIKEQADFKNQKYLEIQKNAKYNLVNVCNDCHKKIHSGKIVNLMYKQTTEGVELKITX

SEQ ID NO: 17 - protein, 880 aa, synthetic construct
  REGION 1..880: note = EpiCas017
  SITE 880: note = misc_feature - Xaa =
MPSLIKEYFKIQEESEKKFGDKTVIVMHVGGFYEVYSYEGLGKADVVANECNMMLTSKDKSKEISITNPQMCGFPLASLLRYMYFLTSKGFTCVTVKQDEKVKEKRTIDRIFSPGTCVDDSESSIVASIYADDGCIAVSWIDLTSGKVMFEEIYNDNEAYRREELTRIIETCGCKEIICMSKNGIMYDDAHEIDFCNIYEHISHQNDVISRAYPNDSTVSPIEFIDMEMFHIARVSLILLIEWVEDHHQSLIQRIRIPERINRKSLALHNTSVHQLQLVSQDKKSLFDVINKTNTSMGKMLLKQTLLNPYSDVSKLNGMYEDIERISKVDVEVVKKVLKNIGNVDRLARRIANKSINLEDIRHLILCFENGLDIIEHMRELSVHNMISENDVKRCYIAWHSTIDMEKDVFREGVYDDVDILKKERDTIMYMMDANAKRFSKTLGVNEGVKFELHKGTYGLITTPGRAKTLKNRVGNNVVFQADCKQKVVISTPDIQSLIHKLHGAIDAYDECMEEKMKEFVEILYSYHEIICTFGTYIAQVDVLLSHYLVAKAFNYTKPVVKEGDKSYITGKNIRHAIVERLNGNTLYMGNDVDLSNEKGLLLYGVNGSGKSCFSKSVGICVIMAQIGMFVPAETFEFCPYERIFTRISSEDNIYKGQSSFYVEMMEMNTILRFANEKSLIIGDEICKGTENISAISIVASMCNMISKIGATFVFATHLHGLVDLEPIKQIIDTIQIKHIGVTIESGVVTYDRHIKNGEGEHLYGLEIATHILGNKEFASLALETRNALLKKTPPKKSKYNARVLKKVCHICGRKDEQLDTHHINYQCDAHENIKNTKGNLVVLCKKCHDDEHHGFLSIKGWKDTSKGVILDYEFVSEKX

SEQ ID NO: 18 - protein, 927 aa, synthetic construct
  REGION 1..927: note = EpiCas018
  SITE 927: note = misc_feature - Xaa =
MPQLLVDEYIELTNEYRKKYGEKTIIWMQTGSFYEVYAWNEEDEQIKVSQNILQIRITTKKSGNNRSCLMAGFPDHSYKRFEKRLLKENYTIVYVDQIKKDPIERGVTKISSPGCVFDSDDDSKESILMSVLIEIEDNDFYGYYTIYDSNIGEIRMLSIKNEENQTIDHIFDNIGDIISENRVNEVLLNIVSEQYIKLPETNSKILFHYNKIDKIDELLKPLLQNDILSKYFKKYLSIYENVIDSLELSKCLPQEIVNLIYMLDFLKEHEPIFVKNLQRPIVDGPNQIKYMEFYNHALQKLQVISNEGNDLIKFIDKTLTYGGSKKLKYLLKNPSNNIEELKKRYKSVDLFVNNRQLLNETKTYLKICDLHRFYRRFAIGKINVYNDIPRIVNINENINILINIFKNVDNSIYWLPNDKIIQNFKDYCGDLIYTFCIDNCKSSGNVFNKDIVPELDDLYLKSESLNQELESIRTYLCNLINEPIYLKNTDKDGFFFETTKKRGTKIAKQLKENNKFDLEISNSTSVSKISSAGVKKISVQLCDLQTKIIDLTQKKVSEKVLFYYDTYFESSIATIIESMAWLDVYYSYSKSAIEWNYVKPNLVECENSYIDAKQLRHPIIEQLLSIEKQAFIPNDIRIGFKESYLLYGVNSVGKSSLLKSVGLSVIMAQAGMFVPASDYKLCPYDKLIVRIGNTDNLFEAHSSFICEIREANQCVSNTNNRSLVLADEFCASTERESATQIVTSMLLWLNEKKSSFIFATHLFELIEAPIVNVKICHLKVRIESDSLVFDRKLTSGPPTERNYGILVAKKIFKNNKFLKMMDRCQTKTSTRTDINRSRYNRGVLLSECAICAYSPIDEMSLPLDTHHINMQCMANNDGFIGNYHKDIVSNLVVLCKKCHIMAHNGKLNIKCWEQRDCGNVLNYEINX

SEQ ID NO: 19 - protein, 806 aa, synthetic construct
  REGION 1..806: note = EpiCas019
  SITE 806: note = misc_feature - Xaa =
MLHPRLQEMLAARGIRRLYTHQAQAANLALGGAHVVVVTPTASGKTLCYQLPVLDRLLRRPQSRALYLFPTKALAQDQHHGLTQDLLEAGTDAAAMIYDGDTPQAQRRAARRIAQVLITNPDMLHVGILPYHTQWRELLAELDYVVIDEMHAYRGVFGSHVAHVLRRLQRLCAFYGSAPQFILTSATIANPAELATNLIGEPVEVVAESGAPSGERHVALVNPPVIEARLGIRRSPLVDARQLALSLAAQGEQVVCFTRSRLAVEQLVIALRERAGRVGLAPEAIRGYRAGYLAAERREIEAGLREGRVRCVVATSALELGIDIGGLTVAVLVGYPGSVASTWQRIGRVGRGQAPSAAFLIASASPLDQYLMAHPEHLFGGGAEAAHINPDNLYVRSGHEQAALYELPMAEGEAAQDDDRRAILAALEDAGEARLSRGRWFWSGQGFPAGEISLRSAEAARVSIVARRAEEGRDITIGEVERSSAPRWLHEEAIYLHEGQPYLVRTLDLEGGVAQVEPATTDYFTVASEREEIEIERVVASTDGERMTTAHGEIRLTRQVTGYRRQRFETQEVLGWGVVDLPEQVILTSAFWLGVKPELVARLDAQGLWTADRGGARGPDWEQQRDRARLRDGYRCAHCGAPERPERAHDVHHIVPFREFGWEPGRNDAYRYANRLANLVTLCPRCHQLAERQVALGSTLSDMGHVLRYLAPLWLLCDPEDIGIHADSAGRRAERPTLFIYDQLPGGAGLSDQLPRLIVPLLKSAAQVVSDCPCETGCPACIGPVLAPAIGRKRRAVGLLEALAWX

SEQ ID NO: 20 - protein, 853 aa, synthetic construct
  REGION 1..853: note = EpiCas020
  SITE 853: note = misc_feature - Xaa =
MSWNEEITPLAALLQRWRQDPAFRRRVAAWARAPAREAQWAPIPEDLHPRWREALRQAGFSMLYTHQVEAYRAARSGAHVALFTGTASGKTLAFLLPILQALCEDPQTTALFIYPTKALAHDQLAVLRAWLSALRLPAAALPYDGDTPGEARRFVRERGRLLLTNPDMLHLGILPQHPRWAAFLSHLRFVVIDEAHVYRGVFGSHMVNVLRRLRRLAAAYGASPQFLLASATVANGPELAEGLVEGSVRIIEEDGAPYGERHFILYRPPLLDAATGLRQSALTAAAGLIWTLLEHGIPTIAFARSRMAVERLLRMVRSAWAERGGDPEEVHGYRGGYLPEERRAIEKGLREGRIRAVIATSALELGMDIGTLEACVMVGYPGTIASVRQQAGRAGRRAPLSVAIMVLTATPLDEYLAGHPEFLFRNPPEAARFDPDNLAILADHLRCAAFERPLDPGEPFARTLDTGWIVERLIADGEPLYRNPTDGRVYFVADRYPAQGVSLRTSTGDRVKIRLGAGKGGRIIGEVDRPSAPRLVHPGAVYLHEGAAYRIVSVDWEQGEAMAEPFDGDEITEPIVEARWYLDAERARRTEPWGIGAWGEVTIVHQVVGYRRLRWPGGELLGWAEVETPEEILSTTAWWLTIELGLVERLKEEGIQIGPLDYGPEWEAIRRQVRARDGYRCRVCGAPEPPGQRHDVHHLRPLRTFRDPAEAYALENLITVCRRCHRRLEQMLGTRSALSGLAHLLHGLAPIFLMSDPADLGLLVDPESREGGGPTVLLYEGVPGGVGFAAHLWAVQEALLEAALEVVRRCPCERGCPACVGPPGEMPDLKGETRRLLECIFAADEAAASKVQX

SEQ ID NO: 21 - protein, 845 aa, synthetic construct
  REGION 1..845: note = EpiCas021
  SITE 845: note = misc_feature - Xaa =
MADLERLLERLRRDPTFGPNVTAWRRREGRPARYGETPAWLDPRLQEALRAGGIERLYTHQVAALQAVRQGEHTVVASGTASGKSLCHHLPVLQALLEDPSDCALYLFPTKALAHDQEAVLRALVERIPDLPDSAKPFPASYDGDTPGQARRAIRERVRIVLSNPDMLHAGILPSHPHWAPFLHHLRYVILDELHTYRGLFGSHIANLLRRLRRVCAFYGSRPQFLCASATIANPGDLAGRLIGEPATVIEEDGAPRGPMHLLLYNPPLLDPALGIRRSALQEARRLAVRLIGAGLQTVVFGRSRRGVELLLTYLRQDLPPGLRPALRGYRGGYLPALRREIEAGLRSGEVRGVVATNALELGVDIGTLAACIMAGYPGSIASTWQQAGRAGRRDQPGLAVLVAGANPLDQYLVTHPDYFFGRSPEQARINPDNPFILAAHLRCSAFELALEDGAPWGTPAPPDLLEDLVREGSLLHEGGRYYWIGVGSPAREVSLRTASGDTVTIIEESSDGIGTIGQVDRPGAAMLVHEQAVYIHEGTFYRVERLDWEAGLAYVRPAQVDYYTQAHLRVDWRVLSEEAQAPQGRGSRHTGEVEVHAQATAYRRVHLHTQESLGWGAISLPPQEFRTQAFWLTLPWPAQEHLRPDYGPNWEEQRRRARERDRFTCRHCGAREEVAGREHDVHHLRPFRTFGYIPGENDAYLEANRLENLVTLCRVCHARVDHGPRQETVAALQGLGHLLAHVAPLYLLCDRGDIRETTRLRALPEGRPVVLIYDDCPGGAGLSPTLFSCADALLQTARERLQECPCAGGCPSCIGPPEEPARDKVIHILEFLLEEEAPPPGTAX

SEQ ID NO: 22 - protein, 765 aa, synthetic construct
  REGION 1..765: note = EpiCas022
  SITE 765: note = misc_feature - Xaa =
MNKLWQHPNPDWVPVSHFGELRYESIDVVMARWDWDKLIWGKVRRFVFNLQKRIYKATKSGRYRKAKSLMYLLQNSYYATLLAVRTVTTENFRGKCFCARAKTFTSEGKRTAGVDRVKANTPKRKMALVKDMLDTIQRGWDKYRPMPAKRIYIPKANGKPKVSEAKLRPLGIPTIKDRAMQAVTKIALEPFYEAKFESCSYGFRPAMGCHDAIDRITAALLHKQKWVLDADIKGCFDNIDHKFLASQIDTHWRPIVKRWLKAGYMEKSDYNQTNMGTPQGGTISPLLANIALDQMETDLIEHLRGIKGWKKKIGVTTVSIVEKTEKPQKEKKTQKKPKKANNKGTKEPQKKQKNVYEGAKKSYKCRRNLLIDLVRYADDFVVLHKDKEVIEESKRFIGKWLEVRGLTLSEEKTKIVHSTEGFDFLGHHIRHYENRIKGTYKLKLLKGTPTEQRRAKATHVLRVEPTKDKIKGHYRVIGDTIWKLKAATPSELIRILQPKISGWANYYKTVHSSEAFGKLDHLLWKRLYQWAQRRHPNKGKRWVTNKYFATVNGRRWTFAEIVGKGKDKKIVKHLKGYSKHKERTGSYARVGYDRSYYDGDTAYWAERLSKGYGNITPSKAKMLKRQDGICPVCKCRFGNEDLPEAHHIHPRHLGGEDKYTNLVLVHLHCHDKIHRENPGIKGKLVSQTSPELQGFLNNGMAPAFQAEGMKPPANTSTVLRTGKGAGIITPASDEMKSPVGTSTVLRTGKGAGIITPAPDDNKETX

SEQ ID NO: 23 - protein, 771 aa, synthetic construct
  REGION 1..771: note = EpiCas023
  SITE 771: note = misc_feature - Xaa =
MDTLQLSNPDGRVRSQHSLTGLPSDKKHRDHTDSSGRLVPSCYRVINSSDMCDWDWDSIIWGKIRRLVFNLQKRIYKLTKAGKYRKARSLMYLLQHSHYAMLLGVRKVTTENKGKKTPGVDKVKVTTPRQKMNLVVDVLDTIQMGWDKYEAKPAKRIYIPKANGKERPLGIPTVLDRAMQAVTKSALEPFYEAKFESASYGFRPGMGCHDAIDKIASVLLTKQKWILDADIKGFFDNIDHKFIVEQTDKHWRPIVKKWLKAGYMEENKYNPTKNGTPQGGIISPLLANIALDQMETCLIEHLRGIEGWKTRIGNTKISIITDKKTQKKYESRKHLQLSVIRYADDFVVIHEEKEVIEESERFIKEWLGLRGLTLSEEKTKIGNETDGFDFLGHHIRHYENRIKGTYKAKLLNGTPTEQRKAVTPHVLRVEPTKAKVNAHYQELSDIIGKMKATTPSELIGILQPKISGFANYYRTVHSSKAFSRLDHLLWKRLYQWALRRHSNKGKRWVAAKYFCTVKGRKWTFAEIKGKGKDREIVKSLKGYSKHKVRTGSHARVGYDRSYYDGDTAYWAGRLSKGYGNISPSKAKLLKRQDGLCPVCKCALTNEDLPEAHHIKPRQYGGLWEFKNMVLLHLHCHDKIHREYGEQKRKLCKGTREYDELVKKGVFVSPEVEAKYGPDIAKMRKGPEVNKGSSKILRLGSDPGIISRDKDTVPQETHSNGNNEDDELIQVKSWKSGEIKMIPRSKMYRKTKRVRDKITNKWKLVKMWFCKX

SEQ ID NO: 24 - protein, 706 aa, synthetic construct
  REGION 1..706: note = EpiCas024
  SITE 706: note = misc_feature - Xaa =
MNILWQHPNPSEVNVFARAQKQFTSEWIPVSHLDRHRYESIESVMAKWDWDKLVWGKVRRLVFNLQKRIYKATKAGRYSKARNLMYLLQNSYYATLLAVRTVTTENKGKRTAGVDRVKVNTPKRKMALVKDMLDTIQRGWDKYRPMPAKRIYIPKANGKLRPLGIPTIKDRAMQAVTKIALEPYYEAKFESCSYGFRPAMGCHDAIDKIAGTLLNKQKWVLDADIKGCFDNIDHKFLASQLLPLQHWRPIVKRWLKAGYMAKSEATKKSEYYRTDMGTPQGGTISPLLANIALDQMETDLIEHLRSLKGWKTKIGTTTIGIDINKKTKKSYKSRKNLKIDLVRYADDFVVLHEEKEVIEESKRFIGKWLEIRGLTLSEEKTKIVHSTEGFDFLGHHIRHYENRIKGTYKLKLLNGTPTEQRRAKATHVLRVEPTKEKIKGHYQDISDTIWKAKAATPVQLIALLQPKISGWANYYKAVHSSEAFNKLDMLLWRRLYQWACRRHPHKGKRWVANKYFATVSGRKWTFAEIVGKGKDRKIVKYLKGYSKHKERTGSHARVGYDRSYYDGDTVYWAERLSKGYGNITPSKAKMLKRQDGICPVCKCRFGNEDLPEAHHIHPRHLGGEDKYTNLVLVHLHCHDKIHRENPGIKGKLVGQTSSELQGFLNNGMAPAFQAEGMKPIGTSTVLRIGKDAGIITPVSDGNKETX

SEQ ID NO: 25 - protein, 747 aa, synthetic construct
  REGION 1..747: note = EpiCas025
  SITE 747: note = misc_feature - Xaa =
MNILWQHPNPEWIPVSHLGRYRYESIESVMAKWDWDKLIWGKVRRLVFNLQKRIYKATKSGRYSKARNLMYLLQNSYYATLLAVRTVTTENKGKRTAGVDRVKANTPKRKMALVKDVLDTIQRGWDKYRPMPAKRIYIPKANGKLRPLGIPTIKDRAMQAVTKIALEPFYEAKFESCSYGFRPAMGCHDAIEKIAAALLKKQKWVLDADIKGCFDNIDHKFLAVQIDTHWRPIVKRWLKAGYMEKSDYNQTNMGTPQGGTISPLLANIALDQMETNLIEHLRGIKGWKKKIGTTTVSIVVGGKKAKRPQKENEKSQKEPKKANNKGTKESQDKPKKVYEGAEKSYKARKHLHIDLVRYADDFVVLHEDKEVIEESKRFIGKWLEVRGLTLSEEKTKIVHSTDGFDFLGHHIRHYENRVKGTYKLKLLNGTPTEQRRAKATHVLRVEPTKEKVKLHYREISDTIWKLKAATPVQLIAILQPKISGWANYYKTVHSSRAFGKLDMLLWRRLYQWACRRHPNKGKRWVANKYFATVNGRKWTFAQIVGKGKDRKIVKYLKGYSKHKERTGSYAKVGYDRSYYDGDTAYWAERLSKGYGNITPSKAKMLKRQDGICPVCKCRFGNEDLPEAHHIHPRHLGGEDTYLNLVLVHLHCHDKIHRENKGIKGKKVSQTSPELQGVLNNGMAPAFQANGMKTPTLTDTVFRVGEGAGIITPALDEKKPNADTSTVLRTGKCAGIITPAPDDNKETX

SEQ ID NO: 26 - protein, 758 aa, synthetic construct
  REGION 1..758: note = EpiCas026
  SITE 758: note = misc_feature - Xaa =
MKQNGIDEITIKSSGEINPKSGTNTRILYEHQKNAMECLDIMNKEKAYSTLVVLPTGGGKTYTASMWLLKNAIDRKKKILWIAHRQMLLEQAAESFQKFAYAEVIPHISSFHFRIVSGASSHDQTIHIRPTDQLLIVSKDSIGRNLQRLDAWMAGENEIYMIVDEAHHSTAKTYRKVISYIKEKVPNVKLIGLTATPFRTAEEEQGLLAKIYTDGVQNGQAVHGDIGITYQIGLKELINRRILSKPVFESYYTDEFYGKELGLKAWESIQHLDMIPDDLAKKMAESSARNKLIVETYQANQEKYGQTILFAVSVEHAIQLTAQFRKAGVAADYVVSSIKDMITGVTLSREENEKKINAYRVGDLQVLINVNILTEGVDLPKTQTVFLTRPTVSTILMTQMIGRALRGTAAGGTANAYIVSFIDAWDEHIAWVNPESLFVGNNDFQENAYEQKQRDLRMIAISKIEEFARILDDSTDTSLLEKVPFTQRIPVGMYAFTYLEENGGIEHAYQVMVYNSSQKAYENMMDSLPDLFQSFHAEEEYLSEHQLMEMEKQCRDTFFCGEMVPPYEPKDVIHILKYYAQYESVPKFYTFDEVDRSKLDVGMIAQHIWAEDMGERKKAEYIDKIWNDADDNMLRLFFGKKLYFLRQLDIELMKIRYPDIYEETANVVYETRKLEELSLHDIGKVNPKLEMQLRDAAFEKAKTSDGKYQCAVCGMKNRSKTCFHVDHIIPMNQGGKSVPENLQILCRQCNGIKGDQIX

SEQ ID NO: 27 - protein, 755 aa, synthetic construct
  REGION 1..755: note = EpiCas027
  SITE 755: note = misc_feature - Xaa =
MARDYIEVKSFGKVFPKKGANTRMPYEHQRDAMENLDIINKSNKFSTMIVLPTGGGKTYTASMWLLRNAIDKKKKILWIAHRQILLDQAAESFQKFAYSEVIPHIPFFQYRIVSGASCHDRVINIQALDNLLIISKDSIGRNLNGLDVWLKDEKEIFIIVDEAHHSTAKTYRKVIEYVKSKVSNVKLIGLTATPFRTASDEQGLLAKIYEDGVENGKAIHGNIGITYQIGLKELINHRILSKPIFESYYTDEMYGESLGLNSWKSIQHLDNLPEDVAEQMADSAARNKLIVNTYKAKQKEYGQTIVFAINMVHAVHLSALFNKEGIKSEFIVSDVRDSVTGVRISREENERKLEEYRSGNVKVLVNVNILTEGVDLPQTKTVFLARPTVSTVLMTQMIGRALRGEAAGGTTLAYIVSFVDNWNEHIAWVNPDSLFSGNNEFTDNPVEHVKHELRMIAISKIEEFASVLDDSVDTTMLEKVPFIQRIPIGMYAFTYLEENGVDFSYQVMVYDSTRKAYEDLMASLPQLFKIFDCKDEYPSEELLEEIAEHCRDTFFLGDMIPPYEEKDCLRILKYYAQYEIPPQFYLFDDIDRNKLDVAVIAKYIWDEDMGQRRKTEYINSIWENSDENLLRLFFGRKLYFWRQLDIELTKLSNPNIYKKEENVQLGIRKLEDLSLFEIGKVNPEMEKNLRDTAFEKAKDSEGNYICACCGQKRTDRIFFHVDHIIPMNKGGKTVPENLQILCRQCNGMKGDKFAX

SEQ ID NO: 28 - protein, 781 aa, synthetic construct
  REGION 1..781: note = EpiCas028
  SITE 781: note = misc_feature - Xaa =
MVAINKRALSEEDIKMKYITPAIEKAGWDIKTQVRAEYTFTDGRIIVRGNLVARGKKKRADYILSYKPNMPLAIIEAKDNKKPLGAGMQQALEYGEILDIPFIYSSNGDGFLEHDKFTGKERVLSLDEFPSPNELWERYKKGKGIQPHEEKIIKEDYFFDMSGKTPRYYQRIAINRTIEAIAKGQKRILLVMATGTGKTYTAFQIIYRLWKSRTKKRILFLADRNILIDQTMANDFKHFGDKMIKVNRKNISKAHEIYLALYQSMTGSEEWQDIYKQFSPDFFDLVIVDECHRGSARDNSAWREVLEYFSSATQIGLTATPKETRDVSTSTYFGEPVYTYSLKQGIEDGFLAPYKVVRVSLDKDLEGYRPAKGKVDKYGNLIEDRIYNVTDFDKNLILEKRTEIVAKKITEFLKKTNRFDKTIVFCVDIEHAERMRQVLINENSDLVKENPKYIMRITGDDEEGKAQLDNFIDPASKYPTIVTTSKLLTTGVDAQTCKLIVLDSNINSMTEFKQIIGRGTRIKEEYGKYFFTIMDFRGVTRLFADPEFDGDPVVVYEPKKGEDIVPPAEGDYGDFGDSVDGTVGEPDSDENETGTRIKYVVDDVEVMVVNERVEYYDKDGKLVTESLKDYTKKNIRNEYADLNEFINRWNSEDKKSAIIEELKERGVFLDAIKEEVGKDLDEFDLILHLAFDQKPLTRKERAYNVRKRNYFSKYSDVAREVLEALLDKYMNEGITELESMEILKLDPFRKIGTPKKIIKAFGGKEKYIQTIKELEREIYAX

SEQ ID NO: 29 - protein, 821 aa, synthetic construct
  REGION 1..821: note = EpiCas029
  SITE 821: note = misc_feature - Xaa =
MSNPGNSVLSTRYRDARTLVRRVCRLPGEDRAPFKEKVARLREHFEQFNVDVSELCQWFMGLRKAHAAAHAANAATSPAGFGPLGDFLLVPALDGVDADESECDRWRLAVFDAVAGFRDLTAPIREAVPPALHAAIDATARNGPHTNPKNVAMKRLFERLRTLDSAHRLVLLKSAAEWVVARYRRGMENWVRQREEWEKEKTAWETARPQLTPEVRERFTQVFRSLVWDRDKRPGVTNKRPRICPYERLKGNLDNCIYAGQKGHGPLCWKYAGFKKTREEQFSRFNDRGFEKDAAEFLARRKDGVRRHEVLRQMFRGRSADEQRFTDNWSAYLRALSLNEDTVVEHGRLPHCLRIGETFEKSKCEWNPHTELCKQYKRALDNPDNGFDEETLRLEPLYRQWRRDYLAGPRKPSFRYPSSRDLPMPKIFGAGFHEIDFDRSIVRLRLDDMSAGQWIEFGFTPWPRGYKPSRDEIKAAGRVTSVHVHFIGTRARLGFRFSVRPKPSRFTCSQDELDELRSRCFPRQAQDQQFLDAARQRLLDSFPGGAEEAKRNMRLLAVDLGETGACAAVYQGTTHQTDCPLAIIKINRLYAGRPDALEPDVKGRPSKEKRKFDKGDPRGVRKEHVARHLARIAQKTAEITQHPRRQPAVPQTVTPGAHDLRSLKRHTAWMIRDWTRLNAAQIVKVAEDQRCNLIVFESLRGFLAPGYDKLCPKEEDKKRWLAMFAYGRVRRKVVEKAVERGMRVVTVPYYKSSQVCSTCGAVQENTNLHRENKRDRKFICEKNTCAVELNSDANAARVLARIFWGEITLPSPDEKTVRRSX

SEQ ID NO: 30 - protein, 773 aa, synthetic construct
  REGION 1..773: note = EpiCas030
  SITE 773: note = misc_feature - Xaa =
MTRIKYRQERTLVRGLQRLPNQDKAEFNKNVLGLRRHFEQFNLNVAELCQWLISFKPENPGSVCETKLFWEFMLEPENFCPDTYDRGPDWLRHEIFVLAAGWRTFEDIKAHNMPESLFESIKIASSKPRSKTAEALFIRLKSLEASHVMVLLKSASEWLSTRYVRQSENWKQNEQEWQKKKAAWEDKHPELTPAIRDKYNAIFVELGISEKRPHVCSWKKLSENKDNCDWAGERKNIGDKWISHSDLCIKYHEFARKLRSKQRQHFVDNANQYLELRRRYPQWTRDMAMNGLFKNVPLARNWFRNAWTNYLNALNILETTILENYSGHLPHCEKLSDECVFKKHTDNCRRYKLLLGEKLSNQERELEETYREWRREFLAPPNKPFLRYPSAQKLPTPKLFGRGYYDLDFTRHVVKLRLDDMPADNFVSFGFKPWPRGYDKKPGEINITSVHVHFIGTRARVGFRFAVPHSDSRFSVSQDKIDELRSGGFPGKSQDQEFLNEARQRLLDGMNENQKSALRIMAVDLGTHRAAAAFFTGCIFNKAKLLKLKKIDLLTEPKTDTTKPEKLSADEKKIQREKGLTQHHVGKHFETLEARTKEIISKRQNMKMAPSDDTPDIVGDHDLRHLTSHIRRMIRDWVRLNARQITELAEEENVDLIVFESMRGFRAPGYDKLDLKKKRRLAFFAYGQIRRKVAEKAVERGMRVITVPYFKSSQICAQCGRSQNDKNKLRDNKWKQSFQCEFSDCNYKTHSDENAARVLGRVFWGEITLPTDX

SEQ ID NO: 31 - protein, 950 aa, synthetic construct
  REGION 1..950: note = EpiCas032
  SITE 950: note = misc_feature - Xaa =
MQQGCDSRFDTTIKEQEVSLFNTYTKYVDCVNKLPNAQLVDADFSLKLLSMVIANALEVLNGIKKTVDNDKKYLLLSGGFKLPEVVDVLARLTSNVRQDGAIEIANFGLNSRAVRKRDILNSKKNELDEIESELGALTNKIKKSAQKPKKEDINSKGRLTQERNSLVAEIKKLQAMNKYGLIFRRKNCDGDFEYFLALVDRDHMENLSDKSKFKSAQSTGYQYMEYNCLKLKSLLQIIFESDSDNLSGVRKLERYGTVKPLFLSKEHSRELEKSKTLIAWLDENIQKIVDTIAGTTNPKITYTEYGNTDAAKNAADVWRDFERHFNRQSYSISWCHLNFEKLKTTKSVELFQIANKDHSIHPDFTSDERDRKKLNRSSGRPNLFTTYLDNVLTDEIGNHYQLLGEGVEYFKHKCGAEPSTPRRKSIDRYYVEFRVAFVPNKSESWEETNSSVKNAISQSDSPKHFIGIDRGENAIANIVVIDENNRAILKQDMSCLAIFSDITPHSAKKSYIFLTGDEPVYIATKSATDALTDKTEIKKLSDVMFTEYRDKLYKLLPPSEDKKVIPSKSSPCLDEMNIEDLKKLISKLESPEYNPASRKMYLAKTNTPIIDYVYIRRYNILLLQAKYMLGKKQVRVTDSNFEQEKIQRKEYLLHATNSIKDNYSAYFVHHVCKLAEKYNAYIVFENLNKKNGDTREINFLSGEQISGLTPKQQNQLKGVSFYVNMEQKLINKLNYLATKDAQSHSLTLKGQFTQSIDYKGVITSMTNEQINLITSPKKQEQVEALKSGLGKGKKNCYQIGCILYVDAANTSKECCNCGFSVNTALTRCERTDEGLSFSGSSNTSYKWGDTRLTERGIDESFDLNNKSDGVKLSVRPGKVVNAKLSTRDVYDPISCLACGFDGRGTGHDHLHENDNDAYQKIKLLQTCDELAAFNIAKRGGKLIKGQEEVX

SEQ ID NO: 32 - protein, 1213 aa, synthetic construct
  REGION 1..1213: note = EpiCas033
  SITE 1213: note = misc_feature - Xaa =
MNYSDFVGLYSISKTLRFELKPTPATKKLLDDSGVKETDKIRHEHFKQAKKILDEVHREFINDALKNVSLSTSDLQDYIKLTLDKASKKADVQKAQKKIFSSFEQAYKITNYEWQEKLDAKKFFLQSPGIQLEIASQLAEKIAKNLEMNEDDVKNTLKQFDKFSTYFKGYAENRKNCYSFDGKATEIANRTIAQNLITFYKNIEKFNKYYSGNSLLADDVSKYFLLENYNQFITQQSIAQNYNVKIGELNYIINQERQKQKKDAKANLPLFKVLYKQILGDATKEVPFEFIKDDAEYKAIIHNLKDKMPKWIEEIEDHFVSQAKQLQNPEGVYLGKKAINTLLQKYISIDVRPLINEELPELAKNKSSKTDDDESLRNQFISVKDFFEALDKVQEQSETSILRSDESAALLPSQFIWNKLCNDIEKDVKVAKDSAPKIDTSNKNSVKSALDSFNDLFRMYSYFELRYKNQPVAVMDEDAKFYQIFNAEDTPFANEKDKRFSQVYDLIRNYLTKKQYSLDKWKLNFDCSILLGGWDLNKEPEKHGVLLRHKQQYYLAIIDNSAKNAFDKKENLDLYTAGADDWQKMEYKLLPGANKMLPKCLFSKSFRENFGVPSDIDVLYKNDEYKKGDKFDINKMHKLIDFYKDAIKKYEGWSMYEFVFSDTKTYQSIDQFYHEVDRFAYRLDFVNINNQVLSKMNENGQIYLFEISNKDWLKEARGKANLHTQYFLNTFRGGDFKLNGEAEIFFRPKSIEAKVDKERKSKHEIIENRRFSEDKILFHVPITFNRNSKLSSNFAFNQHAIERIKTNGVNAVIGIDRGEKHLAYVAVVDKNGKLLDKPVSLNQIHSICKGRDFPKDYFDELKKREDERRSNRQDWDAVRRIKDLKDGYVGHCVKQVVDLMVKHNAVVALENLNFGFKQGRSKIERSTYNQFEQALLKKLQYVVDKNKDDDEIFGVQKGVQLAPPDVAPGKISNHMGFVFYVDPSYTSAIDPKTGYRQHVRLDDRVKTKNFSKFVDDAFDKIYFKDDKLIFEFNWRGLAKAQNGLGVSKNKKTDIKQDKKWGITLDVPRTVFHKNVAGKSETEIVNPQQLLICSLNEAGIKLNEDIKLQLVKNTNLSSKFVKSFVYCFNLANKLRNQIDGEDAIISPVYPNGFDSRNQKLDGKYKWNGDANGVYNIARKGAILLQKLNKASTPKEFNCKVSSEEYDGFVGGEKX

SEQ ID NO: 33 - protein, 1132 aa, synthetic construct
  REGION 1..1132: note = EpiCas034
  SITE 1132: note = misc_feature - Xaa =
MIFNCILTEHQETQNTKVLVEKFVNDFKDLMGDMQKQEEYLAENYGVDKSLYKIESIKNEGDEKSKMDTATFYIYPYFDFDKNLSIEECIKRVDSFIGDKKLNRNVEELIGVSDNAGGFSFYFNNGLQLLQNNRIDEIKNAILQASSLWNGKENELQERLEFLNKKAKQVLPVRIVKNWHEYRSDIGGSIQSWVSNSLRQDIEIKKLLYGYKEKKVKRGGEIEEHDIEGHIQEIEKVLGDAELGGYKQYFENKEDEGGIRQTEEVIAKVKQLKKHLDDEKEKIDTEQPKINPAILNDYRDVLADFRNTFNHLYQKRYGLEEQDEGIEQKDEKGKKIQTVNKKYPKLFKELPKIPKFLGAVKIEEKGVYDKYICSYNGLKKGVEFLGGVTFTGSKRIDDYYTYRNDSSKDKEEIEKARKRSIERVQRVLENILRLYRSTDAKQLKGQKIKSLLAKYCKDISLLDGEYNYIYRNERYARDKRGQKIELKRVDDELVEDDFIQGLISDLQSFEWRLDNIKQGKWYERVAGWGALVEIEKIKIGLMAWFYEISVPHNFQEIEKNKLHFRKVEAIVKRYNQDEVLDNKEKNTIIQQGIVSEMRGMIARMSKQEIIARYVVQPVNAEQKYPLVMDEGKYYIHPKEILDKDEIKEQPVNMIDISKEKDLTEEKNSRIKVRRDSLFAITSSKYQTQFLNNSLNRQLEKWQNLNPQLSEYSFIVEDTHKIKWVQDGDSYTPNCDEVLLSRLFVSVPFKIGVENKDKTVAIKQQNKFIGIDIGEYGVAYYGLDGSDFSAKPFVAGFFFQPDMRKIREGIAKNKERQQAGTFTNSNTQIKRVRDNATTKIRNQVHQLVVENNALPIYEKEVSAFESGSGKISAIYNSIKRSDVYAESKADDMEHKLIWGNDKIMVGAEIGAYATSYMCSVCYESIYAYIAKDDYEREYEVIDIVGEQKQIKDKWNATVKFDIEGKEMYAYIEQKDKPVGKGDTFNGKGTINFVRKYERPPLDVVRKIERLPSAIQQELNECTKKERVKSNGEKEKISVWENRRGSQGVFRCAFCNKCSDADVQASMWIALKGYLQNVKNAVQKKENKEQYKMYEGSIGKEVVGEIAKGFSQGGKEQVRFILDFAKDNSIMLRX

SEQ ID NO: 34 - protein, 745 aa, synthetic construct
  REGION 1..745: note = EpiCas035
  SITE 745: note = misc_feature - Xaa =
MATKTYRARLSSIDNRTQQAVVRTHYFFNHCLRQMIERYLDMRKGKYGPFCKQLGDLLLTRSHTDAHGIMDQLTRGAPSTQTDQEWAVLVKHHHREYGPLFLQHEGFAVVDGVVVHTKPQGRHEPTPGRLAVTAKFWHQICDMACAFLKSNQELMAVWRKDKTEWLKTKNAWEVDNPEFMTFWNGPYADFERACEAARVAAQEAAGQTPTARKRDSRVRGKRIDRWHLWYEWLVAHPETVGWRQRAEAGDFKPVPDAVQAAIRKKTKRQDKYVGKYLDWLRENNPELKALDSLRRTYVRRYLRFKRPPTLTLPSANKHPYWFTLELNEFYKGADFEKGCVKMRLIDCDADGLLEMKWFDVRMGCDHRLKPAWRKEKFASDGRYPPYLGGKIGRKLDRPAECAADRKAGVKGVKLVLDKGRRELFFTLVEQDCPPRLKFKKTKNRRCTADNLFDAGDQRVPIRVMSVDLGIRHIGAYAICEGTKQDDHWEMKYLKKGLLSDSSLPELGQIRLHDRHLKKLRSRQGDAPTGERNFVALQDHRTGMADDRFKKAAHLLIETARRAGVDIIVFEKLDTLKPDAFDERWINRQLRDMNRRQIVTHVAQQAGEFGLLCKDDISPWLTSQVCSRCYRPGWRFSIKPKAPYKEQCSRAACQDFGYPIWDPGGHLFRCPHCGYKVNADINAAGNLAAKFFGHGFWFDNNLSRDKASGCFIWTDDQRRCFDAREAFEQWAAEASRRQALKEAPFX

SEQ ID NO: 35 - protein, 4488 aa, synthetic construct
  REGION 1..4488: note = EpiCas036
  SITE 748: note = misc_feature - Xaa =
  SITE 1496: note = misc_feature - Xaa =
  SITE 2244: note = misc_feature - Xaa =
  SITE 2992: note = misc_feature - Xaa =
  SITE 3740: note = misc_feature - Xaa =
  SITE 4488: note = misc_feature - Xaa =
MATKSYRARILTDSRLAAALDRTHVVFVESLKQMINTYLRMQNGKFGPDHKKLAQIMLSRSNTFAHGVMDQITRDQPTSTLDEEWTDLARRIHKTTGPLFLQAERFATVKNRAIHTKSRGKVIPSPETLAVPAKFWHQVCDSASAYIRSNRELMQQWRKDRAAWLKDKNEWQQKHPEFMQFYNGPYQNFLKLCDDDRITSQLAAEQQPTASKNNRPRKTGKRFARWHLWYKWLSENPEIIEWRNKASASDFKTVTDDVRKQIITKYPQQNKYITRLLDWLEDNNPELKTLENLRRTYVKKFDSFKRPPTLTLPSPYRHPYWFTMELDQFYKKADFENGTIQLLLIDEDDDGNWFFNWMPASLKPDPRLVPSWRAETFETEGRFPPYLGGKIGKKLSRPAPTDAERKAGIAGAKLMIKNNRSELLFTVFEQDCPPRVKWAKTKNRKCPADNAFSSDGKTRKPLRILSIDLGIRHIGAFALTQGTRNDSAWQTESLKKGIINSPSIPPLRQVRRHDYDLKRKRRRHGKPVKGQRSNANLQAHRTNMAQDRFKKGASAIVSLAREHSADLILFENLHSLKFSAFDERWMNRQLRDMNRRHIVELVSEQAPEFGITVKDDINPWMTSRICSNCNLPGFRFSMKKKNPYREKLPREKCTDFGYPVWEPGGHLFRCPHCDHRVNADINAAANLANKFFGLGYWNNGLKYDAETKTFTVHTDKKTPPLIFKPRPQFDLWADSVKTRKQLGPDPFXMATKSYRARILTDSRLAAALDRTHVVFVESLKQMINTYLRMQNGKFGPDHKKLAQIMLSRSNTFAHGVMDQITRDQPTSTLDEEWTDLARRIHKTTGPLFLQAERFATVKNRAIHTKSRGKVIPSPETLAVPAKFWHQVCDSASAYIRSNRELMQQWRKDRAAWLKDKNEWQQKHPEFMQFYNGPYQNFLKLCDDDRITSQLAAEQQPTASKNNRPRKTGKRFARWHLWYKWLSENPEIIEWRNKASASDFKTVTDDVRKQIITKYPQQNKYITRLLDWLEDNNPELKTLENLRRTYVKKFDSFKRPPTLTLPSPYRHPYWFTMELDQFYKKADFENGTIQLLLIDEDDDGNWFFNWMPASLKPDPRLVPSWRAETFETEGRFPPYLGGKIGKKLSRPAPTDAERKAGIAGAKLMIKNNRSELLFTVFEQDCPPRVKWAKTKNRKCPADNAFSSDGKTRKPLRILSIDLGIRHIGAFALTQGTRNDSAWQTESLKKGIINSPSIPPLRQVRRHDYDLKRKRRRHGKPVKGQRSNANLQAHRTNMAQDRFKKGASAIVSLAREHSADLILFENLHSLKFSAFDERWMNRQLRDMNRRHIVELVSEQAPEFGITVKDDINPWMTSRICSNCNLPGFRFSMKKKNPYREKLPREKCTDFGYPVWEPGGHLFRCPHCDHRVNADINAAANLANKFFGLGYWNNGLKYDAETKTFTVHTDKKTPPLIFKPRPQFDLWADSVKTRKQLGPDPFXMATKSYRARILTDSRLAAALDRTHVVFVESLKQMINTYLRMQNGKFGPDHKKLAQIMLSRSNTFAHGVMDQITRDQPTSTLDEEWTDLARRIHKTTGPLFLQAERFATVKNRAIHTKSRGKVIPSPETLAVPAKFWHQVCDSASAYIRSNRELMQQWRKDRAAWLKDKNEWQQKHPEFMQFYNGPYQNFLKLCDDDRITSQLAAEQQPTASKNNRPRKTGKRFARWHLWYKWLSENPEIIEWRNKASASDFKTVTDDVRKQIITKYPQQNKYITRLLDWLEDNNPELKTLENLRRTYVKKFDSFKRPPTLTLPSPYRHPYWFTMELDQFYKKADFENGTIQLLLIDEDDDGNWFFNWMPASLKPDPRLVPSWRAETFETEGRFPPYLGGKIGKKLSRPAPTDAERKAGIAGAKLMIKNNRSELLFTVFEQDCPPRVKWAKTKNRKCPADNAFSSDGKTRKPLRILSIDLGIRHIGAFALTQGTRNDSAWQTESLKKGIINSPSIPPLRQVRRHDYDLKRKRRRHGKPVKGQRSNANLQAHRTNMAQDRFKKGASAIVSLAREHSADLILFENLHSLKFSAFDERWMNRQLRDMNRRHIVELVSEQAPEFGITVKDDINPWMTSRICSNCNLPGFRFSMKKKNPYREKLPREKCTDFGYPVWEPGGHLFRCPHCDHRVNADINAAANLANKFFGLGYWNNGLKYDAETKTFTVHTDKKTPPLIFKPRPQFDLWADSVKTRKQLGPDPFXMATKSYRARILTDSRLAAALDRTHVVFVESLKQMINTYLRMQNGKFGPDHKKLAQIMLSRSNTFAHGVMDQITRDQPTSTLDEEWTDLARRIHKTTGPLFLQAERFATVKNRAIHTKSRGKVIPSPETLAVPAKFWHQVCDSASAYIRSNRELMQQWRKDRAAWLKDKNEWQQKHPEFMQFYNGPYQNFLKLCDDDRITSQLAAEQQPTASKNNRPRKTGKRFARWHLWYKWLSENPEIIEWRNKASASDFKTVTDDVRKQIITKYPQQNKYITRLLDWLEDNNPELKTLENLRRTYVKKFDSFKRPPTLTLPSPYRHPYWFTMELDQFYKKADFENGTIQLLLIDEDDDGNWFFNWMPASLKPDPRLVPSWRAETFETEGRFPPYLGGKIGKKLSRPAPTDAERKAGIAGAKLMIKNNRSELLFTVFEQDCPPRVKWAKTKNRKCPADNAFSSDGKTRKPLRILSIDLGIRHIGAFALTQGTRNDSAWQTESLKKGIINSPSIPPLRQVRRHDYDLKRKRRRHGKPVKGQRSNANLQAHRTNMAQDRFKKGASAIVSLAREHSADLILFENLHSLKFSAFDERWMNRQLRDMNRRHIVELVSEQAPEFGITVKDDINPWMTSRICSNCNLPGFRFSMKKKNPYREKLPREKCTDFGYPVWEPGGHLFRCPHCDHRVNADINAAANLANKFFGLGYWNNGLKYDAETKTFTVHTDKKTPPLIFKPRPQFDLWADSVKTRKQLGPDPFXMATKSYRARILTDSRLAAALDRTHVVFVESLKQMINTYLRMQNGKFGPDHKKLAQIMLSRSNTFAHGVMDQITRDQPTSTLDEEWTDLARRIHKTTGPLFLQAERFATVKNRAIHTKSRGKVIPSPETLAVPAKFWHQVCDSASAYIRSNRELMQQWRKDRAAWLKDKNEWQQKHPEFMQFYNGPYQNFLKLCDDDRITSQLAAEQQPTASKNNRPRKTGKRFARWHLWYKWLSENPEIIEWRNKASASDFKTVTDDVRKQIITKYPQQNKYITRLLDWLEDNNPELKTLENLRRTYVKKFDSFKRPPTLTLPSPYRHPYWFTMELDQFYKKADFENGTIQLLLIDEDDDGNWFFNWMPASLKPDPRLVPSWRAETFETEGRFPPYLGGKIGKKLSRPAPTDAERKAGIAGAKLMIKNNRSELLFTVFEQDCPPRVKWAKTKNRKCPADNAFSSDGKTRKPLRILSIDLGIRHIGAFALTQGTRNDSAWQTESLKKGIINSPSIPPLRQVRRHDYDLKRKRRRHGKPVKGQRSNANLQAHRTNMAQDRFKKGASAIVSLAREHSADLILFENLHSLKFSAFDERWMNRQLRDMNRRHIVELVSEQAPEFGITVKDDINPWMTSRICSNCNLPGFRFSMKKKNPYREKLPREKCTDFGYPVWEPGGHLFRCPHCDHRVNADINAAANLANKFFGLGYWNNGLKYDAETKTFTVHTDKKTPPLIFKPRPQFDLWADSVKTRKQLGPDPFXMATKSYRARILTDSRLAAALDRTHVVFVESLKQMINTYLRMQNGKFGPDHKKLAQIMLSRSNTFAHGVMDQITRDQPTSTLDEEWTDLARRIHKTTGPLFLQAERFATVKNRAIHTKSRGKVIPSPETLAVPAKFWHQVCDSASAYIRSNRELMQQWRKDRAAWLKDKNEWQQKHPEFMQFYNGPYQNFLKLCDDDRITSQLAAEQQPTASKNNRPRKTGKRFARWHLWYKWLSENPEIIEWRNKASASDFKTVTDDVRKQIITKYPQQNKYITRLLDWLEDNNPELKTLENLRRTYVKKFDSFKRPPTLTLPSPYRHPYWFTMELDQFYKKADFENGTIQLLLIDEDDDGNWFFNWMPASLKPDPRLVPSWRAETFETEGRFPPYLGGKIGKKLSRPAPTDAERKAGIAGAKLMIKNNRSELLFTVFEQDCPPRVKWAKTKNRKCPADNAFSSDGKTRKPLRILSIDLGIRHIGAFALTQGTRNDSAWQTESLKKGIINSPSIPPLRQVRRHDYDLKRKRRRHGKPVKGQRSNANLQAHRTNMAQDRFKKGASAIVSLAREHSADLILFENLHSLKFSAFDERWMNRQLRDMNRRHIVELVSEQAPEFGITVKDDINPWMTSRICSNCNLPGFRFSMKKKNPYREKLPREKCTDFGYPVWEPGGHLFRCPHCDHRVNADINAAANLANKFFGLGYWNNGLKYDAETKTFTVHTDKKTPPLIFKPRPQFDLWADSVKTRKQLGPDPFX

SEQ ID NO: 36 - protein, 1292 aa, synthetic construct
  REGION 1..1292: note = EpiCas037
  SITE 1292: note = misc_feature - Xaa =
MENKNCNFDKFTKQYQVSKTVRFALTPIGRTEEHIIEKQYIEAAQRKDQAYKIVKPVIDKKLCVMIDDVLTHCEKQDWEKLNELTLQYQNDKTSVEALGEQQGKIRKNISKEFENSIEYKNFFGKDSEKLFKTFLPQCLEEINASEADKEAVKEFQKFKTYFNNFLTVRKDIFNDDSKQNTIPYRIVNENFMIFAGNRKTFSNIVKLIPDASAEIAKEGIERQEWEFYDVQNIDSCFEPDSFQQCMSQLGIQKYNFIVGLVNSYMNLYIQQHPEALEVKRSRLKLRMLHKQILSDRTNPSWLPEQFAEGEEGEKQIYEAIQALEDDLNKNHFQEKFDNLLQLIDTENPRIYIAASEMPRVSSALNYGWNGLNNVRMNVLQELNSEAKIEKILKQDVSLNELSDALNKYADIYKKEQVPTLQQYIEYGKELLQDCAVACNDYHASIRNNVERLNQNEKLIEVLKTYLDCYQRVMHFMNVFVVGDELDKDVDFYAELDELIEDISQIIPLYNKVRNYVTRKAYSLDKIRIMFEKSDFLGGWGQDFDTKKALIFEKDGLYYIGIIEKKYTNTDVQYLYEEIEEGNKAVHFVYNFQKIDNKNFPRIFIYSKGTNYAPAVRKYNLPIQNIIDIYNERKFQTDYKKVNEQEYYESLEKMIDYFKDGIMKNETYRKFHFNWKPSNEYENIKEFYDDTDNSCFLLEKEEINFNHLKEQADQGKIYLFQISSKDFNKGSTGTPNLQTMYWRELFSDQNCKEGIIKLCGGASIYMRDVSIKQPIIHKKDSWLINKWYMEEGQNKVIPDDTYVKFSQIVQGRMSEAELNVEEQQLWNSGLIQKKKATHDITKDRRFTRKQYMLHAPLIINYKQQDIPTPRRFNEEVRSFLKNNPNINIIGIARGEKNLIYITVIDQKGNILSGMQKSFNQIEEKGANSRIVDYYGKLQSVEDRHTEARKNWKQIGTIRELKEGYLSQVVHEIAQLMIQYNAIIVMANLNMGFKKGRMKVEKNIYQRFEKMLIDKMNYLAFKKNIEGKAINPYEIGGVMNGYQLTNKFTNFADMGSQNGFIFYVPAAYTSVIDPVTGFVDVFQRAEFKTGDFLQKFEDISWDDKEQSFVFTFDYQKFKCNGTCYQNKWSLYADVNRIETVKKNNQVYRQEQCNPNQRLIELFDSKGIAYRDGHNLVNDLGNYDSKLLSDILYNFRLILQLRNSMRDYSTGEVIDYIASPVMYHRERFDSQKKNPSLPLDADANGAYHIALKGLMCLQKINEYADPDGKMDIKNMKITNEEWFKFMQTRRESNVX

SEQ ID NO: 37 - protein, 1261 aa, synthetic construct
  REGION 1..1261: note = EpiCas038
  SITE 1261: note = misc_feature - Xaa =
MRRFFMTKMTDFTKLYQLSHTLKFELRPIGKTSENLQNSGLLEEDFKRSQDYVEVKSVLDEVHKKFLQDVLSDCDLSWQELADALKIFQVNKDRKVLEDVQKKYRKLLADRFNKNKFFKTLTEATPSKLFKSLLAEPDMAERKVETFKRFACYFKGYQETRQNIYSAEAQQTAAAYRAVNENFVKYLRVVELYENFRKNFPELAEEIGRRTAELTNGELSQILRIENYNRFIAQSGIEYLNSLIAQINSAVNLYRQAHNVKLSFVPLLFKQILSDREQAFTLERIEKDADLDEKLRAFCERHIGNVEIRGETGDLFSRLKVLLTTLNDDCELYIDAASLSAIGNALTGNWSCFRDAMTAYANETLKNKSLREKYCKQPVYSFSEIKSWRVVRTDDDGNVQPVCLSDYWHGEKTLELFAAEKILRNRILEMVRVPHDKNFRERKNDVALVKDYLDAVVEILHLLKPLNVGSENGGDLDLLGILTEFYEALSPVIPLYNQIRNYVTQKPSDIGKIKLMFNNPTLADGWDLNKEKDNTAVIFCRNGMYYLGIMNPKSKTDFNSLATDSSTDSYQKMVYKQLQNPNQMLPKVFFSAEKIKFFAPSEELLRRYEAGEYKKGEKFDLAYCHELIDFFKRSIDRHEKWSKFEFKFSETSAYSGINEFYREVAEQGYKMSFVNIPVKAVDQLVEDGKLFLFQIWNKDFSEKSTGTPNKFTLYWKALFDRQNLSDVVFKLNGEAELFLREPAITEPVVHRPGGKLVNKTVVAAVDGNGVAIRNSIPDAVYTEIYKHVNGMEEGTLSPAAREHLNRFPRLDWEPGMGLEATVKRTVVKDVKFQLVKDKRFTERKFSFHVPITVNFKSPRLKGAKLNEMVWEFLKDNPDVNVIGIARGERNLIYVNCIDLKGRILLQKSFNIVGGFDYHQKLDLRERERGQARKSWNEIGTIKELKAGYLSGVVYEIARLMVEYNAIVVMADLNGGFKRSRTGIEKQIYQKFEKALIDKLNYLVFKNESDWHVPGGLLNGYQLTGPLESFAKLGKQCGWLFYVPAAYTSKIDPSTGFVSLFKLSNYTNTEKRKAFFENFESIVYQAEQDAFVFAFDYKKFKDVENCWKTSWEVYSARRRLVYSRRSRQIEEINPTRLIKRALDKRGVVLSDGFDLKHYITSVEAVNENAAFFKDIFDAFGTTLQMRNSSGEEDYIESPVLNENGQFFDSRKAGKEWPRDADSNGAYHIALKGLLRMKSGQTAKLKRLDWFEFVQRRGFITEX

SEQ ID NO: 38 - protein, 1228 aa, synthetic construct
  REGION 1..1228: note = EpiCas039
  SITE 1228: note = misc_feature - Xaa =
MNDLSEFVGLFPVSKTIKWELKPVGMTAERMREAGFLDRDRSKRDAYTVVKSMADRFYRGYIDERLSTLDLDWNHLGDAMSALKESGETKDKRELENIKKSFKDSISKHIFTKKDDEDIFSAKVLARLRGTETDDEEVEALEKFDRFAGYFQDFFVNRRVFADTVRGSCAYRIVEDNFPRHFENCRKYQIIRRDNPELILELKRSMEGYLETDPDVLFSIDHFGKLLRQRDIDAYNRVVGSVFRSESDNSRGFNPILNEFHQRNPDSPKMLMQKLQKQILSEPDSGSFRMRNYENEGQMFEDLQNLWTGIETNRLLEIPASVLEEGEFDKSGVFISKAGVNTLSNWMFSDWERIGGLLQIFKINEMGDSASKSRKKIDKWLDSDSFSLDVLNRAVADETDIGIVPFLSRRLSDAAQQAREAYLGLEGCASMRREQYQGRVKTFVDSLLRYRDILKLFSYDPDLPLDRGFYDTFQFVYEEMASAYRAYNRCRSFITRKEYSTEKFKMSFDCPHLADGWDLNKESSYNSFLFRRDGLYYLGIRNPAWRYEDFSVKADPECDDFYEKAVYKQLQDPVKMLPKVFFSKKGLDKYRPPERILEGYENGLHRQGDSFDLGFCHELIDFYRDAISQNRDWDFFDFKFKETSEYSSISEFYQDVESQGYQMRFIRIPAQTIDEMVDEGRLLLFQMYNKDYSRDKTPGGKPNLHTMYWEAAMSEDNLRDVRIKINGYAELFWRDASIKDGTVHRKGSVLVNRIGKDRKPIPSEAYYDLCRYCNGIRDDLGAGKGYEDQIVCKNSRYDIEKDRRYCHDRMFLHIPLTFNFKSDGKTDVNRKVLEWIRRNDDVKFLGIARGERNLIYLSLVDSDGRILWQRSLNTIVQKDGRGNTRALDYHEKLAVREGERRNAQQSWGPMDAIKNLKEGYVSAAVHEICRIAVEEKAVIVIANLNYGFKNSRKKVEKQTYQTFERMLINKLQNLAFKDAEPGSPGSVLAPYQLCGPIDSMEDIPNHCGMLIHVTAAFTSRIDPVTGFVSVFNLSDITNNAQRADFLSRMTSIRYNQDEDVFEFSFDYGDFRTRLTPKVRKWTVCTYGDRYKYNRKDRTLVRISPTTMIKDALTKAGIRYEDGSDIRKEISGSDAVRQVFEAFEAILDMRVTTRDEDVIVSPVRDSSGRHFVSGTSGPGLPQDADANGAYCIALKGLLLARKIRASDEDRLPLLNNNDWVEFMQTRVMX

SEQ ID NO: 39 - protein, 1247 aa, synthetic construct
  REGION 1..1247: note = EpiCas040
  SITE 1247: note = misc_feature - Xaa =
MIEQFVNRYPLSKTLRFGLIPQGNTEENFKIMQILEKDEALARNYGKAKEIIDRYHKFFINSCLADFHLTDLEKYALLYYEPNKTEEEVAAMDETAKTMRQAISGLFCKENKAIYDRLSKKDLIENFAMSVIETDEERTVLESFRKCTVYFTGFNQNRLNMYTGEGKSTEIAHRLINQNLPKFLDNARVAKTILAALPKNDLDQIDVDFYDIFGINTQNIFEIPFYNQTLTQAGIDRYNQIIGGYTCSDGRKIKGYNEYINHFIQETKQKLPKFKPLYKQILSDRETISFIPKAFQSDSEVLSALRNFYIKKNVETDKSIRDVITELKKLFQEMDSFDEKGIYITNGVAITDLSQAVCDNWFVIKKAMQAEYDAEHSSKNRNEDYEKKRGNDLKKVKSYSLSALQRYMDAEMEDKKSLAEYIKTHTTQLCDLTASAYERVRHLLETEYSPTKKLTADADAIGRIKDFLDPIMEVFHFAKIFLGSGEEAEKDDVFYGIFSPLYDQLADIIEIYDKVRNYVTQKPYKTDKIRLIFERGDFLSGWAQPTESQAKEAHLMEKDGRYYLFITVTAINKADWERALYGKDNFQCACHIEYYKQKPDNKNTPRLFIRSKGDHYAPAVEKYNLPIQEVIDLYDKGYYKAEFKKKDQKLYYTSLRKLIDYFKLGFTKHENYKDFAFAWKESDAYENITEFYQDTMNACYRLERVTVNWNGIMDLVEKGRGFLFQIYNKDFSDHTKGTPNLHTMYFKMLFDERNLENGCYRLLGGAEMFYRKASLKLSETTIHPKGVAIKNKNPRSDRAERVLDYDIIKDKRYTETQFSLHFPIMMNCLAQGNPKLNLDIRKALLKSEHQYIIGIARGERNLLYVCVINEKGEIVEQMSLNEIIGDNGYTVDYHELLDRKEKERDAARKSWGTIENIKELKEGYMSQVIHKICELVLKYDAVIAMADLNGGFMNSRIKIEKQVYQKFEKMLTEKLSYLVDKKADPMSDGGLLRAYQLTNKPDPNKSVQHGMQDGIVFYIPAWCTSKIDPTTGFVDLLKPKYTNKEEAKDFFKRFQKICFNEVENMFEFHFHYPDFQRGITAGNTDWTVYTNGSRIRTFRNPEKNNQWDNTDIVLTDAFKALFAEYAIPCDADMKEAILAQDSPKFFKELCGLLSFTLQMRNSITGRTDVDYIISPVKNAAGRFYDSRKAASDLPCDADANGAYNIARKVLLFIRRLQAQEESNLMNKDLEKITNAQWLSFVQNGHEX

SEQ ID NO: 40 - protein, 1256 aa, synthetic construct
  REGION 1..1256: note = EpiCas041
  SITE 1256: note = misc_feature - Xaa =
MTKMTDFTKLYQLSHTLKFELRPIGKTSENLQNSGLLEEDFKRSQDYVEVKSVLDEVHKKFLQDVLSDCDLSWQELADALKIFQVNKDRKVLEDVQKKYRKLLADRFNKNKFFKTLTEATPSKLFKSLLAEPDMAERKVETFKRFACYFKGYQETRKNIYSAEAQQTAAAYRAVNENFVKYLRVVELYENFRKNFPELAEEIGRRTAELTDGELSQILRIENYNRFIAQSGIEYLNSLIAQINSAVNLYRQAHNVKLSFVPLLFKQILSDREQVFTLERIEKDADLDEKLRAFCEQHIGNVEIRGETGDLFSRLKVLLTTLNDDCELCIDAASLSAIGNALSGNWSCFRDAMTAYANETLKNKSLREKYCKQPVYSFSEIKSWRVVRTDDDGNVQPVCLSDYWHGEKALELFATEKILRNKILEMVRVPHDKNFRERKNDVALVKDYLDAVVEILHLLKPLNVGSENGGDLDLLGILTEFYEALSPVIPLYNQIRNYVTQKPSDIGKIKLMFSNPTLADGWDLNKEKDNTAVIFYRNGMYYLGIMNPKSKTDFDNLATDSSSDCYQKMVYKLLPGPNKMLPKVFFADKNIDFFAPSEELLRRYKAGEHLKGEKFDLAYCHKLIDFFKRSITRHEEWSKFDFQFSETSAYAGIDEFYREVAEQGYKMSFVNIPVKAVDQLVEDGKLFLFQIWNKDFSEKSTGTPNKFTLYWKALFDRQNLSDVVFKLNGEAELFLREPAITEPVVHRSGEKLVNKTVVAAVDGNGMAIRNSIPDAVYTEIYKHVNGMEEGTLSPAAREHLNRFPRLDWEPGMGLEATVKRTVVKDVKFQLVKDKRFTERKFSFHVPITVNFQSPGLKGAKLNEMVWEFLKDNPDVNVIGIARGERNLIYVNCIDLKGRILLQKSFNIVGGFDYHQKLDMRERERGQARKSWNEIGTIKELKAGYLSGIVYEIARLMVEYNAIVVMADLNGGFKRSRTGIEKQIYQKFEKALIDKLNYLVFKSESDWHVPGGLLNGYQLTGPLESFAKLGKQCGWLFYVPAAYTSKIDPSTGFVSLFKLSNYTNTEKRKAFFENFESIVYQTEQDAFVFAFDYKKFKDVESCWKTSWEVYSARRRLVYGRRSRQIEEINPTRLIKRALEQRGVVLSDGFDLKHYITSVEAVNENAAFFKDIFDAFGTTLQMRNSSGEEDYIESPVLNENGQFFDSRKAGKEWPRDADSNGAYHIALKGLLRMKSGQTAKLKRLDWFEFVQRRGFITEX

SEQ ID NO: 41 - protein, 1234 aa, synthetic construct
  REGION 1..1234: note = EpiCas042
  SITE 1234: note = misc_feature - Xaa =
MRNRYSKILCLLLLFACCLPQEGNAFWPFKKKKKEDKRLRKLIAQNLKAHPLVDKLKVKNAFGKNGYLETLPLGKEEKEAVKVFAGFGGFFNNYNKNRENYFSTEEKSTAIANRIVNENFSKHFSNVEIVTKIQKEVPELIQIVEAQFKGYDAIFTVNGYNMALSQAGIDTYNEMVAIWNKEANLYAQKAGKLPDGHPLKKKRNYLLSALFKQIGSEKEHLIQIDRFDGDEEVIEALTGVKKMLQEADVFEKLNMLVEDMENWDYSKIYLSAQSLSNVSVFLNNLYEDERENSWNYLDNVLREKWQIELQGKKKGTDLEEAIRKKKQSFYSIEELQEAVNAIEETDKCYNVSKWLLGAMKSERVIEEKKKDVEDFCTQWKNERNSLKETDITALKEYLEQWIFLARYCKSFYANGIEKKEKDEAFYHILEDVLYVLDEVIYFYNKVRNYVTKKPYSLEKMHLKFGHNELANGWSVNKEGNYGTAILRRNGKYYLAITNSLNKKMSIPTQLESTGNNYEKMVLNVFPNVFRMIPKCTTGRNDVKSCFERKEPNEYFFIDTPEFVNPFKVTREEYELNKITYDGVKKWQSDYSKNTQDEKGYKEAVTKWIQFCMRFLQSYKSTAIYDYSTLQQPEKYETVDSFYHDVEKILYECHFEYVPANKIEQLEEEGRIFLFQIYNKDFSENRRPDSKKNLHTLYWEALFSEENRKAKVIQLNGKAEIFRREKSIEHPIVHKAGEVLVNKRTKDGEPIPDDIYKDLSNYFNGRNVTSEKEEYKECLDKVYTSTKKYDITKDKRFTETKYEFHVPITLNYQADGVKYLNQKILHVLRDNPDVNIIGLARGERNLISYVVLNREGKIVNNQQGSFNIVGKMDYQKKLYQKEKNRDKERKTWKNIETIKDLKEGYISQVVHELTDMAIRNNAIIVMADLNFGFKRGRTKVERQVYQKFELALLKKLHYLVTDKTEGEAMLKPGGVLQGYQLAREVKTLKEIGKQCGCVFYVPPGYTSKIDPTTGFVDVFNMSGVTNREKKKAFFEKFDNMFYDEKRDMFGFSFNYEKFTTYQSSYRNDWTVYSNGSKYVWNSLKRTDELIDVTKELKLLFEKYAIDYRNEALFEQIMSQDTDKNNADFWNKLFWYFRVLLRLRNSSDELDQIVSPVLNQNGEFFETPKKITEKSYLSDYPMDADTNGAYHIALKGVYLIQEKIADESVDLDNKLPKDFYKISNAEWFMFRQKEKX

SEQ ID NO: 42 - protein, 1293 aa, synthetic construct
  REGION 1..1293: note = EpiCas043
  SITE 1293: note = misc_feature - Xaa =
MVSNKEKTPTYNSLTNLYSVSKTLRFELRPQYSTLDHINEDQIVGKGEELKNHYKTFKKILDQVFSRIINDSLDKTYLDQKYISTYQDLAFKHRDQLTDKDRAELKTLKETLKKQIDKSLDHKDKKAIFSDPVKFLLDNESEFTDLIGDNRPSIEAFNRQKGYLSGYLQNRANIFDHTTNETSVAFRIVEENLAIFLNNRITLQHFLEKVAGKDGLLKSLQEALFQLGFKLKLEDLLSLDYFNRTLSQSGIDQYNLLISGKTLEDGAKLQGINEILNQYLKQHQEEKLHKIKLKQLYKQILSESKTESFTLDFVEDNKGLAAMFLQFIDFANQLIEEKMPLLGMIQELKNSSVSAELLSRLHLNRKNIKRLSNFIYKDYGYIEQALEENFLSTVEGKITKKVLGEHRKQDTFTIHEILVALQKQQYEKDGTLESADRLFLPSIVDFVYQNLNCEYSTLLEKVRSEKQPLLELFKERQLLEDQDTESHSSKYPDHPFNDHEIKIIKTTLDFYKNLQSNLALLQISDENLKLDSEFYSEFDEFYQGLKNIIPVYNKSRNFLTKKPFSTEKTKLIFNSPQLLDGWSKSKESDCLGTIFIKDGKYYIGIINSATNAKKTLFEPHNFANFDQSQYFEKMNLFFLSDLKRDFPKKYFSEKWHNQYPIPADLREKYDYYRIDEHKDERKNDLEYHHQLIAYYQDCLKKDTEWQIYQFKYKSPEEYSDINEFLSELTPNTYKMEFTKIPAEYIKKLVDDGKLYFFQIYSKDFSEFAKGKPNLHTLYLKAVFDQKNAEEFNYNYKISGSAEIFYRPASIETRVTHPKNQPIKNKNKNNPKIESIFQYDLCKDRRYMSDKFFLHLPVELNRTPLLPNDSLVNSMVNQVVSSRNQNYFLGIARGERHLIYLVLIDQSGKIIKQQTLNQITSSYQEKSNNQTVEVVTDYHDLLNDKEKIRKKNLQEWQSVENIKELKAGYLSNVVNEIGKLIAEYQPVIMLANLNTGFKNSRIKIEKQVYQKFEKALIDKCNYFMRKDIDPSTIGGLYHALQLTKEYSKQYNGKQNGIIYYIPASYTSNIDPTTGFISAFVQTRYENVEKAKALIEKFNDITYDADESLFCFTVDYKKFSPEAKLWQQNIWQIYTNGDRIYTFRDKEEWQSKNYILVEEFKDLFTKYQINYRNDLKTQILSQTDAGFFKQFLFLLRLTLQMRNSRTADSNEADIDTKKRENDYIISPVKNQYGKFYDSRQDYMDWPENADANGAYNIARKGLIMLKHLKEGLPEKRICDISTEEWVQFVEELNKX

SEQ ID NO: 43 - protein, 1245 aa, synthetic construct
  REGION 1..1245: note = EpiCas044
  SITE 1245: note = misc_feature - Xaa =
MTRVFIFCLLYLKKTKYAPGVHKEGKMKINAFINCYSMSKTLRFKLVPEYETEKNLLEKGFLDRDKLRADDYDLMKKVIDKYHKHFIDKALEGFKFDLLQDYAEAFYSQSADDDGKKLEEIKKKMCKELATCFSKQDEFKLLDKKELVEKLIPAAEFIEDEEKDIAKRFKGFTTYFTGFNENRQNLYAAELKHGTIAFRLIEENLPAFLYNCKKGVKIFEELDEGDVETLNNELGEILSIGNVKDILNVEYYNKTLTQNGIDVYNQIIGGYTQEDGTKIKGVNEYVNLYNQTHDKKLPSLAKLKKQILSDSYSLSFLPAKFNDDSELLLSLKKFYSMVNEETGLSVEKAIQEMRNVFLHIDDCDLHNVFIDAKFINKVSNDVFGNWSVLIDGINAEYEKLNPFNGKNLGNYEEKRKAFLNKIESYSVDALQAYSGKEEKIADYVQKRAVELCDSVACAYENMSNKVINAREGKVKLYQDDEKTEIIKTFLDAVQEFKKFAEMFCYDGTDGDTTFYGEFANYYGQIAEIIPLYNKCRNYLTKKPYSEDKIKINFDNSQLLDGWDANKEKDYLTVLLLKGNNYYLGILDKNHKNVLIKDVPEKGQGEPCFKKMIYKLLPGPEKMLPKVVFSAKNIGFYNPDREILRIRENGTFKTGDGFNIDDCHKLIDFYKECISKNEDWKTFGFRFKETSEYKNIGQFYNEVKEQGYKISFTDIPESYVKDLVNDGKLYLFRLANKDFSPYSKGKKNLHTMYFEGIFDPENIKEKVYALNGGGELFFRCASLNYDKPTHPKNVPIKNKTYEFRTDNAKKETSTFEYDLIKDKRYTKDQYTLHCPVTLNFKERGIERINDLVRQSLRESDDNYVIGIARGERNLIYISVIDGKGKIVEQFSMNNLSSGNDVSIDFHKMLETRERERDASRKNWNTIDNIKDLKQGYLSYVVKKICDLVVKYDAIVAMADLNVGFKHGREKFERQVYQKFEKALVDKMSYIVNKNASPHSAGGLFRAYQLTNKKYNENEKQNGFIFYVRAWNTSKIDPTTGFVNMLPLKYQSKEKSKEFFDKFEDIFYDENKDMFGFTFRYDDFGINIDHKNEWTAYSNGERIITVRNSFGKWDKAKIALTPAFKKLFDDYNVDCRGDVKRQIMNVDDKDFFVRLYKLLSYTMQLRNSDDADDYILSPVVNAEGMFFDSRNSDGSLPCDADANGAYHIAKKAMWAIGKIKEADEESFKKTSLAIDNKTWLEFVQKAX

SEQ ID NO: 44 - protein, 1293 aa, synthetic construct
  REGION 1..1293: note = EpiCas045
  SITE 1293: note = misc_feature - Xaa =
MVSNNENTPTYNSLTNLYSVSKTLRFELKPQYSTLDHIRDDQIVDKGEDLKNHYKTFKKILDQVFSRIINDSLDKTYLDQKYISTYQDLAFKHRDQLTEKDRAELKTLKETLKKQIDKSLDHKDKKAIFSDPVKFLLDNESEFADLIGDNRPSIEAFNRQKGYLSGYLQNRANIFDRTTNETSVAFRIVEENLAIFLNNRITLQHFLEKVTDKDGLLKSLKEALSQLGFKLKLEDLLSLDYFNRTLSQSGIDQYNLLISGKTLENGTKLQGINEILNQYLQQHQEEKLHKIKLKQLYKQILSESKTESFTLDFVEDNKGLAAMLLQFIDFANQLIEEKMPLLGMIQELKNSSVSVEFLSRLHLNRKNIKRLSNFIYKDYGYIEQSLEENFLSTIEGKITKKVLEEHHKQDTFTFHEILVALQKQQYEKNGTLESADQLLLPGIVNFIYQNLDCECSTLLEKARSEKQPLLDLFKEKQLLEDQNTESHASKYSDRPFNDHEIKTIKTTLDFYKNLQSNLAIFRISDENLKLDSEFYSEFDEFYQGLKNIIPVYNKSRNFLTKKPFSTEKTKLIFNSPQLLDGWSKSKESDCLGTIFIKDGKYYIGIINSVTNVKKTLFEPHNFANIDQSQYFEKMNLFFLSDLKRDFPKKYFSEKWHSQYPIPADLRKKYDYYRIDEHKDERKNDLEYHHQLIAYYQDCLKKDTEWQIYQFKYKSPEEYSDVNEFLSELTPSTYKMEFTKIPAEYIKKLVDDGKLYFFQIYSKDFSEFAKGKPNLHTLYLKAVFDQKNAEEFNYNYKISGSAEIFYRPASIEVRVTHPKNQPIKNKNKNNPKTESVFQYDLYKDRRYMSDKFFLHLPVELNRTPLLPNDSSVNSMVNQVVSSRNQNYFLGIARGERHLIYLVLIDQNGKIIKQQTLNQITSSYQEKSNNQTVEVVTDYHDLLDDKEKLRKKNLQEWQSVENIKELKAGYLSNVVNEIGKIIAEYQPVIMLANLNTGFKNSRIKIEKQVYQKFEKALIDKFNYFMRKDIDPSTIGGLYHALQLTKEYSKQYNGKQNGIIYYIPASYTSNIDPTTGFISAFVQTRYENVEKAKALIEKFNDITYDADESLFCFTADYKKFGPEAKLWQQNVWQIYTNGDRIYTFRDKEEWQSKSYILVEEFKDLFTKYQINYHNDLKTQILSQTDAGFFKQFLFLLRLTLQMRNSRTTDSNEADIDTKKRENDYIISPVKNQYGKFYDSRQDYMEWPENADANGAYNIARKGLIMLKHLKEGLPEKRICDISTEEWVQFVEELNKX

SEQ ID NO: 45 - protein, 1293 aa, synthetic construct
  REGION 1..1293: note = EpiCas046
  SITE 1293: note = misc_feature - Xaa =
MVSEKENTPTFNSLTNLYSVSKTLRFELRPQYSTLDHIKDDQIVDKGEELKNHYKTFKKILDQVFSRIINDSLDKTYLDQKYISTYQDLVFKHRDQLTDKDRAELKALKETLKKQIDKSLDHKDKKAIFSDPVKFLIDNESDFADLIGDNRPSIEAFNRQKGYLSGYLQNRANIFDHTTNETSVAFRIVEENLAIFLNNRLTLQHFLEKVADKDGLLKSLQETLSQLGFKLKLEDLLSLDYFNRTLSQPGIDQYNLLISGKALEDGKKMQGINEILNQYLQQHQEEKLHKIKLKQLYKQILSESKTESFTLDFVEDNKGLAAMLLQFIDFVNKLIEEKMPLLDMIQGLKDSSVSSEFLSRLYFERKNIKRLSNFIYKDYGYIEQSLEENFLSTIEGKITKKALEEHRKQDTFTIHEILVALQKQQYEKDGTLESADHLLLPGVVDFLYQNLDCKHSTLLEKVGSEKQPLLDLFNEKQLLEGQDAESHASKYSDRPFNDHEIKVVKTALDFYKNLQSNFAIFQITDENLKLDSEFYSEFDEFYQGLKNIIPVYNKSRNFLTKKPFSTEKTKLIFNNPQLLDGWSKSKESDCLSTIFIKDGKYYVGIINSATNAKKILFEPYNFANLDQNQYFEKMNLFFLSDLKRDFPKKYFSEKWHNQHPVPADLREKYDYYRIDEHKDERKNDLKYHHQLIAYYQDCLKKDTEWQIYQFKYKAPEEYSDVNEFLSELTPNTYKMEFTKIPAEYIKKLVDDGKLYFFQIYSKDFSEFAKGKPNLHTLYLKAVFDQRNAEEFNYNYKISGSAEIFYRPASIETRVTHPKNQPIKNKNKNNPKAESVFQYDLCKDRRYMSDKFFLHLPIELNRIPLLANDSSVNSMVNQVVSSRNQNYFLGIARGERHLIYLVLIDQNGRIIKQQTLNQITSSYQEKANNQTVEVITDYHDLLNDKEKLRKKNLQEWQSVENIKELKAGYLSNVVNEIGKIIVEYQPVIMLANLNTGFKNSRIKIEKQVYQKFEKALIDKFNYFMRKDLDSSAIGGLYHALQLTKEYSKQYNGKQNGIIYYIPASYTSNIDPTTGFISAFIQTRYENVEKTKSLIEKFNDITYDAEESLFCFSADYKKFSPEAKLWQQTIWQIYTNGDRIYTFKNKEEWQSKSYILVEEFKDLFAKYHIDYCRDLKAQILSQTDASFFKQFLFLLRLTLQMRNSRTTELNGTDADTKKRENDYIISPVKNQYGKFYDSRKDYVDWPENADANGAYNIARKGLIMLKHLKEGLPEKRICDISTEEWVQFVEELNKX

SEQ ID NO: 46 - protein, 1295 aa, synthetic construct
  REGION 1..1295: note = EpiCas048
  SITE 1295: note = misc_feature - Xaa =
MKSIYENFIGLESKNLTLRFALNPEAKTQENLKLYWDKLRDEERDRAYPIVKKILDKEYQQLISEGLKLLENQNVLDWTELAEYIRTSDLSKKKKEDKRLRKLIAQNLKAHPLVDKLKVKNAFGKNGYLETLPLGKEEKEAVKVFAGFGGFFNNYNKNRENYFSTEEKSTAIANRIVNENFSKHFSNVEIVTKIQKEVPELIQIVEAQFKGYDAIFTVNGYNMALSQAGIDTYNEMVAIWNKEANLYAQKAGKLPDGHPLKKKRNYLLSALFKQIGSEKEHLIQIDRFDGDEEVIEALTGVKKMLQEADVFEKLNMLVEDMENWDYSKIYLSAQSLSNVSVFLNNLYEDERENSWNYLDNVLREKWQIELQGKKKGTDLEEAIRKKKQSFYSIEELQEAVNAIEETDKCYNVSKWLLGAMKSERVIEEKKKDVEDFCTQWKNERNSLKETDITALKEYLEQWIFLARYCKSFYANGIEKKEKDEAFYHILEDVLYVLDEVIYFYNKVRNYVTKKPYSLEKMHLKFGHNELANGWSVNKEGNYGTAILRRNGKYYLAITNSLNKKMSIPTQLESTGNNYEKMVLNVFPNVFRMIPKCTTGRNDVKSCFERKEPNEYFFIDTPEFVNPFKVTREEYELNKITYDGVKKWQSDYSKNTQDEKGYKEAVTKWIQFCMRFLQSYKSTAIYDYSTLQQPEKYETVDSFYHDVEKILYECHFEYVPANKIEQLEEEGRIFLFQIYNKDFSENRRPDSKKNLHTLYWEALFSEENRKAKVIQLNGKAEIFRREKSIEHPIVHKAGEVLVNKRTKDGEPIPDDIYKDLSNYFNGRNVTSEKEEYKECLDKVYTSTKKYDITKDKRFTETKYEFHVPITLNYQADGVKYLNQKILHVLRDNPDVNIIGLARGERNLISYVVLNREGKIVNNQQGSFNIVGKMDYQKKLYQKEKNRDKERKTWKNIETIKDLKEGYISQVVHELTDMAIRNNAIIVMADLNFGFKRGRTKVERQVYQKFELALLKKLHYLVTDKTEGEAMLKPGGVLQGYQLAREVKTLKEIGKQCGCVFYVPPGYTSKIDPTTGFVDVFNMSGVTNREKKKAFFEKFDNMFYDEKRDMFGFSFNYEKFTTYQSSYRNDWTVYSNGSKYVWNSLKRTDELIDVTKELKLLFEKYAIDYRNEALFEQIMSQDTDKNNADFWNKLFWYFRVLLRLRNSSDELDQIVSPVLNQNGEFFETPKKITEKSYLSDYPMDADTNGAYHIALKGVYLIQEKIADESVDLDNKLPKDFYKISNAEWFMFRQKEKX

SEQ ID NO: 47 - protein, 882 aa, synthetic construct
  REGION 1..882: note = EpiCas049
MEKFPRCSHLKVKQHCGPFVEWYEDLQSDRQKYVSLFFPWIGIGYGERKDEGDDIDFISPEQTLERRKAELGKLEELVVRFVTVMLKGGSSASSCYSLFYEDYKGKDTAKKSTSKVNFIKALPLLSKKEIEDRVLGDNQLSLINLDEWMELGQSGLSADDIWDKVSQRLVTGERSLGVDVRHTLKIRCQRPRDRGYCVVLMEMVARQLRSCYECYKNHLNELQELREKTTKQITESRDDLFSLVCDLATVLTEQDSGLSERTLFSGRKQALKPQGKPSKIQAIVDELRQPQYSPLLEADDKELRQAYKAWNSQRRLRDRETRRPYPCRPNWRNDYQVSLGLTGRGGFWMWMDGSDVVVDLQDCGRLTCSPSHYFGDLAIEGQLHQYDIRYRNKLKRRGKKLRKPPAYGEWIEATIKEIGIQRKGGDYYVYLLPVISHDSTNFQAAKKFFAAAAPKQEIIDALPDEMKVLALDLNISNPVCSVKARIGRALDGPLSVLDYGQGEIVDGPKILVTDGPRCVALIELHSDVFFVKDAIREYKRTHGVAFNGAGMDDEMLERLSSIPSPSPSVRCQIQAWVAAIGKRLHLLHYGMRREGYKNLGEAIRLLAAMDAYDSMLQSYQRIHLKKGQSLPRQAKNDHSRAGLRETITRRIAYAIAQEARDCNVVFVEDLKADFDADNDNNALLRLFAVKTLIRYIQEALEKIGVGLVLVAKDGTSKTNPMNGDLGWRDRNNKEHLYFELNGEAVRCHADLVASLNVLLRGLDHSVCPYSFVTKDTNKKPGRADQKDKGYGKRLKRFFKDRFGSSNLRFVAKPDGEVTATTRRPKDALIGERVYYHGGKLVTSEVHYRMENEIKHLLTLKSPAKELSLTEDGIRSYENFTHV

SEQ ID NO: 48 - protein, 831 aa, synthetic construct
  REGION 1..831: note = EpiCas050
MVTPESQSDAKKAFADALFAGQEAAYGSFYAKYTPLPFPRKDSALGRLTAELGTIGDEKYAKALKLNGLDPDEWAGYRNRAIAGEPPDALWEEIKVKVGVTNKATLASRGVGNLPTLRPDSKSYATALAYMLSSSLSSWEECAKLHRARREEIAAKAAVPDSMTEEYALVCQLAQALEEAGSGLTAKMLNGAIREMAKTDSVYMVAITELADPKYKPLLALDKEDRARLMDTWQAERKLSTSLAAPKRPLFDKDYQIPFGMTGRGESFALRTDDSGRLWVKIGDHEEFSCAASDYFGNLKVEALPSDKGYKITYRKMVKNRRRQRAGYKSSVGGPLIEGEVKQILLQRRMNRRGKESFYVYLPHSIAVKDDRRHLSWFFKRADWKDGKGLEELPDQLIVSGIDLNIDQPVTVTKAIVSKNYTEGEINCPYGGGHLTGKPRSVCPDTPISQEAKLTHRKMRLLIEVIRESKACHKAGTPLSSEGSERLKILYADISKPPCRNNRESIQVVYSSLKKTYRRLKYELMQQGANDVSGCIRMLQLDDTHRALTACFDAFSGKPALAGRNFGVARKKTSKGTARLNFREHVSHLYANAVLRACHGSDVVFIEDLSTSFDGNAHNSLKRLFAPGQLIDAITSLLESHGIAVVTVDPSGTSRRHPITGDIWYRDSMKKRELVGLIDGELVSVNDDLAASINVLTKGLNHSVVPHKFKVDPSGRVNVKEDGGKRLKVFLREKGLSGRLPVGSADAAKSKKAKALTVYPSSSGLLSDRQVFEVLEQIKHLLAAGCKPRPVELMAGPGETYAAFSLKEVLEWSKSKSSEDLRHTGLGDETG

SEQ ID NO: 49 - protein, 865 aa, synthetic construct
  REGION 1..865: note = EpiCas051
MSNIKTTNILIPKQQDNYFEIENMLDRQNKIANDVFKLLLTYQGHILDQHFFGEDSKEINFIQKRQELYLVAKQADPLVTEDVFNLTCDGFVNQIASKSNMSNDLFKAFEVAYEELSEMKSYVAGKSEAKKLACKLKQWGVLPSFDNHIGEIKSGLSNAFGRFKSWYECDKMTQENFQKHVDSKSAYLEEMGDVISDRFQEFANELGNVYNSKGLDNFDYFGGKFLLFYEQILKPSFEKGEVCYSGSIEFSNGKKQQYSIYGGIIDLLFKYKELWETKSWSKKVKRKIETVEQCTFSRFYNIFEDFKYLRKNKQRAGFREFSSTSSASICLSNSNIIKYDITQVDGDRNNFYLTINGKQIQCRYRTKKIKYNKTTVEKTVENKCYLDNLEIEKQIKNDKPTGNYIFKFDVNKKRSNIATVNEPKIFKNRKGIYISLCMNIDLDDGKYDENKNIAFYLKTKYFNTYTKEADTLPLLKNKTVRIMGVDTGIKPIYTYSILDYKNGKITDPNIHGKLEGKYEFTNYFNMKSLKNVIRDLPKYFQTDDHKELFKSHLFNDLTFTRDELFDELKNFNTLREYKSRKNKGCLIRREIKSYRHKIGRMKDTNFKSDVKDITNVFGIVKYIDSYKQVCSSWNYIGETVETKTQPNFAFADSHLAKYRENLKDNMIKTLVFNIIDEAKKHDVDILAIEDFSSEYSTSTKRDNVLKALFAPSQIQSEIERCAKKEGIALMTVTRHYTSQVVFGKDIFGYRPKENDKTKLKWIENGEIKFVDADINAAKNIAAKLALKDVSPYTLDIEGDGKYFKSSKWDKSKVFKKVNDKFVNVSDQKPKNTKTKMKIFLNGDNYITKEKKNELVEEIKNYKIKT

SEQ ID NO: 50 - protein, 900 aa, synthetic construct
  REGION 1..900: note = EpiCas052
MKSIKSIKSIKTKVVKNNELKLIELSTWCSSICEQLERYIFILGGKQIHDRDGVVVLDGAVERKIYCKKDKSLIAACEVVYKHFTDKSSKSRTFGSWFLGGKSEGDNTNKGRKSTKEKTEKQIAKQIADKKELTDSLQLLWDKKLLPFPIDNKGYDFINTPRAKSYKWAITKTIHAKIKSYNEQCVETKKEYDALNAEINTYKTILFSGYSEKDIDDLQKFVDICEANNHRINYKFISFLKRKDLNFDEQTGKYRKEGKWIQHKNGKEVKSKYSMKDEIVEALYKYKSLTKNDVSVLCNEHQKEDEMGKVVHYNMKRYSDLLFRKKNKKEIPSYTKISLATSKIELGLNNVKYNVEQVEDKLIWTICDQTGKDIQFVTVYTRKKEDNRTNGKKGAGFYKGKHHQLEDLKIVPVGDIGTYDISFKVNGKRPFTGTLKEPNIICRGGKVFVQMPININIDKTLNDARKKVLYAYRETYSGSVNGKKQKMIKIENSKIAESLKSLGRDAIVLGVDLGLRGLATAVVSHNGKNETVKSSQYIKGDIVEWEKYRVFNDNIREVKKYIFLTKKSYTATTEEYTEFYKECSKPEQDYLDSLKTYKDKNVKLNELKYTKNAWSVSKMFEDVSKMFETLKQDRLKYYDIFNMPYWAASLKNYMSLMKSYNYVGVDIKVSKEYMSKYQSLYNNIKEDYAKKIGSYIVQLAVAKNCDIIVLEELKSNLGSVDRKSKRDNEMSLMWNCGRIKTHVENMAKDYGMFIDEVPEYGTSQVYHKTGNYGYRDEDNREIFWYEDNKDVAYIHADENAAINIAKRFLSQHTDNSSFSVILKGDAYYLNIASNSKRMRAAALKTFGDLNKPFKINANDKNGNLYKKTRIFKSDSRWIGVNDKDLYIEHIKSLRNLRVRQ

SEQ ID NO: 51 - protein, 903 aa, synthetic construct
  REGION 1..903: note = EpiCas053
MNHFTQNLAVTKIDSSVQTLYDDFQEDFRKWYSILCSWAKVPYRVEDDNGNITHVHAKQRAAELSSLYSAQEQLLIERFMRVFLGASKEASSSYSLFYDKYAPNGAKKTAALKEFLGEIPTLDDSQVEKKANTNKNCKRITVKEWRDFAAQFNKLGIDAIWGKLKEKITSPDRGVGLQVRGFVSERCKHPENAGYCRQLCQKLTEQVKSTVRICELYIQETADLQSEIGNKTKQPEVKKCFDLLCQLSDELRDVNSGLSGRVLFQSIKDIQGGKDSDRKNKVCRTVMSDDKYLCLIDSDKKIVQRAFQAWKLSITLKKRQEKLYPKQRSHQNDVPMPFGLTGLASFDVSPDGSKFTFSEGSVETKPSLYFDGLRFQKNKHSFDMEYRVAYASRRTKKGRRPKRVGRLRKATLKQVELFNKGGKFVIKLPHGIELPEHRAKLATFLMCADPKEKGYSKGGLVDEFRALAIDVNLSNPLAACVADVSKHGDGPIQALDYGRAKLCVDPFFLVANTPVCGQLIKLCKECKAVVQAIKEFKECQAAGSDFSFETDLFLPAGHSPRHRIQSKVQELSRVLRDWKFKLQNTNQVAEMIRLLELMDAYQSMISSYQRIHLKAGQTLPPQKKNSTKRANYRKDISRRLAFVVADYAQSLNVDVVFGEDLKADFDRDKNTNSLSRLFAGGMFLQHLENALAIRGIAFVKCAKNGTSITDPVSGVFGWRDKFNKERLWIERDGELGWVNSDHAACLNVLLVGLMHSVVPYRVYVKAGRKTTDDVEVFEEDHPIGPRKKRFFELCFGENKPKFEVVENRVILDNAGTYQGFIYAHCLDAMQSEKQHWAEYDRIKELALAETNPKQFGLTPKKGEGYRNFCQPDIHEQVEVVGNKRVAATKQILESLADEKIEAT

SEQ ID NO: 52 - protein, 737 aa, synthetic construct
  REGION 1..737: note = EpiCas054
MSQEGEVKFKSNSDMKDRGVVTGYDYSLINAFCSKYTNLWEERDDYDSTYLDKGGRKRQACIMTDRYYISHMIKRLKYMTKKHVNVPLFEQGKKAPCQLFGKNYMSYTLRQDEETGTFEFSFTDPTSESEGRAVKKFNASLAKNGYLNNLKIVESSNKDGVYKVSFNTAVENKDTLTIQTTYTGYIKEPRIRFNLEKNVTYLDLCISGIESDNDTFNKILSEEQKENKEAIFKGFSSYFKASYAKGRDGSQKGSLDVDVFRAMGVDLGLNPLAALSIYEVKKSDKGEDIGGQKVKIKHLTDHKSSDINKANKDCRVKKAKRTLKFIEGVKGLISVANHHCNYLEDVEATGEGKEVNVGYMEMLCGDVIENHTPFKDLEDYMKYIENNLYGVDRKEWKKKTSDWVVPSLIQQAKKKISEMRREYFDAEDKHYHTTKVNHVCNLQLHKIQAVKEMISTLNSFSTLGLNDEEKQAHADNGRPCADLWEYINGLRNYLSKGIASIIINHALRNSVNIIFIEDLDMKASSFDSKEENKLKSLWSASQIMDYLEKFAAKHTIAVQEVNKFMTSQFSSENGTLGVRGASGNKSQFLYEDKGEVCDVDSDINAARNIAIRGITRHSNMPMFKVKVASDKEFILEMPKAAGMQKLSSMMKYLDSDNPRYVKFVKANNGTLKASVLEKEEFNKLKKQAIAWKKDNKDADSEVSILRSGKHFYIRKELEAIVKAKLCPEVEEETVKAK

SEQ ID NO: 53 - protein, 972 aa, synthetic construct
  REGION 1..972: note = EpiCas055
MATRTSHKSSKIRILPTGTTKKALVEYNLLFHDQVAKIMLDLLTMRGVPYVLRDKDGEHEITATQIREAQWKLINSGRDSGDCIRLSQSIIDMMAQIYGGIMETGNPTKYRANLYLKKTNSGNEIGQGRSSASFMLFKDVSRGLSRPEFTRQIKDKNGKIKKPFAWATEERLMELYDAVRNDEMQPIEVEAERKSLEPDVTMENLVKLRKVGILPLPLPGGHLYQGRGLGKLLAMPFDAAVGRLKSHYQANLAAVEARAALDKVVADKKDNVPAPLYALFLEFAEECRQNGFGVSKRFAKKLHGLNIPKTDFEPGDPFIVGLEIIKQYKYRPLWPQIGTLAGVYLAGVKAEKTKGYAAITIADAYRSPALIRFGITNYARFEAEVNDQQGIDFSLQIPVDDQWTTVTVSGMPSNYFQNPELIRQTSNYALSFTKGNRQQRRMGVILKEPLLTVRYSSDPEQEPRFYVHLAYNYDKTSYRMIGLDKIRAFFSSNLSKGAKLPHGTPYGLRTLSIDLGIRPIISSHLMELVSPHDIEAAQESRNGIEPIEVPDMGFARLVDSREMGGVWNSGLVGRMIDASRRCKSARHMILVSKLMRDGKPLNTHQQFLIEKYVKMYGVFLPPDDWARKDIIGEFIRQILADYRVIKDTMAKRNHPDHKGKFPDIICSDVFRMLFLIKDVISMLKSWARYKRKTGDKEIQGQNPTELNQYWRYYNNLKDDLLKKIVHSLVRYADEHGVHLLLLEDITGNRDSTKHRKENSMFAIWSPTLIRTRLEEEFEACGMLVQAINPSFTSQTHYMTGEFGFRDPRQKECLYFKREGRLYLIDSDGNSSMGLQVRFWTRHRDLWTLKTVKARRDRAAKLLKLDPKRAECTFVAKPTFEYAKSYLKRNLASPVAAFVPDDNGNFILHKLGVNAANQLTEGQERGETFFRHGTDWITHASHKKRMSAIEAMVEKVKKKGDKMTEADLVRLKV

SEQ ID NO: 54 - protein, 1007 aa, synthetic construct
  REGION 1..1007: note = EpiCas056
MSSDVVRPYNTKLLPDNRKHNMVVDTMNWCDNACSVFFDLFVGLYGGVKIGDVTNFLTEKQDTTTDADLLCAINWFRAMPVSNPDAVVGPEQLVVRFRDYSGHNPSPMASMYLSAPVNPRYTWVDCRFLYQQMCQTLGANLDVDISTLVQTGLLPIQKDTQLNAYSFCSNVFGEGVKEDPSAKVTSYTAAANALSGATNPIITYEDYRQILSSAITNRPSRKGAKDILAADLDSTKTGVLPGNYVSQRIAMYQASAASKARGVVLPNRLRVKAYLQNLVGLNYICTTWAAPMLRAVGDIKSKNSNNYRFVGERLERQQEIDNLLAVSNIRSAQAILQQFRANESNQFYIKKRHIGKGLPSLYDMWDLMDEKEGIDNYIQSLKGDKTERLPIRELLQIIYPHRKSVSAELFLSAAELTDVEDRQNRCMVHPTVRGSLVINFGKSSTIFGAITPPDTLIKFRGEMVPAGQTGMIWFTMHLVDGGKWVKHHIPCHSSRYFEEIYAWKKDLPTLPFPRRSLYGYAIGNKISDTRKIDLRRKKASKQYLRTLENMTHNVEFDPTTQFMVDQELNVTITARVKKIPPVRDVPVGSRIMGLNKNQTIRDCYSIWERVEANTSGSFQHPVVQDVWLRLVADGHVTSTVNGPNGQIDQMSYSGPDVANCGNWMQERSNFITSVDDADQSIMKHFLWNNRVKLYAWNCVYAGTLMKAISKQMTTANRNLFRNEILSFVGGRFGCRLGSLAQVSLDLLRRMKSVISCYFSRNNAFTIEERSAFDKELMELFESLDNKMNNKRKEKVNRTLSSIFQVAKQHNVVRLVVTKNLQTPDANVRSVMNQRSVDWCARKIEEKIVDLGNVIGIYVDLVEALDLSHLDPFIYIAKGDVGKECQFDEVESSSLLPIHTSMFRDWHGLVNKGRTTTPIYHSALRSFASHYGLRFDDLARIKAAELAKMLPDQKVFIPHRGGRFFMSTYPVTSTSRPVSYDGRQRFLNSGDMVAPVNTMLRGFRRARS

SEQ ID NO: 55 - protein, 1011 aa, synthetic construct
  REGION 1..1011: note = EpiCas057
MGITMSDTTFRPYKSKLNPNERKMPMVVDTMNWCDNACSVFFDLFVGLYGGVKIGDVTNFLTEKQDTTTDADLLCAINWFRAMPVSNPDAVVGPEQLVVRFRDYSGHNPSPMASMYLSAPVNPRYTWVDCRFLYQQMCQTLGANLDVDISTLVQTGLLPIQKDTQLNAYSFCSNVFGEGVKEDPSAKVTSYTAAANALSGATNPIITYEDYRQILSSAITNRPSRKGAKDILAADLDSTKTGVLPGNYVSQRIAMYQASAASKARGVVLPNRLRVKAYLQNLVGLNYICTTWAAPMLRAVGDIKSKNSNNYRFVGERLERQQEIDNLLAVSNIRSAQAILQQFRANESNQFYIKKRHIGKGLPSLYDMWDLMDEKEGIDNYIQSLKGDKTERLPIRELLQIIYPHRKSVSAELFLSAAELTDVEDRQNRCMVHPTVRGSLVINFGKSSTIFGAITPPDTLIKFRGEMVPAGQTGMIWFTMHLVDGGKWVKHHIPCHSSRYFEEIYAWKKDLPTLPFPRRSLYGYAIGNKISDTRKIDLRRKKASKQYLRTLENMTHNVEFDPTTQFMVDQELNVTITARVKKIPPVRDVPVGSRIMGLNKNQTIRDCYSIWERVEANTSGSFQHPVVQDVWLRLVADGHVTSTVNGPNGQIDQMSYSGPDVANCGNWMQERSNFITSVDDADQSIMKHFLWNNRVKLYAWNCVYAGTLMKAISKQMTTANRNLFRNEILSFVGGRFGCRLGSLAQVSLDLLRRMKSVISCYFSRNNAFTIEERSAFDKELMELFESLDNKMNNKRKEKVNRTLSSIFQVAKQHNVVRLVVTKNLQTPDANVRSVMNQRSVDWCARKIEEKIVDLGNVIGIYVDLVEALDLSHLDPFIYIAKGDVGKECQFDEVESSSLLPIHTSMFRDWHGLVNKGRTTTPIYHSALRSFASHYGLRFDDLARIKAAELAKMLPDQKVFIPHRGGRFFMSTYPVTSTSRPVSYDGRQRFLNSGDMVAPVNTMLRGFRRARS

SEQ ID NO: 56 - protein, 754 aa, synthetic construct
  REGION 1..754: note = EpiCas058
  SITE 754: note = misc_feature - Xaa =
MARNNKKLEGLVKSYKFQAKNVDIMIDILEEYSEYYNRVSNWINDNLMTLTIGDIALKCNTSQSVGYMQIALSDDYKQLPMYKLFEKKYPSTHCLNLLYAYITNNNIDNYTGNIWGLSTTNYRKYGYINLVINNYRSKFANLNFNVKRSKIDINSNVEEIEKQCLYERIRLGLIKIEDWKKHIDSLKRQEIINEKALHRFNILSDYFNKNGESINERQSLLTIEQLQKFNGCQMKNKSMRIQVQNFKLNEKPNSLGYILQIHLNKKLFNIELLGNRQIRKGNKDNYTTLVDIINNHGIDIIFKLENNKLYVILTSTDTTFNKTITTPNKICGIDINIKHALLNTSERDSMNIQGYVNLYKRVLENDNFVSLLSKEEYETFSNMASYLTFCPIEFNYLYSRISNDEYTEKERLFSKILIDIQKEYENKKGCDLEKNYIHSVNKLRAKIIAYHKLKTIYTQKKQEYDIKMGFVDDSTLSKDGMDKRRFESPFNNTDCAKQIKSKLDNVLQDIEGCRKNIITYVYKIFETNGYVTIGLENLDNSNFEYHKPLCSIKSLLNYHKLLNKTIEQVKENNSVADLIEKDYYIFTFDENKNIIDAKFSDKGFYKINKSWFINQLIKVLHFASIKNYFITLSNNGKTQIVLVPSEFTSQINSLTHKLPMIKNDKGENVRPTKFRVRKTQEKHYNGLNADINATLNIKYIVENEEWRNVLCKSPNKKEYKDARGYNFPTLIATQKHYNVSKQLEKLGGIEFIQX

SEQ ID NO: 57 - protein, 911 aa, synthetic construct
  REGION 1..911: note = EpiCas059
MEETRTPEKIACQQDRSAFFKLGKLPQKTTSAIYHLMRCSKRYIDNVSETISNNIEKAAMTSDNHIFRSALKEEYKKIYREKFYPDVTGQPFPDKGPDNTHIVERTVENLCGQYISALKGVMKVRKPKWQDDIFEDESDKVIAEMLMASGNEADIHPKLEKKIASAKKKDKMDEWQKVLDRYDYIKSKTDIEWTYTTLLYDHIARECARSMFEDGNKPKFCYTNGNKFAKQVVDELWGSERVEYEYEKYLHCRTLEAYWNEENKYFFLENQKKSKKTYEARQIIDHFIENEDAVKAETEEYMAKVAKEFGENGGCKFRTENILYLVNSVSINKKQDEERCPIFKVTDIPQYAEAGIDRIGECKYVIKLKLFTVGERYGTTYMPEAFSGLYDRRTNQRYDLIDRACKGSYVYLPIYISDKDSRKWSDRLKNTFTMSAFSISERKTKKDGRVLCVNLPYTHIQHKPRNYFKVYPTYGVDINVKHSLFSTNATNLNGYIDVNGELIDFYNSIGRPDKLKNINLAVTLGDKGGTAGNHTNFLLVSDLGDWDDHGKKRNDRFVKREDGTYYSRPDLLADGLNFLKKKYSGDRKSYDYINTTIAFRNNQTRLRCIDKEWNDRKRAYDEEHGKPEKGERSGFYPTEDAERLTMERQALRREIAENTRQVIAYMLWLFQENGIKSIALEHLDCGSWKNFRDQLKPKWFCNNCKYWAEKYGIPYEATKYYRSNRKYFDIEDGELIPENVKLNALGEAENDKRYFQTSIAKAVGMSSIKQMFSIVSQNYDIQVNYTEQAYTSQTDSRNGTVDKDFRVSQECYIGSDGTKMNCDFNAAVNIADRISDDTLREEFNKELPMKEFVKYGATQIVSRNRRWNAENAERVTMAAFQKRKNADGGAHTAAVKPTSKTEESSLKLVAE

SEQ ID NO: 58 - protein, 913 aa, synthetic construct
  REGION 1..913: note = EpiCas060
  SITE 913: note = misc_feature - Xaa =
MIDRNETHLSKKSTRSVEFKLAVPNRIAPVIDEMLDLSITMSNAISKDISEHLTDWVQRAEVTKEQKRPYDYLYASEKEGIRYWYKHSGLRDKMYFDFCSKYFGYPVLKNKNAHFLTRTIENVAAAYEGRFTRFQEETKIRATDQSQLTEEEELLKKNIKEILNIMCSLKPGQTVDQILVRRSKTGKNQEKYQKLLSFYVDVTSDEKSDKYINFDILFADMCYRNSATFILKTMEISVDDSGVVNFGMVSPLVELPTKIGSSEEATMRHILENRSVRLINEVNDMIFELTVAQYIKSSCRYRFVDELTEKANSKDSVFHKNLLMYYTSHRDKVDEGYKQYLHSVNESFGKKQIVWKNSTLKLNYEEKVEKDRQVPIKMISSIKQFADLGITSISGCKYVLRVHMILDDEKKFKDQHLFCDLYDKRTGRRFDLLDHETKGYAYIPIMVPENDRRTYDISDFDCQMTEISSRDGMYFAKLTRDIDYVKPVNRFGEEQVCGVDINIRHAMIDVSERSIMNSEKYVDVEGFIIDYFRNVKNLPSVADDLVTNRYLGEAEEAGKHTFFGLMSSINKSISRETGGLKNRFVKNVDGTYTILPDCFSEPLNVLMKKYEQGSLQYRYVASVKALRVQLAQMHVLCMEHDDRRQVYDNLYGKPYIDDHPYEDPDFVYAHRKLHQKIETNTQFIVSYAIQLIQEAGFSCISVEQIDKKNLGKMLNLKSAKVFYNGCIYASSENGQAIADTRYFRTNCRYFDYPSDLNLFDIDHIKLNGVGEAYNINAKLMNSLGKYVGFASFKHMFAHIGTAHDVQVVFVEPAFTSQVDSKTGELRADKKEMRPYHHTYKHTDGTVSHADENGAINAKKIVTEEILRTRLLKENSVKDIMEYGGVQLERSGKSINGVRKVYEEVYAEKNGLVX

SEQ ID NO: 59 - DNA, 22 bp, synthetic construct
  misc_feature 1..22: note = sgRNA target-1
  source 1..22: mol_type = other DNA
caagtcccctcatccccacaga

SEQ ID NO: 60 - DNA, 20 bp, synthetic construct
  misc_feature 1..20: note = sgRNA target-2/Example5 spacer/Example6 spacer-20nt
  source 1..20: mol_type = other DNA
aagtcccctcatccccacag

SEQ ID NO: 61 - DNA, 1790 bp, synthetic construct
  misc_feature 1..1790: note = Example1 reporter
  misc_feature 939: note = n =
  misc_feature 940: note = n =
  misc_feature 941: note = n =
  misc_feature 942: note = n =
  misc_feature 943: note = n =
  misc_feature 944: note = n =
  misc_feature 967: note = n =
  misc_feature 968: note = n =
  misc_feature 969: note = n =
  misc_feature 970: note = n =
  misc_feature 971: note = n =
  misc_feature 972: note = n =
  source 1..1790: mol_type = other DNA
atgagcgagctgattaaggagaacatgcacatgaagctgtacatggagggcaccgtggacaaccatcacttcaagtgcacatccgagggcgaaggcaagccctacgagggcacccagaccatgagaatcaaggtggtcgagggcggccctctccccttcgccttcgacatcctggctactagcttcctctacggcagcaagaccttcatcaaccacacccagggcatccccgacttcttcaagcagtccttccctgagggcttcacatgggagagagtcaccacatacgaagacgggggcgtgctgaccgctacccaggacaccagcctccaggacggctgcctcatctacaacgtcaagatcagaggggtgaacttcacatccaacggccctgtgatgcagaagaaaacactcggctgggaggccttcaccgagacgctgtaccccgctgacggcggcctggaaggcagaaacgacatggccctgaagctcgtgggcgggagccatctgatcgcaaacatcaagaccacatatagatccaagaaacccgctaagaacctcaagatgcctggcgtctactatgtggactacagactggaaagaatcaaggaggccaacaacgagacctacgtcgagcagcacgaggtggcagtggccagatactgcgacctccctagcaaactggggcacaagcttaatggatccggcgcaacaaacttctctctgctgaaacaagccggagatgtcgaagagaatcctggaccggctgagcaggctcgttgggaagcagcctccaaagaaaccatcaagaaaaccaccaagccctgtccccgctgccatgtaccagtggaaaaaaatggaggctgcatgcacatgaagtgtccgcagccccagtgcaggctcgagtggtgctggaactgtggctgcgagcccccggcnnnnnncaagtcccctcatccccacagannnnnntcgggttaggggaccactggttcgacgtgagcggttctggcgaagggcgaggttccttgctgacctgtggcgatgtagaagaaaatcccggccccggatccgtgagcaagggcgaggagctgttcaccggggtggtgcccatcctggtcgagctggacggcgacgtaaacggccacaagttcagcgtgtccggcgagggcgagggcgatgccacctacggcaagctgaccctgaagttcatctgcaccaccggcaagctgcccgtgccctggcccaccctcgtgaccaccctgacctacggcgtgcagtgcttcagccgctaccccgaccacatgaagcagcacgacttcttcaagtccgccatgcccgaaggctacgtccaggagcgcaccatcttcttcaaggacgacggcaactacaagacccgcgccgaggtgaagttcgagggcgacaccctggtgaaccgcatcgagctgaagggcatcgacttcaaggaggacggcaacatcctggggcacaagctggagtacaactacaacagccacaacgtctatatcatggccgacaagcagaagaacggcatcaaggtgaacttcaagatccgccacaacatcgaggacggcagcgtgcagctcgccgaccactaccagcagaacacccccatcggcgacggccccgtgctgctgcccgacaaccactacctgagcacccagtccgccctgagcaaagaccccaacgagaagcgcgatcacatggtcctgctggagttcgtgaccgccgccgggatcactctcggcatggacgagctgtacaagtaa

SEQ ID NO: 62 - DNA, 2013 bp, synthetic construct
  misc_feature 1..2013: note = Example2 reporter
  source 1..2013: mol_type = other DNA
atgagcgagctgattaaggagaacatgcacatgaagctgtacatggagggcaccgtggacaaccatcacttcaagtgcacatccgagggcgaaggcaagccctacgagggcacccagaccatgagaatcaaggtggtcgagggcggccctctccccttcgccttcgacatcctggctactagcttcctctacggcagcaagaccttcatcaaccacacccagggcatccccgacttcttcaagcagtccttccctgagggcttcacatgggagagagtcaccacatacgaagacgggggcgtgctgaccgctacccaggacaccagcctccaggacggctgcctcatctacaacgtcaagatcagaggggtgaacttcacatccaacggccctgtgatgcagaagaaaacactcggctgggaggccttcaccgagacgctgtaccccgctgacggcggcctggaaggcagaaacgacatggccctgaagctcgtgggcgggagccatctgatcgcaaacatcaagaccacatatagatccaagaaacccgctaagaacctcaagatgcctggcgtctactatgtggactacagactggaaagaatcaaggaggccaacaacgagacctacgtcgagcagcacgaggtggcagtggccagatactgcgacctccctagcaaactggggcacaagcttaatggatccggcgcaacaaacttctctctgctgaaacaagccggagatgtcgaagagaatcctggaccggctgtgagcaagggcgaggagctgttcaccggggtggtgcccatcctggtcgagctggacggcgacgtaaacggccacaagttcagcgtgtccggcgagggcgagggcgatgccacctacggcaagctgaccctgaagttcatctgcaccaccggcaagctgcccgtgccctggcccaccctcgtgaccaccctgacctacggcgtgcagtgcttcagccgctaccccgaccacatgaagcagcacgacttcttcaagtccgccatgcccgaaggctacgtccaggagcgcaccatcttcttcaaggacgacggcaactacaagacccgcgccgaggtgaagttcgagggcgacaccctggtgaaccgcatcgagctgaagggcatcgacttcaaggaggacggcaacatcctggggcacaagctggagtacaactacaacagccacaacgtctatatcatggccgacaagcagaagaacggcatcaaggtgaacttcaagatccgccacaacatcgaggacggcagcgtgcagctcgccgaccactaccagcagaacacccccatcggcgacggccccgtgctgctgcccgacaaccactgataaggatcctttgaagtcccctcatccccacagtggtaggatatcggcaagctgaccctgaagttcatctgcaccaccggcaagctgcccgtgccctggcccaccctcgtgaccaccctgacctacggcgtgcagtgcttcagccgctaccccgaccacatgaagcagcacgacttcttcaagtccgccatgcccgaaggctacgtccaggagcgcaccatcttcttcaaggacgacggcaactacaagacccgcgccgaggtgaagttcgagggcgacaccctggtgaaccgcatcgagctgaagggcatcgacttcaaggaggacggcaacatcctggggcacaagctggagtacaactacaacagccacaacgtctatatcatggccgacaagcagaagaacggcatcaaggtgaacttcaagatccgccacaacatcgaggacggcagcgtgcagctcgccgaccactaccagcagaacacccccatcggcgacggccccgtgctgctgcccgacaaccactacctgagcacccagtccgccctgagcaaagaccccaacgagaagcgcgatcacatggtcctgctggagttcgtgaccgccgccgggatcactctcggcatggacgagctgtacaagtaa

SEQ ID NO: 63 - DNA, 81 bp, synthetic construct
  misc_feature 1..81: note = EpiCas001-DR
  source 1..81: mol_type = other DNA
gttgaataaccttaaggttattcgactaaaatggataaaatgaacaaaaaaattgatttaaagtataattattcaccctat

SEQ ID NO: 64 - DNA, 19 bp, synthetic construct
  misc_feature 1..19: note = EpiCas002-DR
  source 1..19: mol_type = other DNA
aatttctactattgtagat

SEQ ID NO: 65 - DNA, 20 bp, synthetic construct
  misc_feature 1..20: note = EpiCas005-DR
  source 1..20: mol_type = other DNA
taatttctactattgtagat

SEQ ID NO: 66 - DNA, 20 bp, synthetic construct
  misc_feature 1..20: note = EpiCas032/033-DR
  source 1..20: mol_type = other DNA
aatttctactaatgtagata

SEQ ID NO: 67 - DNA, 58 bp, synthetic construct
  misc_feature 1..58: note = EpiCas034-DR(1)
  source 1..58: mol_type = other DNA
aaacaaagtattagaacaatgaaatttccattgttgccttatgatgcggacagtaaga

SEQ ID NO: 68 - DNA, 14 bp, synthetic construct
  misc_feature 1..14: note = EpiCas034-DR(2)
  source 1..14: mol_type = other DNA
acggagagaaaggc

SEQ ID NO: 69 - DNA, 81 bp, synthetic construct
  misc_feature 1..81: note = EpiCas035-DR
  source 1..81: mol_type = other DNA
ttacagaaattatatcctatgtattcacacgcttattgcttaaaaacacaatgtcccgccggggtaaccgcgaatggacac

SEQ ID NO: 70 - DNA, 36 bp, synthetic construct
  misc_feature 1..36: note = EpiCas037-DR
  source 1..36: mol_type = other DNA
atctacaatagtagaaattcttaggttcttataaag

SEQ ID NO: 71 - DNA, 42 bp, synthetic construct
  misc_feature 1..42: note = EpiCas038-DR
  source 1..42: mol_type = other DNA
tagatctacaacagtagaaattagggaagattgcaaaacctt

SEQ ID NO: 72 - DNA, 36 bp, synthetic construct
  misc_feature 1..36: note = EpiCas039-DR
  source 1..36: mol_type = other DNA
gtccaaaactcatttcgaatttctactgatgtagat

SEQ ID NO: 73 - DNA, 36 bp, synthetic construct
  misc_feature 1..36: note = EpiCas040-DR
  source 1..36: mol_type = other DNA
atctacaacagtagaaattataagggagtattaatc

SEQ ID NO: 74 - DNA, 36 bp, synthetic construct
  misc_feature 1..36: note = EpiCas041-DR
  source 1..36: mol_type = other DNA
gtttaggcagcttctctaatttctactgttgtagat

SEQ ID NO: 75 - DNA, 36 bp, synthetic construct
  misc_feature 1..36: note = EpiCas042-DR
  source 1..36: mol_type = other DNA
ctttgaaagaatataatttctactgaaagtgtagat

SEQ ID NO: 76 - DNA, 36 bp, synthetic construct
  misc_feature 1..36: note = EpiCas043/045-DR
  source 1..36: mol_type = other DNA
gtttaataattagaaataatttctactgttgtagat

SEQ ID NO: 77 - DNA, 36 bp, synthetic construct
  misc_feature 1..36: note = EpiCas044-DR
  source 1..36: mol_type = other DNA
gtttataaaccttatttaatttctactgttgtagat

SEQ ID NO: 78 - DNA, 36 bp, synthetic construct
  misc_feature 1..36: note = EpiCas046-DR
  source 1..36: mol_type = other DNA
gtttaacgattagaaataatttctactgttgtagat

SEQ ID NO: 79 - DNA, 36 bp, synthetic construct
  misc_feature 1..36: note = EpiCas047-DR
  source 1..36: mol_type = other DNA
atctacaacagtagaaattatttctaattattaaac

SEQ ID NO: 80 - DNA, 36 bp, synthetic construct
  misc_feature 1..36: note = EpiCas048-DR
  source 1..36: mol_type = other DNA
atctacactttcagtagaaattatattcttccaaag

SEQ ID NO: 81 - DNA, 37 bp, synthetic construct
  misc_feature 1..37: note = EpiCas049/055-DR
  source 1..37: mol_type = other DNA
agtgctggttctcgtcgctaggggagagtcaaagcac

SEQ ID NO: 82 - DNA, 36 bp, synthetic construct
  misc_feature 1..36: note = EpiCas050/053-DR
  source 1..36: mol_type = other DNA
gtgccttggcgatccgccgtagcaggtcgccagcac

SEQ ID NO: 83 - DNA, 36 bp, synthetic construct
  misc_feature 1..36: note = EpiCas051/054-DR
  source 1..36: mol_type = other DNA
gtgtcagaagacttataaaatgagtcttattgtgac

SEQ ID NO: 84 - DNA, 36 bp, synthetic construct
  misc_feature 1..36: note = EpiCas052-DR
  source 1..36: mol_type = other DNA
gtgtcaacgcatcctctatagttgaggaagcaacac

SEQ ID NO: 85 - DNA, 23 bp, synthetic construct
  misc_feature 1..23: note = EpiCas056/057-DR(1)
  source 1..23: mol_type = other DNA
agaaatccgtccttggttgacgg

SEQ ID NO: 86 - DNA, 23 bp, synthetic construct
  misc_feature 1..23: note = EpiCas056/057-DR(2)
  source 1..23: mol_type = other DNA
agaaatccgtcctacgttgacgg

SEQ ID NO: 87 - DNA, 36 bp, synthetic construct
  misc_feature 1..36: note = EpiCas058/059/-DR/Example6 DR-36nt
  source 1..36: mol_type = other DNA
agtggatgcggtatcaacttgattggtactgacacc

SEQ ID NO: 88 - DNA, 36 bp, synthetic construct
  misc_feature 1..36: note = EpiCas060-DR
  source 1..36: mol_type = other DNA
ggtatcactcatcccattatggataggtgaaccatt

SEQ ID NO: 89 - DNA, 23 bp, synthetic construct
  misc_feature 1..23: note = sgRNA target-3
  source 1..23: mol_type = other DNA
cctcactcctgctcggtgaattt

SEQ ID NO: 90 - DNA, 22 bp, synthetic construct
  misc_feature 1..22: note = Example6 DR-22nt
  source 1..22: mol_type = other DNA
caacttgattggtactgacacc

SEQ ID NO: 91 - DNA, 31 bp, synthetic construct
  misc_feature 1..31: note = Example6 DR-31nt
  source 1..31: mol_type = other DNA
atgcggtatcaacttgattggtactgacacc

SEQ ID NO: 92 - DNA, 31 bp, synthetic construct
  misc_feature 1..31: note = Example6 DR-31.1nt
  source 1..31: mol_type = other DNA
atgcggtatcaacttgattggtaccgacacc

SEQ ID NO: 93 - DNA, 31 bp, synthetic construct
  misc_feature 1..31: note = Example6 DR-31.2nt
  source 1..31: mol_type = other DNA
atgcgggatcaacttgattggtcctgacacc

SEQ ID NO: 94 - DNA, 31 bp, synthetic construct
  misc_feature 1..31: note = Example6 DR-31.3nt
  source 1..31: mol_type = other DNA
atgcggtgtcaacttgattggcactgacacc

SEQ ID NO: 95 - DNA, 31 bp, synthetic construct
  misc_feature 1..31: note = Example6 DR-31.4nt
  source 1..31: mol_type = other DNA
atgcggtaccaacttgattggtactgacacc

SEQ ID NO: 96 - DNA, 31 bp, synthetic construct
  misc_feature 1..31: note = Example6 DR-31.5nt
  source 1..31: mol_type = other DNA
atgcggtatcgacttgatcggtactgacacc

SEQ ID NO: 97 - DNA, 31 bp, synthetic construct
  misc_feature 1..31: note = Example6 DR-31.6nt
  source 1..31: mol_type = other DNA
atgcggtatcagcttgactggtactgacacc

SEQ ID NO: 98 - DNA, 30 bp, synthetic construct
  misc_feature 1..30: note = Example6 DR-31.7nt
  source 1..30: mol_type = other DNA
atgcggtatcagcttgactggtactgcacc

SEQ ID NO: 99 - DNA, 31 bp, synthetic construct
  misc_feature 1..31: note = Example6 DR-31.8nt
  source 1..31: mol_type = other DNA
acgcggtatcaacttgattggtactgacgcc

SEQ ID NO: 100 - DNA, 24 bp, synthetic construct
  misc_feature 1..24: note = Example6 Spacer-24nt
  source 1..24: mol_type = other DNA
aagtcccctcatccccacagtggt

SEQ ID NO: 101 - DNA, 23 bp, synthetic construct
  misc_feature 1..23: note = Example6 Spacer-23nt
  source 1..23: mol_type = other DNA
aagtcccctcatccccacagtgg

SEQ ID NO: 102 - DNA, 22 bp, synthetic construct
  misc_feature 1..22: note = Example6 Spacer-22nt
  source 1..22: mol_type = other DNA
aagtcccctcatccccacagtg

SEQ ID NO: 103 - DNA, 21 bp, synthetic construct
  misc_feature 1..21: note = Example6 Spacer-21nt
  source 1..21: mol_type = other DNA
aagtcccctcatccccacagt

SEQ ID NO: 104 - DNA, 19 bp, synthetic construct
  misc_feature 1..19: note = Example6 Spacer-19nt
  source 1..19: mol_type = other DNA
aagtcccctcatccccaca

SEQ ID NO: 105 - DNA, 18 bp, synthetic construct
  misc_feature 1..18: note = Example6 Spacer-18nt
  source 1..18: mol_type = other DNA
aagtcccctcatccccac

SEQ ID NO: 106 - DNA, 17 bp, synthetic construct
  misc_feature 1..17: note = Example6 Spacer-17nt
  source 1..17: mol_type = other DNA
aagtcccctcatcccca

SEQ ID NO: 107 - DNA, 16 bp, synthetic construct
  misc_feature 1..16: note = Example6 Spacer-16nt
  source 1..16: mol_type = other DNA
aagtcccctcatcccc

SEQ ID NO: 108 - DNA, 23 bp, synthetic construct
  misc_feature 1..23: note = Example7 EMX1 Spacer-23nt
  source 1..23: mol_type = other DNA
tggttgcccaccctagtcattgg

SEQ ID NO: 109 - DNA, 23 bp, synthetic construct
  misc_feature 1..23: note = Example7 VEGFA Spacer-23nt
  source 1..23: mol_type = other DNA
ctctcaagacccacaatccaggc

SEQ ID NO: 110 - DNA, 8207 bp, synthetic construct
  misc_feature 1..8207: note = EpiCas002 plamid DNA
  source 1..8207: mol_type = other DNA
tgagcaaaaggccagcaaaaggccaggaaccgtaaaaaggccgcgttgctggcgtttttccataggctccgcccccctgacgagcatcacaaaaatcgacgctcaagtcagaggtggcgaaacccgacaggactataaagataccaggcgtttccccctggaagctccctcgtgcgctctcctgttccgaccctgccgcttaccggatacctgtccgcctttctcccttcgggaagcgtggcgctttctcatagctcacgctgtaggtatctcagttcggtgtaggtcgttcgctccaagctgggctgtgtgcacgaaccccccgttcagcccgaccgctgcgccttatccggtaactatcgtcttgagtccaacccggtaagacacgacttatcgccactggcagcagccactggtaacaggattagcagagcgaggtatgtaggcggtgctacagagttcttgaagtggtggcctaactacggctacactagaagaacagtatttggtatctgcgctctgctgaagccagttaccttcggaaaaagagttggtagctcttgatccggcaaacaaaccaccgctggtagcggtttttttgtttgcaagcagcagattacgcgcagaaaaaaaggatctcaagaagatcctttgatcttttctacggggtctgacgctcagtggaacgaaaactcacgttaagggattttggtcatgagattatcaaaaaggatcttcacctagatccttttaaattaaaaatgaagttttaaatcaatctaaagtatatatgagtaaacttggtctgacagttaccaatgcttaatcagtgaggcacctatctcagcgatctgtctatttcgttcatccatagttgcctgactccccgtcgtgtagataactacgatacgggagggcttaccatctggccccagtgctgcaatgataccgcgagacccacgctcaccggctccagatttatcagcaataaaccagccagccggaagggccgagcgcagaagtggtcctgcaactttatccgcctccatccagtctattaattgttgccgggaagctagagtaagtagttcgccagttaatagtttgcgcaacgttgttgccattgctacaggcatcgtggtgtcacgctcgtcgtttggtatggcttcattcagctccggttcccaacgatcaaggcgagttacatgatcccccatgttgtgcaaaaaagcggttagctccttcggtcctccgatcgttgtcagaagtaagttggccgcagtgttatcactcatggttatggcagcactgcataattctcttactgtcatgccatccgtaagatgcttttctgtgactggtgagtactcaaccaagtcattctgagaatagtgtatgcggcgaccgagttgctcttgcccggcgtcaatacgggataataccgcgccacatagcagaactttaaaagtgctcatcattggaaaacgttcttcggggcgaaaactctcaaggatcttaccgctgttgagatccagttcgatgtaacccactcgtgcacccaactgatcttcagcatcttttactttcaccagcgtttctgggtgagcaaaaacaggaaggcaaaatgccgcaaaaaagggaataagggcgacacggaaatgttgaatactcatactcttcctttttcaatattattgaagcatttatcagggttattgtctcatgagcggatacatatttgaatgtatttagaaaaataaacaaataggggttccgcgcacatttccccgaaaagtgccacctgacgtcgacggatcgggagatctcccgatcccctatggtgcactctcagtacaatctgctctgatgccgcatagttaagccagtatctgctccctgcttgtgtgttggaggtcgctgagtagtgcgcgagcaaaatttaagctacaacaaggcaaggcttgaccgacaattgcataatacgactcactatagggcggccgccaaaaaacccctcaagacccgtttagaggccccaaggggttatgctagatctgcttagggttaggcgttttgcgctgcttcgcgatgtacgggccagatatacgcgttgacattgattattgactagttattaatagtaatcaattacggggtcattagttcatagcccatatatggagttccgcgttacataacttacggtaaatggcccgcctggctgaccgcccaacgacccccgcccattgacgtcaataatgacgtatgttcccatagtaacgccaatagggactttccattgacgtcaatgggtggagtatttacggtaaactgcccacttggcagtacatcaagtgtatcatatgccaagtacgccccctattgacgtcaatgacggtaaatggcccgcctggcattatgcccagtacatgaccttatgggactttcctacttggcagtacatctacgtattagtcatcgctattaccatggtgatgcggttttggcagtacatcaatgggcgtggatagcggtttgactcacggggatttccaagtctccaccccattgacgtcaatgggagtttgttttggcaccaaaatcaacgggactttccaaaatgtcgtaacaactccgccccattgacgcaaatgggcggtaggcgtgtacggtgggaggtctatataagcagagctctctggctaactagagaacccactgcttactggcttatcgaaattaatacgactcactatagggagacccaagctggctagcgtttaaacttaggagagccaccatgaaacggactgctgacggcagcgaatttgagagccccaagaagaagaggaaagtcaacatcaagttcaacaagttcaccggcgtgaagcccgtgtctaagaccctgagaaacgctctgatccccaccgagttcaccatggtcaacctggaacggaacggcatcatcagcgccgatgagctgagagccgagaagcggcaagagctgaagaaaatcatggacgactactaccgggacctgatcgagagaaccctggccgagaaccacagcatcaactggcacatcctgttcgagctgatgaagtccaagatgcacggcgacgagaaggacaccgccaagaagctggaaaacgagcagaagtctaagcgggaagagatccaccggctgttcgccgagcaagaggaattcggcaagatcttcagcgccaagctggtgtccgatatcctgcctggctttgtggccagctacgccatgtacaacgacgaggacagaaccgagaaggccgaggtggtcaagctgtttaacaagtttatgagcagcttcaccgagtttttcgagaaccggaagaacgtgttcagcaaagagaacatcagcaccagcctgtgccaccggatcgtgaacgacaacgccctgatcttcctgaacaacatggacagctacaagcggatcatggaaaacttcaagagcgagagcgaactggtgtccaaaggcctggaaaccatgctcggagagtggaagatctcccagatctacagcgaggacttcttcggcatgaccatgacacagagcggcatcgagttctacaacgacatctgcggcgagctgaacctggtcctgaacctgtactgccagaaaagcaagaagaacagcgcccggttcaagatgaagcggctgcacaagcagatcctgtgcaccgagaagtccagcttcgagatcagctataagtacgacaacgacaaggatgtgtacaccagcgtgaacggcttcattaagaatatcaagaacaacaacatcatcgagcggctgctgaagctgggcaccgagacagagcagtacgacctgaacaagatctacatcagctcccagagctacgagacagtgtctatcgccatcggcggcacctgggagacaatcagaaactgcctgacctcttggtacgacgacaacatcaaaggcagcggcaaggccaaagaaaacaagatcaaggccgtggtcaaggccgacaagtaccagagcattgccagagtggactacctgaccgagacatacaatgccagcggcaccgatctgcagaaagccgagagctacctgagccacatcgtgcagatcatcggcgactacgagcccgaggaactgtacttcgacgagagcatccacctgattgagaacggcgacaagatcagcgagatcaagaagatcctggacatctacatcgacgtggtgcactggatcaagacctttgagatctccgagagcgtggaaaaagagcctgagttttactacgagctggacgacatctacgacaagattctggacgccgtgcctctgtacaacaaagtgcggaactacgtgacccagaagccgtacaatcaagagaagttcaagctcaacttcgacagccccacactggccaacggctggtccaagtccaaagagagagacaacaacgccatcatcctgagccgcgacggcaagtactatctgggcgtgttcaacgtgcggaacaagcccgacaaagagatcctcgagggccacagcaagcccaagaacgagacagactacgccaagatggtctacaacctgctgccaggcgccagcaagatgctgcctaaggtgttcctgagcaagaagggcatcgacaacttcaagcccagcgactacatcctggaaggctacatcaagaaaaagcacatcaagagcagcgaaaccttcgacatcaagtactgcagggatctgatcgattacttcaagaacagcatcagcagacaccccgagtggaaaaacttcggcttcaacttcaccgaaaccagcaagtacaacgatatcagcgagttttacaaagaggtcgagaagcagggctacaagatcgagtggacctacatcaccgaagaggacatcaacaagctggatgaggccggccagatctatctgttccagatcttcaacaaggatttcgccgtgggcagcaagggcacccctaatctgcacaccctgtacctgaagaacctgttctctaaagaaaacctggacaacgtggtgctcaagctgaacggcgaggccgagctgttctttcggagaagctccatcaagacccctgtgatccacaaaaagggcagcatcctggtcaaccggtgctacgtggacgccgacgatggcaagagaaagcccattcctgagaaagagtacatggaaatctacaactactgcaacggcaagcgggacaccgagctgtctgaaagcgcccggaagtactacaacatcagccagagatacgaggccaccatggacatcgtgaaggactaccggtacagcgtggacaaactgttcatccatctgccgatcaccatcaatttcaaggccaccgagaacaagaacgtcaacgacatggtgctcgagtatatcgccaagagcgacgacatccacatcatcggcatcgaccggggcgagagaaacctgatctacgtgtccgtgatcgacatgcacggacacatcgtgatgcagaaaagctacaacgtcgtcaacgagtacgactacaagaccaagctgaaagagtgcgagcagggcagagatgccgccagaaagaactggaaagagatcgggaagatcaaagaactcaaagagggctacctcagcatggtcatccacgagatcacccagctgatcatcgagtacaacgcaatcgtgatgatggaagatttgaatttcgggttcaagcgcggcaggttcaaggtggaaagacaggtgtaccagaaattcgagaacatgctgatcaacaaactgaactacctggtggacaagcacaaagccgtggatgagcctggcggcctgctgaatggataccagctgacctacattcccgaccggatgtccgaactgggcagacagtgtggcatcatcttctacgtgccagccgcctacacctccaagatcgatcctaccaccggctttttcaacgccttccggtttaacctgctgacctccgccgagagcagacgggacttcctgaatcggttcaagtgcatcaagtataacggcagcatgaatatgttcgagttcgacttcgattacaacgatttcatcacccacaacaccacaatcgcccggacacagtggaaggtgttcaccaacggcggcaggattaagaacatcatctccaagagcggctggaacggcacaaagaagatcgacgatatcacagccctgatgaaggaaatcttcgactcccgcaagatcgacttcagcgacggcggaaatctgctgcctgagatcctggcctatgagggcgccgacaaggacaagttcatcgtggaactgctggatatcttcaagctgaccgtgcagctgcggaacagcatgcctgatggctccgacatcgagtatgaccggatcatcagccccgtgatcaacgagaacaacaccttctacgacagcgacatgtacaccgagcctaacagccctctgcctatcgacgccgatgccaatggcgcctactgtatcgccctgaagggcctgtacgaagtgaatcaaatcaaagagaattggaaagaaggcgagacattccccaagtccgtgctgaaactgaacaatgccaattggttcgatttcgtgcagaacaagagatatgagcatcatcatcaccatcaccctgctgctaagagagtgaaactggatgactacaaagaccatgacggtgattataaagatcatgatatcgattacaaggatgacgatgacaagggatccaaaagaactggaagcggagctactaacttcagcctgctgaagcaggctggagacgtggaggagaaccctggacctgttaacatggtgagcaagggcgaggaggataacatggccatcatcaaggagttcatgcgcttcaaggtgcacatggagggctccgtgaacggccacgagttcgagatcgagggcgagggcgagggccgcccctacgagggcacccagaccgccaagctgaaggtgaccaagggtggccccctgcccttcgcctgggacatcctgtcccctcagttcatgtacggctccaaggcctacgtgaagcaccccgccgacatccccgactacttgaagctgtccttccccgagggcttcaagtgggagcgcgtgatgaacttcgaggacggcggcgtggtgaccgtgacccaggactcctccctgcaggacggcgagttcatctacaaggtgaagctgcgcggcaccaacttcccctccgacggccccgtaatgcagaagaagaccatgggctgggaggcctcctccgagcggatgtaccccgaggacggcgccctgaagggcgagatcaagcagaggctgaagctgaaggacggcggccactacgacgctgaggtcaagaccacctacaaggccaagaagcccgtgcagctgcccggcgcctacaacgtcaacatcaagttggacatcacctcccacaacgaggactacaccatcgtggaacagtacgaacgcgccgagggccgccactccaccggcggcatggacgagctgtacaagtaagctcgagcctagagggcccgtttaaacccgctgatcagcctcgactgtgccttctagttgccagccatctgttgtttgcccctcccccgtgccttccttgaccctggaaggtgccactcccactgtcctttcctaataaaatgaggaaattgcatcgcattgtctgagtaggtgtcattctattctggggggtggggtggggcaggacagcaagggggaggattgggaagacaatagcaggcatgctggggatgcggtgggctctatggtaccgtcgacctctagctagagcttggcgtaatcatggtcatagctgtttcctgtgtgaaattgttatccgctcacaattccacacaacatacgagccggaagcataaagtgtaaagcctggggtgcctaatgagtgagctaactcacattaattgcgttgcgctcactgcccgctttccagtcgggaaacctgtcgtgccagctgcattaatgaatcggccaacgcgcggggagaggcggtttgcgtattgggcgctcttccgcttcctcgctcactgactcgctgcgctcggtcgttcggctgcggcgagcggtatcagctcactcaaaggcggtaatacggttatccacagaatcaggggataacgcaggaaagaacatg

SEQ ID NO: 111 - DNA, 7842 bp, synthetic construct
  misc_feature 1..7842: note = EpiCas002 gRNA plamid DNA
  source 1..7842: mol_type = other DNA
gaagatcctttgatcttttctacggggtctgacgctcagtggaacgaaaactcacgttaagggattttggtcatgagattatcaaaaaggatcttcacctagatccttttaaattaaaaatgaagttttaaatcaatctaaagtatatatgagtaaacttggtctgacagttaccaatgcttaatcagtgaggcacctatctcagcgatctgtctatttcgttcatccatagttgcctgactccccgtcgtgtagataactacgatacgggagggcttaccatctggccccagtgctgcaatgataccgcgagacccacgctcaccggctccagatttatcagcaataaaccagccagccggaagggccgagcgcagaagtggtcctgcaactttatccgcctccatccagtctattaattgttgccgggaagctagagtaagtagttcgccagttaatagtttgcgcaacgttgttgccattgctacaggcatcgtggtgtcacgctcgtcgtttggtatggcttcattcagctccggttcccaacgatcaaggcgagttacatgatcccccatgttgtgcaaaaaagcggttagctccttcggtcctccgatcgttgtcagaagtaagttggccgcagtgttatcactcatggttatggcagcactgcataattctcttactgtcatgccatccgtaagatgcttttctgtgactggtgagtactcaaccaagtcattctgagaatagtgtatgcggcgaccgagttgctcttgcccggcgtcaatacgggataataccgcgccacatagcagaactttaaaagtgctcatcattggaaaacgttcttcggggcgaaaactctcaaggatcttaccgctgttgagatccagttcgatgtaacccactcgtgcacccaactgatcttcagcatcttttactttcaccagcgtttctgggtgagcaaaaacaggaaggcaaaatgccgcaaaaaagggaataagggcgacacggaaatgttgaatactcatactcttcctttttcaatattattgaagcatttatcagggttattgtctcatgagcggatacatatttgaatgtatttagaaaaataaacaaataggggttccgcgcacatttccccgaaaagtgccacctgacgtcgacggatcgggagatctcccgatcccctatggtgcactctcagtacaatctgctctgatgccgcatagttaagccagtatctgctccctgcttgtgtgttggaggtcgctgagtagtgcgcgagcaaaatttaagctacaacaaggcaaggcttgaccgacaattgcatgaagaatctgcttagggttaggcgttttgcgctgcttcgcgatgtacgggccagatatacgcgttgacattgattattgactagttattaatagtaatcaattacggggtcattagttcatagcccatatatggagttccgcgttacataacttacggtaaatggcccgcctggctgaccgcccaacgacccccgcccattgacgtcaataatgacgtatgttcccatagtaacgccaatagggactttccattgacgtcaatgggtggagtatttacggtaaactgcccacttggcagtacatcaagtgtatcatatgccaagtacgccccctattgacgtcaatgacggtaaatggcccgcctggcattatgcccagtacatgaccttatgggactttcctacttggcagtacatctacgtattagtcatcgctattaccatggtgatgcggttttggcagtacatcaatgggcgtggatagcggtttgactcacggggatttccaagtctccaccccattgacgtcaatgggagtttgttttggcaccaaaatcaacgggactttccaaaatgtcgtaacaactccgccccattgacgcaaatgggcggtaggcgtgtacggtgggaggtctatataagcagcgcgttttgcctgtactgggtctctctggttagaccagatctgagcctgggagctctctggctaactagggaacccactgcttaagcctcaataaagcttgccttgagtgcttcaagtagtgtgtgcccgtctgttgtgtgactctggtaactagagatccctcagacccttttagtcagtgtggaaaatctctagcagtggcgcccgaacagggacttgaaagcgaaagggaaaccagaggagctctctcgacgcaggactcggcttgctgaagcgcgcacggcaagaggcgaggggcggcgactggtgagtacgccaaaaattttgactagcggaggctagaaggagagagatgggtgcgagagcgtcagtattaagcgggggagaattagatcgcgatgggaaaaaattcggttaaggccagggggaaagaaaaaatataaattaaaacatatagtatgggcaagcagggagctagaacgattcgcagttaatcctggcctgttagaaacatcagaaggctgtagacaaatactgggacagctacaaccatcccttcagacaggatcagaagaacttagatcattatataatacagtagcaaccctctattgtgtgcatcaaaggatagagataaaagacaccaaggaagctttagacaagatagaggaagagcaaaacaaaagtaagaccaccgcacagcaagcggccgctgatcttcagacctggaggaggagatatgagggacaattggagaagtgaattatataaatataaagtagtaaaaattgaaccattaggagtagcacccaccaaggcaaagagaagagtggtgcagagagaaaaaagagcagtgggaataggagctttgttccttgggttcttgggagcagcaggaagcactatgggcgcagcgtcaatgacgctgacggtacaggccagacaattattgtctggtatagtgcagcagcagaacaatttgctgagggctattgaggcgcaacagcatctgttgcaactcacagtctggggcatcaagcagctccaggcaagaatcctggctgtggaaagatacctaaaggatcaacagctcctggggatttggggttgctctggaaaactcatttgcaccactgctgtgccttggaatgctagttggagtaataaatctctggaacagatttggaatcacacgacctggatggagtgggacagagaaattaacaattacacaagcttaatacactccttaattgaagaatcgcaaaaccagcaagaaaagaatgaacaagaattattggaattagataaatgggcaagtttgtggaattggtttaacataacaaattggctgtggtatataaaattattcataatgatagtaggaggcttggtaggtttaagaatagtttttgctgtactttctatagtgaatagagttaggcagggatattcaccattatcgtttcagacccacctcccaaccccgaggggacccgacaggcccgaaggaatagaagaagaaggtggagagagagacagagacagatccattcgattagtgaacggatcggcactgcgtgcgccaattctgcagacaaatggcagtattcatccacaattttaaaagaaaaggggggattggggggtacagtgcaggggaaagaatagtagacataatagcaacagacatacaaactaaagaattacaaaaacaaattacaaaaattcaaaattttcgggtttattacaggggagggcctatttcccatgattccttcatatttgcatatacgatacaaggctgttagagagataattagaattaatttgactgtaaacacaaagatattagtacaaaatacgtgacgtagaaagtaataatttcttgggtagtttgcagttttaaaattatgttttaaaatggactatcatatgcttaccgtaacttgaaagtatttcgatttcttggctttatatatcttgtggaaaggacgaaacaccgaatttctactattgtagataagtcccctcatccccacagtttttttaggcagctgtagatctaggtcttgaaaggagtgggaattggctccggtgcccgtcagtgggcagagcgcacatcgcccacagtccccgagaagttggggggaggggtcggcaattgatccggtgcctagagaaggtggcgcggggtaaactgggaaagtgatgtcgtgtactggctccgcctttttcccgagggtgggggagaaccgtatataagtgcagtagtcgccgtgaacgttctttttcgcaacgggtttgccgccagaacacaggaccggttctagagcgctgccaccatggcgcgtaaggtcgatctcacctcctgcgatcgcgagccgatccacatccccggcagcattcagccgtgcggctgcctgctagcctgcgacgcgcaggcggtgcggatcacgcgcattacggaaaatgccggcgcgttctttggacgcgaaactccgcgggtcggtgagctactcgccgattacttcggcgagaccgaagcccatgcgctgcgcaacgcactggcgcagtcctccgatccaaagcgaccggcgctgatcttcggttggcgcgacggcctgaccggccgcaccttcgacatctcactgcatcgccatgacggtacatcgatcatcgagttcgagcctgcggcggccgaacaggccgacaatccgctgcggctgacgcggcagatcatcgcgcgcaccaaagaactgaagtcgctcgaagagatggccgcacgggtgccgcgctatctgcaggcgatgctcggctatcaccgcgtgatgttgtaccgcttcgcggacgacggctccgggatggtgatcggcgaggcgaagcgcagcgacctggagagctttctcggtcagcactttccggcgtcgctggtcccgcagcaggcgcggctactgtacttgaagaacgcgatccgcgtggtctcggattcgcgcggcatcagcagccggatcgtgcccgagcacgacgcctccggcgccgcgctcgatctgtcgttcgcgcacctgcgcagcatctcgccctgccatctcgaatttctgcggaacatgggcgtcagcgcctcgatgtcgctgtcgatcatcattgacggcacgctatggggattgatcatctgtcatcattacgagccgcgtgccgtgccgatggcgcagcgcgtcgcggccgaaatgttcgccgacttcttatcgctgcacttcaccgccgcccaccaccaacgcggatccggcgagggcagaggtagcctgctgacctgcggcgacgtggaggagaaccccggccccaccgagtacaagcccacggtgcgcctcgccacccgcgacgacgtccccagggccgtacgcaccctcgccgccgcgttcgccgactaccccgccacgcgccacaccgtcgatccggaccgccacatcgagcgggtcaccgagctgcaagaactcttcctcacgcgcgtcgggctcgacatcggcaaggtgtgggtcgcggacgacggcgccgcggtggcggtctggaccacgccggagagcgtcgaagcgggggcggtgttcgccgagatcggcccgcgcatggccgagttgagcggttcccggctggccgcgcagcaacagatggaaggcctcctggcgccgcaccggcccaaggagcccgcgtggttcctggccaccgtcggagtctcgcccgaccaccagggcaagggtctgggcagcgccgtcgtgctccccggagtggaggcggccgagcgcgccggggtgcccgccttcctggagacctccgcgccccgcaacctccccttctacgagcggctcggcttcaccgtcaccgccgacgtcgaggtgcccgaaggaccgcgcacctggtgcatgacccgcaagcccggtgcctgaacgcgttaagtcgaccgatatcaagcttatcgataatcaacctctggattacaaaatttgtgaaagattgactggtattcttaactatgttgctccttttacgctatgtggatacgctgctttaatgcctttgtatcatgctattgcttcccgtatggctttcattttctcctccttgtataaatcctggttgctgtctctttatgaggagttgtggcccgttgtcaggcaacgtggcgtggtgtgcactgtgtttgctgacgcaacccccactggttggggcattgccaccacctgtcagctcctttccgggactttcgctttccccctccctattgccacggcggaactcatcgccgcctgccttgcccgctgctggacaggggctcggctgttgggcactgacaattccgtggtgttgtcggggaaatcatcgtcctttccttggctgctcgcctgtgttgccacctggattctgcgcgggacgtccttctgctacgtcccttcggccctcaatccagcggaccttccttcccgcggcctgctgccggctctgcggcctcttccgcgtcttcgccttcgccctcagacgagtcggatctccctttgggccgcctccccgcgtcgactttaagaccaatgacttacaaggcagctgtagatcttagccactttttaaaagaaaaggggggactggaagggctaattcactcccaacgaagacaagatctgctttttgcttgtactgggtctctctggttagaccagatctgagcctgggagctctctggctaactagggaacccactgcttaagcctcaataaagcttgccttgagtgcttcaagtagtgtgtgcccgtctgttgtgtgactctggtaactagagatccctcagacccttttagtcagtgtggaaaatctctagcagggcccgtttaaacccgctgatcagcctcgactgtgccttctagttgccagccatctgttgtttgcccctcccccgtgccttccttgaccctggaaggtgccactcccactgtcctttcctaataaaatgaggaaattgcatcgcattgtctgagtaggtgtcattctattctggggggtggggtggggcaggacagcaagggggaggattgggaagacaatagcaggcatgctggggatgcggtgggctctatggcttctgaggcggaaagaaccagcggtatcagctcactcaaaggcggtaatacggttatccacagaatcaggggataacgcaggaaagaacatgtgagcaaaaggccagcaaaaggccaggaaccgtaaaaaggccgcgttgctggcgtttttccataggctccgcccccctgacgagcatcacaaaaatcgacgctcaagtcagaggtggcgaaacccgacaggactataaagataccaggcgtttccccctggaagctccctcgtgcgctctcctgttccgaccctgccgcttaccggatacctgtccgcctttctcccttcgggaagcgtggcgctttctcatagctcacgctgtaggtatctcagttcggtgtaggtcgttcgctccaagctgggctgtgtgcacgaaccccccgttcagcccgaccgctgcgccttatccggtaactatcgtcttgagtccaacccggtaagacacgacttatcgccactggcagcagccactggtaacaggattagcagagcgaggtatgtaggcggtgctacagagttcttgaagtggtggcctaactacggctacactagaagaacagtatttggtatctgcgctctgctgaagccagttaccttcggaaaaagagttggtagctcttgatccggcaaacaaaccaccgctggtagcggtggtttttttgtttgcaagcagcagattacgcgcagaaaaaaaggatctcaa

SEQ ID NO: 112 - DNA, 7160 bp, synthetic construct
  misc_feature 1..7160: note = EpiCas057 plamid DNA
  source 1..7160: mol_type = other DNA
tgagcaaaaggccagcaaaaggccaggaaccgtaaaaaggccgcgttgctggcgtttttccataggctccgcccccctgacgagcatcacaaaaatcgacgctcaagtcagaggtggcgaaacccgacaggactataaagataccaggcgtttccccctggaagctccctcgtgcgctctcctgttccgaccctgccgcttaccggatacctgtccgcctttctcccttcgggaagcgtggcgctttctcatagctcacgctgtaggtatctcagttcggtgtaggtcgttcgctccaagctgggctgtgtgcacgaaccccccgttcagcccgaccgctgcgccttatccggtaactatcgtcttgagtccaacccggtaagacacgacttatcgccactggcagcagccactggtaacaggattagcagagcgaggtatgtaggcggtgctacagagttcttgaagtggtggcctaactacggctacactagaagaacagtatttggtatctgcgctctgctgaagccagttaccttcggaaaaagagttggtagctcttgatccggcaaacaaaccaccgctggtagcggtttttttgtttgcaagcagcagattacgcgcagaaaaaaaggatctcaagaagatcctttgatcttttctacggggtctgacgctcagtggaacgaaaactcacgttaagggattttggtcatgagattatcaaaaaggatcttcacctagatccttttaaattaaaaatgaagttttaaatcaatctaaagtatatatgagtaaacttggtctgacagttaccaatgcttaatcagtgaggcacctatctcagcgatctgtctatttcgttcatccatagttgcctgactccccgtcgtgtagataactacgatacgggagggcttaccatctggccccagtgctgcaatgataccgcgagacccacgctcaccggctccagatttatcagcaataaaccagccagccggaagggccgagcgcagaagtggtcctgcaactttatccgcctccatccagtctattaattgttgccgggaagctagagtaagtagttcgccagttaatagtttgcgcaacgttgttgccattgctacaggcatcgtggtgtcacgctcgtcgtttggtatggcttcattcagctccggttcccaacgatcaaggcgagttacatgatcccccatgttgtgcaaaaaagcggttagctccttcggtcctccgatcgttgtcagaagtaagttggccgcagtgttatcactcatggttatggcagcactgcataattctcttactgtcatgccatccgtaagatgcttttctgtgactggtgagtactcaaccaagtcattctgagaatagtgtatgcggcgaccgagttgctcttgcccggcgtcaatacgggataataccgcgccacatagcagaactttaaaagtgctcatcattggaaaacgttcttcggggcgaaaactctcaaggatcttaccgctgttgagatccagttcgatgtaacccactcgtgcacccaactgatcttcagcatcttttactttcaccagcgtttctgggtgagcaaaaacaggaaggcaaaatgccgcaaaaaagggaataagggcgacacggaaatgttgaatactcatactcttcctttttcaatattattgaagcatttatcagggttattgtctcatgagcggatacatatttgaatgtatttagaaaaataaacaaataggggttccgcgcacatttccccgaaaagtgccacctgacgtcgacggatcgggagatctcccgatcccctatggtgcactctcagtacaatctgctctgatgccgcatagttaagccagtatctgctccctgcttgtgtgttggaggtcgctgagtagtgcgcgagcaaaatttaagctacaacaaggcaaggcttgaccgacaattgcataatacgactcactatagggcggccgccaaaaaacccctcaagacccgtttagaggccccaaggggttatgctagatctgcttagggttaggcgttttgcgctgcttcgcgatgtacgggccagatatacgcgttgacattgattattgactagttattaatagtaatcaattacggggtcattagttcatagcccatatatggagttccgcgttacataacttacggtaaatggcccgcctggctgaccgcccaacgacccccgcccattgacgtcaataatgacgtatgttcccatagtaacgccaatagggactttccattgacgtcaatgggtggagtatttacggtaaactgcccacttggcagtacatcaagtgtatcatatgccaagtacgccccctattgacgtcaatgacggtaaatggcccgcctggcattatgcccagtacatgaccttatgggactttcctacttggcagtacatctacgtattagtcatcgctattaccatggtgatgcggttttggcagtacatcaatgggcgtggatagcggtttgactcacggggatttccaagtctccaccccattgacgtcaatgggagtttgttttggcaccaaaatcaacgggactttccaaaatgtcgtaacaactccgccccattgacgcaaatgggcggtaggcgtgtacggtgggaggtctatataagcagagctctctggctaactagagaacccactgcttactggcttatcgaaattaatacgactcactatagggagacccaagctggctagcgtttaaacttaggagagccaccatgaaacggactgctgacggcagcgaatttgagagccccaagaagaagaggaaagtcggatccgaagagacacggacccctgagaagatcgcctgccagcaggatagaagcgccttcttcaagctgggcaagctgccccagaaaaccaccagcgccatctaccacctgatgcggtgtagcaagcggtacatcgacaacgtgtccgagacaatcagcaacaacatcgagaaggccgccatgaccagcgacaaccacatcttcagaagcgccctgaaagaagagtacaagaagatctaccgcgagaagttctaccccgacgtgaccggccagccttttccagataagggccccgacaacacccacatcgtggaacggaccgtggaaaacctgtgcggccagtacatctctgccctgaagggcgtgatgaaagtgcggaagcccaagtggcaggacgacatcttcgaggacgagagcgacaaagtgatcgccgagatgctgatggccagcggcaacgaggccgacattcaccccaagctggaaaagaagattgccagcgccaagaaaaaggacaagatggacgagtggcagaaggtgctggacagatacgactacatcaagagcaagaccgacatcgagtggacctacaccacactgctgtacgaccacattgcccgcgagtgcgccagatccatgttcgaggatggcaacaagcctaagttctgctacaccaacggcaacaagttcgccaaacaggtggtggacgagctgtggggctctgagagagtggaatacgagtacgagaagtacctgcactgcagaaccctggaagcctactggaacgaggaaaacaagtacttcttcctggaaaatcaaaagaagtccaagaaaacctacgaggcccggcagatcatcgaccacttcatcgagaacgaggacgccgtgaaggccgaaaccgaagagtatatggccaaggtggccaaagagttcggcgagaacggcggctgcaagttcagaaccgagaacatcctgtacctggtcaacagcgtgtccatcaacaagaagcaggacgaggaacggtgccccatcttcaaagtgaccgacattccccagtatgccgaggccggcatcgatagaatcggcgagtgcaaatacgtgatcaagctgaagctgttcaccgtgggcgagagatacggcaccacctatatgcctgaggccttcagcggcctgtacgacagaaggaccaaccagagatacgacctgatcgacagagcctgcaagggcagctacgtgtacctgcctatctacatcagcgacaaggacagccggaagtggagcgacagactgaagaacaccttcaccatgtccgccttcagcatcagcgagcgcaagaccaagaaagacggcagagtgctgtgcgtgaacctgccttacacacacatccagcacaagccccggaactacttcaaggtgtaccccacctacggcgtggacatcaacgtgaagcacagcctgttcagcaccaacgccaccaacctgaacggctacatcgacgtgaacggcgagctgatcgacttctacaacagcatcggcagacccgataagctcaagaacatcaacctggccgtgacactgggcgacaaaggcggcacagctggcaaccacaccaactttctgctggtgtccgacctcggcgactgggatgatcacggcaagaagcggaacgacagattcgtgaagagagaggacggcacctactacagcagacctgacctgctggccgacggcctgaacttcctgaagaagaagtatagcggcgaccggaagtcctacgattatatcaacaccacaatcgccttccggaacaaccagaccagactgagatgcatcgacaaagagtggaacgatcggaagcgggcctacgatgaggaacacggcaagcctgagaagggcgaaagaagcggcttctaccctaccgaggatgccgagcggctgacaatggaaagacaggccctgcggagagagattgccgagaacaccagacaagtgattgcctacatgctgtggctgttccaagagaacggcatcaagtctatcgccctggaacacctggattgcggcagctggaagaacttccgggaccagctgaagccaaagtggttctgcaacaactgcaagtactgggccgagaagtatggcatcccttacgaggccaccaagtactacagaagcaaccggaagtactttgacatcgaggacggggagctgattcccgagaatgtgaagctgaacgccctgggcgaagccgagaacgacaagagatacttccagacctctatcgccaaggccgtgggcatgagcagcatcaagcagatgttcagcatcgtgtcccagaactacgacatccaagtgaactacaccgagcaggcctacaccagccagaccgacagcagaaatggcaccgtggacaaggacttcagagtgtcccaagagtgctacatcggcagcgacggcaccaagatgaactgcgactttaacgccgccgtgaatatcgccgaccggatctccgatgacaccctgcgggaagagttcaacaaagaactgcccatgaaggaatttgtgaagtacggcgccacacagatcgtgtctcggaacagaagatggaacgccgaaaacgccgagagggtcacaatggccgccttccagaagagaaagaacgctgacggcggagcccataccgccgctgtgaagcctacatccaagaccgaggaaagcagcctgaagctggtggccgaaggatcccatcatcatcaccatcaccctgctgctaagagagtgaaactggatgactacaaagaccatgacggtgattataaagatcatgatatcgattacaaggatgacgatgacaagggatccaaaagaactggaagcggagctactaacttcagcctgctgaagcaggctggtgacgtggaggagaaccctggacctgttaacatggtgagcaagggcgaggaggataacatggccatcatcaaggagttcatgcgcttcaaggtgcacatggagggctccgtgaacggccacgagttcgagatcgagggcgagggcgagggccgcccctacgagggcacccagaccgccaagctgaaggtgaccaagggtggccccctgcccttcgcctgggacatcctgtcccctcagttcatgtacggctccaaggcctacgtgaagcaccccgccgacatccccgactacttgaagctgtccttccccgagggcttcaagtgggagcgcgtgatgaacttcgaggacggcggcgtggtgaccgtgacccaggactcctccctgcaggacggcgagttcatctacaaggtgaagctgcgcggcaccaacttcccctccgacggccccgtaatgcagaagaagaccatgggctgggaggcctcctccgagcggatgtaccccgaggacggcgccctgaagggcgagatcaagcagaggctgaagctgaaggacggcggccactacgacgctgaggtcaagaccacctacaaggccaagaagcccgtgcagctgcccggcgcctacaacgtcaacatcaagttggacatcacctcccacaacgaggactacaccatcgtggaacagtacgaacgcgccgagggccgccactccaccggcggcatggacgagctgtacaagtaagctcgagcctagagggcccgtttaaacccgctgatcagcctcgactgtgccttctagttgccagccatctgttgtttgcccctcccccgtgccttccttgaccctggaaggtgccactcccactgtcctttcctaataaaatgaggaaattgcatcgcattgtctgagtaggtgtcattctattctggggggtggggtggggcaggacagcaagggggaggattgggaagacaatagcaggcatgctggggatgcggtgggctctatggtaccgtcgacctctagctagagcttggcgtaatcatggtcatagctgtttcctgtgtgaaattgttatccgctcacaattccacacaacatacgagccggaagcataaagtgtaaagcctggggtgcctaatgagtgagctaactcacattaattgcgttgcgctcactgcccgctttccagtcgggaaacctgtcgtgccagctgcattaatgaatcggccaacgcgcggggagaggcggtttgcgtattgggcgctcttccgcttcctcgctcactgactcgctgcgctcggtcgttcggctgcggcgagcggtatcagctcactcaaaggcggtaatacggttatccacagaatcaggggataacgcaggaaagaacatg

SEQ ID NO: 113 - DNA, 7854 bp, synthetic construct
  misc_feature 1..7854: note = EpiCas057 gRNA plamid DNA
  source 1..7854: mol_type = other DNA
gaagatcctttgatcttttctacggggtctgacgctcagtggaacgaaaactcacgttaagggattttggtcatgagattatcaaaaaggatcttcacctagatccttttaaattaaaaatgaagttttaaatcaatctaaagtatatatgagtaaacttggtctgacagttaccaatgcttaatcagtgaggcacctatctcagcgatctgtctatttcgttcatccatagttgcctgactccccgtcgtgtagataactacgatacgggagggcttaccatctggccccagtgctgcaatgataccgcgagacccacgctcaccggctccagatttatcagcaataaaccagccagccggaagggccgagcgcagaagtggtcctgcaactttatccgcctccatccagtctattaattgttgccgggaagctagagtaagtagttcgccagttaatagtttgcgcaacgttgttgccattgctacaggcatcgtggtgtcacgctcgtcgtttggtatggcttcattcagctccggttcccaacgatcaaggcgagttacatgatcccccatgttgtgcaaaaaagcggttagctccttcggtcctccgatcgttgtcagaagtaagttggccgcagtgttatcactcatggttatggcagcactgcataattctcttactgtcatgccatccgtaagatgcttttctgtgactggtgagtactcaaccaagtcattctgagaatagtgtatgcggcgaccgagttgctcttgcccggcgtcaatacgggataataccgcgccacatagcagaactttaaaagtgctcatcattggaaaacgttcttcggggcgaaaactctcaaggatcttaccgctgttgagatccagttcgatgtaacccactcgtgcacccaactgatcttcagcatcttttactttcaccagcgtttctgggtgagcaaaaacaggaaggcaaaatgccgcaaaaaagggaataagggcgacacggaaatgttgaatactcatactcttcctttttcaatattattgaagcatttatcagggttattgtctcatgagcggatacatatttgaatgtatttagaaaaataaacaaataggggttccgcgcacatttccccgaaaagtgccacctgacgtcgacggatcgggagatctcccgatcccctatggtgcactctcagtacaatctgctctgatgccgcatagttaagccagtatctgctccctgcttgtgtgttggaggtcgctgagtagtgcgcgagcaaaatttaagctacaacaaggcaaggcttgaccgacaattgcatgaagaatctgcttagggttaggcgttttgcgctgcttcgcgatgtacgggccagatatacgcgttgacattgattattgactagttattaatagtaatcaattacggggtcattagttcatagcccatatatggagttccgcgttacataacttacggtaaatggcccgcctggctgaccgcccaacgacccccgcccattgacgtcaataatgacgtatgttcccatagtaacgccaatagggactttccattgacgtcaatgggtggagtatttacggtaaactgcccacttggcagtacatcaagtgtatcatatgccaagtacgccccctattgacgtcaatgacggtaaatggcccgcctggcattatgcccagtacatgaccttatgggactttcctacttggcagtacatctacgtattagtcatcgctattaccatggtgatgcggttttggcagtacatcaatgggcgtggatagcggtttgactcacggggatttccaagtctccaccccattgacgtcaatgggagtttgttttggcaccaaaatcaacgggactttccaaaatgtcgtaacaactccgccccattgacgcaaatgggcggtaggcgtgtacggtgggaggtctatataagcagcgcgttttgcctgtactgggtctctctggttagaccagatctgagcctgggagctctctggctaactagggaacccactgcttaagcctcaataaagcttgccttgagtgcttcaagtagtgtgtgcccgtctgttgtgtgactctggtaactagagatccctcagacccttttagtcagtgtggaaaatctctagcagtggcgcccgaacagggacttgaaagcgaaagggaaaccagaggagctctctcgacgcaggactcggcttgctgaagcgcgcacggcaagaggcgaggggcggcgactggtgagtacgccaaaaattttgactagcggaggctagaaggagagagatgggtgcgagagcgtcagtattaagcgggggagaattagatcgcgatgggaaaaaattcggttaaggccagggggaaagaaaaaatataaattaaaacatatagtatgggcaagcagggagctagaacgattcgcagttaatcctggcctgttagaaacatcagaaggctgtagacaaatactgggacagctacaaccatcccttcagacaggatcagaagaacttagatcattatataatacagtagcaaccctctattgtgtgcatcaaaggatagagataaaagacaccaaggaagctttagacaagatagaggaagagcaaaacaaaagtaagaccaccgcacagcaagcggccgctgatcttcagacctggaggaggagatatgagggacaattggagaagtgaattatataaatataaagtagtaaaaattgaaccattaggagtagcacccaccaaggcaaagagaagagtggtgcagagagaaaaaagagcagtgggaataggagctttgttccttgggttcttgggagcagcaggaagcactatgggcgcagcgtcaatgacgctgacggtacaggccagacaattattgtctggtatagtgcagcagcagaacaatttgctgagggctattgaggcgcaacagcatctgttgcaactcacagtctggggcatcaagcagctccaggcaagaatcctggctgtggaaagatacctaaaggatcaacagctcctggggatttggggttgctctggaaaactcatttgcaccactgctgtgccttggaatgctagttggagtaataaatctctggaacagatttggaatcacacgacctggatggagtgggacagagaaattaacaattacacaagcttaatacactccttaattgaagaatcgcaaaaccagcaagaaaagaatgaacaagaattattggaattagataaatgggcaagtttgtggaattggtttaacataacaaattggctgtggtatataaaattattcataatgatagtaggaggcttggtaggtttaagaatagtttttgctgtactttctatagtgaatagagttaggcagggatattcaccattatcgtttcagacccacctcccaaccccgaggggacccgacaggcccgaaggaatagaagaagaaggtggagagagagacagagacagatccattcgattagtgaacggatcggcactgcgtgcgccaattctgcagacaaatggcagtattcatccacaattttaaaagaaaaggggggattggggggtacagtgcaggggaaagaatagtagacataatagcaacagacatacaaactaaagaattacaaaaacaaattacaaaaattcaaaattttcgggtttattacaggggagggcctatttcccatgattccttcatatttgcatatacgatacaaggctgttagagagataattagaattaatttgactgtaaacacaaagatattagtacaaaatacgtgacgtagaaagtaataatttcttgggtagtttgcagttttaaaattatgttttaaaatggactatcatatgcttaccgtaacttgaaagtatttcgatttcttggctttatatatcttgtggaaaggacgaaacaccgatgcggtatcaacttgattggtactgacaccaagtcccctcatccccacagtttttttaggcagctgtagatctaggtcttgaaaggagtgggaattggctccggtgcccgtcagtgggcagagcgcacatcgcccacagtccccgagaagttggggggaggggtcggcaattgatccggtgcctagagaaggtggcgcggggtaaactgggaaagtgatgtcgtgtactggctccgcctttttcccgagggtgggggagaaccgtatataagtgcagtagtcgccgtgaacgttctttttcgcaacgggtttgccgccagaacacaggaccggttctagagcgctgccaccatggcgcgtaaggtcgatctcacctcctgcgatcgcgagccgatccacatccccggcagcattcagccgtgcggctgcctgctagcctgcgacgcgcaggcggtgcggatcacgcgcattacggaaaatgccggcgcgttctttggacgcgaaactccgcgggtcggtgagctactcgccgattacttcggcgagaccgaagcccatgcgctgcgcaacgcactggcgcagtcctccgatccaaagcgaccggcgctgatcttcggttggcgcgacggcctgaccggccgcaccttcgacatctcactgcatcgccatgacggtacatcgatcatcgagttcgagcctgcggcggccgaacaggccgacaatccgctgcggctgacgcggcagatcatcgcgcgcaccaaagaactgaagtcgctcgaagagatggccgcacgggtgccgcgctatctgcaggcgatgctcggctatcaccgcgtgatgttgtaccgcttcgcggacgacggctccgggatggtgatcggcgaggcgaagcgcagcgacctggagagctttctcggtcagcactttccggcgtcgctggtcccgcagcaggcgcggctactgtacttgaagaacgcgatccgcgtggtctcggattcgcgcggcatcagcagccggatcgtgcccgagcacgacgcctccggcgccgcgctcgatctgtcgttcgcgcacctgcgcagcatctcgccctgccatctcgaatttctgcggaacatgggcgtcagcgcctcgatgtcgctgtcgatcatcattgacggcacgctatggggattgatcatctgtcatcattacgagccgcgtgccgtgccgatggcgcagcgcgtcgcggccgaaatgttcgccgacttcttatcgctgcacttcaccgccgcccaccaccaacgcggatccggcgagggcagaggtagcctgctgacctgcggcgacgtggaggagaaccccggccccaccgagtacaagcccacggtgcgcctcgccacccgcgacgacgtccccagggccgtacgcaccctcgccgccgcgttcgccgactaccccgccacgcgccacaccgtcgatccggaccgccacatcgagcgggtcaccgagctgcaagaactcttcctcacgcgcgtcgggctcgacatcggcaaggtgtgggtcgcggacgacggcgccgcggtggcggtctggaccacgccggagagcgtcgaagcgggggcggtgttcgccgagatcggcccgcgcatggccgagttgagcggttcccggctggccgcgcagcaacagatggaaggcctcctggcgccgcaccggcccaaggagcccgcgtggttcctggccaccgtcggagtctcgcccgaccaccagggcaagggtctgggcagcgccgtcgtgctccccggagtggaggcggccgagcgcgccggggtgcccgccttcctggagacctccgcgccccgcaacctccccttctacgagcggctcggcttcaccgtcaccgccgacgtcgaggtgcccgaaggaccgcgcacctggtgcatgacccgcaagcccggtgcctgaacgcgttaagtcgaccgatatcaagcttatcgataatcaacctctggattacaaaatttgtgaaagattgactggtattcttaactatgttgctccttttacgctatgtggatacgctgctttaatgcctttgtatcatgctattgcttcccgtatggctttcattttctcctccttgtataaatcctggttgctgtctctttatgaggagttgtggcccgttgtcaggcaacgtggcgtggtgtgcactgtgtttgctgacgcaacccccactggttggggcattgccaccacctgtcagctcctttccgggactttcgctttccccctccctattgccacggcggaactcatcgccgcctgccttgcccgctgctggacaggggctcggctgttgggcactgacaattccgtggtgttgtcggggaaatcatcgtcctttccttggctgctcgcctgtgttgccacctggattctgcgcgggacgtccttctgctacgtcccttcggccctcaatccagcggaccttccttcccgcggcctgctgccggctctgcggcctcttccgcgtcttcgccttcgccctcagacgagtcggatctccctttgggccgcctccccgcgtcgactttaagaccaatgacttacaaggcagctgtagatcttagccactttttaaaagaaaaggggggactggaagggctaattcactcccaacgaagacaagatctgctttttgcttgtactgggtctctctggttagaccagatctgagcctgggagctctctggctaactagggaacccactgcttaagcctcaataaagcttgccttgagtgcttcaagtagtgtgtgcccgtctgttgtgtgactctggtaactagagatccctcagacccttttagtcagtgtggaaaatctctagcagggcccgtttaaacccgctgatcagcctcgactgtgccttctagttgccagccatctgttgtttgcccctcccccgtgccttccttgaccctggaaggtgccactcccactgtcctttcctaataaaatgaggaaattgcatcgcattgtctgagtaggtgtcattctattctggggggtggggtggggcaggacagcaagggggaggattgggaagacaatagcaggcatgctggggatgcggtgggctctatggcttctgaggcggaaagaaccagcggtatcagctcactcaaaggcggtaatacggttatccacagaatcaggggataacgcaggaaagaacatgtgagcaaaaggccagcaaaaggccaggaaccgtaaaaaggccgcgttgctggcgtttttccataggctccgcccccctgacgagcatcacaaaaatcgacgctcaagtcagaggtggcgaaacccgacaggactataaagataccaggcgtttccccctggaagctccctcgtgcgctctcctgttccgaccctgccgcttaccggatacctgtccgcctttctcccttcgggaagcgtggcgctttctcatagctcacgctgtaggtatctcagttcggtgtaggtcgttcgctccaagctgggctgtgtgcacgaaccccccgttcagcccgaccgctgcgccttatccggtaactatcgtcttgagtccaacccggtaagacacgacttatcgccactggcagcagccactggtaacaggattagcagagcgaggtatgtaggcggtgctacagagttcttgaagtggtggcctaactacggctacactagaagaacagtatttggtatctgcgctctgctgaagccagttaccttcggaaaaagagttggtagctcttgatccggcaaacaaaccaccgctggtagcggtggtttttttgtttgcaagcagcagattacgcgcagaaaaaaaggatctcaa

SEQ ID NO: 114 - DNA, 7770 bp, synthetic construct
  misc_feature 1..7770: note = EpiCas059 plamid DNA
  source 1..7770: mol_type = other DNA
tgagcaaaaggccagcaaaaggccaggaaccgtaaaaaggccgcgttgctggcgtttttccataggctccgcccccctgacgagcatcacaaaaatcgacgctcaagtcagaggtggcgaaacccgacaggactataaagataccaggcgtttccccctggaagctccctcgtgcgctctcctgttccgaccctgccgcttaccggatacctgtccgcctttctcccttcgggaagcgtggcgctttctcatagctcacgctgtaggtatctcagttcggtgtaggtcgttcgctccaagctgggctgtgtgcacgaaccccccgttcagcccgaccgctgcgccttatccggtaactatcgtcttgagtccaacccggtaagacacgacttatcgccactggcagcagccactggtaacaggattagcagagcgaggtatgtaggcggtgctacagagttcttgaagtggtggcctaactacggctacactagaagaacagtatttggtatctgcgctctgctgaagccagttaccttcggaaaaagagttggtagctcttgatccggcaaacaaaccaccgctggtagcggtttttttgtttgcaagcagcagattacgcgcagaaaaaaaggatctcaagaagatcctttgatcttttctacggggtctgacgctcagtggaacgaaaactcacgttaagggattttggtcatgagattatcaaaaaggatcttcacctagatccttttaaattaaaaatgaagttttaaatcaatctaaagtatatatgagtaaacttggtctgacagttaccaatgcttaatcagtgaggcacctatctcagcgatctgtctatttcgttcatccatagttgcctgactccccgtcgtgtagataactacgatacgggagggcttaccatctggccccagtgctgcaatgataccgcgagacccacgctcaccggctccagatttatcagcaataaaccagccagccggaagggccgagcgcagaagtggtcctgcaactttatccgcctccatccagtctattaattgttgccgggaagctagagtaagtagttcgccagttaatagtttgcgcaacgttgttgccattgctacaggcatcgtggtgtcacgctcgtcgtttggtatggcttcattcagctccggttcccaacgatcaaggcgagttacatgatcccccatgttgtgcaaaaaagcggttagctccttcggtcctccgatcgttgtcagaagtaagttggccgcagtgttatcactcatggttatggcagcactgcataattctcttactgtcatgccatccgtaagatgcttttctgtgactggtgagtactcaaccaagtcattctgagaatagtgtatgcggcgaccgagttgctcttgcccggcgtcaatacgggataataccgcgccacatagcagaactttaaaagtgctcatcattggaaaacgttcttcggggcgaaaactctcaaggatcttaccgctgttgagatccagttcgatgtaacccactcgtgcacccaactgatcttcagcatcttttactttcaccagcgtttctgggtgagcaaaaacaggaaggcaaaatgccgcaaaaaagggaataagggcgacacggaaatgttgaatactcatactcttcctttttcaatattattgaagcatttatcagggttattgtctcatgagcggatacatatttgaatgtatttagaaaaataaacaaataggggttccgcgcacatttccccgaaaagtgccacctgacgtcgacggatcgggagatctcccgatcccctatggtgcactctcagtacaatctgctctgatgccgcatagttaagccagtatctgctccctgcttgtgtgttggaggtcgctgagtagtgcgcgagcaaaatttaagctacaacaaggcaaggcttgaccgacaattgcataatacgactcactatagggcggccgccaaaaaacccctcaagacccgtttagaggccccaaggggttatgctagatctgcttagggttaggcgttttgcgctgctgagggcctatttcccatgattccttcatatttgcatatacgatacaaggctgttagagagataattagaattaatttgactgtaaacacaaagatattagtacaaaatacgtgacgtagaaagtaataatttcttgggtagtttgcagttttaaaattatgttttaaaatggactatcatatgcttaccgtaacttgaaagtatttcgatttcttggctttatatatcttgtggaaaggacgaaacaccgagaaatccgtccttggttgacgggaagtcccctcatccccacagtttttttaggcagctgtagatctcgcgatgtacgggccagatatacgcgttgacattgattattgactagttattaatagtaatcaattacggggtcattagttcatagcccatatatggagttccgcgttacataacttacggtaaatggcccgcctggctgaccgcccaacgacccccgcccattgacgtcaataatgacgtatgttcccatagtaacgccaatagggactttccattgacgtcaatgggtggagtatttacggtaaactgcccacttggcagtacatcaagtgtatcatatgccaagtacgccccctattgacgtcaatgacggtaaatggcccgcctggcattatgcccagtacatgaccttatgggactttcctacttggcagtacatctacgtattagtcatcgctattaccatggtgatgcggttttggcagtacatcaatgggcgtggatagcggtttgactcacggggatttccaagtctccaccccattgacgtcaatgggagtttgttttggcaccaaaatcaacgggactttccaaaatgtcgtaacaactccgccccattgacgcaaatgggcggtaggcgtgtacggtgggaggtctatataagcagagctctctggctaactagagaacccactgcttactggcttatcgaaattaatacgactcactatagggagacccaagctggctagcgtttaaacttaggagagccaccatgaaacggactgctgacggcagcgaatttgagagccccaagaagaagaggaaagtcggcatcaccatgagcgacaccaccttcagaccctacaagagcaagctgaaccccaacgagcggaagatgcctatggtggtggacaccatgaattggtgcgacaacgcctgcagcgtgttcttcgatctgttcgtgggcctgtacggcggcgtgaagatcggcgacgtgaccaatttcctgaccgagaagcaggacaccaccaccgatgccgatctgctgtgcgccatcaactggttcagagccatgcctgtgtctaaccccgatgccgttgtgggacctgagcagctggttgtgcggttcagagactacagcggccacaatccatctccaatggccagcatgtacctgagcgcccctgtgaaccctagatacacctgggtcgactgccggttcctgtaccagcagatgtgtcagaccctgggcgccaacctggatgtggacatctctaccctggtgcagaccggcctgctgcctatccagaaggatacacagctgaacgcctacagcttctgcagcaacgtgttcggcgagggcgtgaaagaagatcccagcgccaaagtgaccagctacacagccgctgccaatgctctgagcggcgccaccaatcctatcatcacctacgaggactaccggcagatcctgtccagcgccatcaccaacagacccagcagaaagggcgccaaggatattctggccgccgatctggatagcaccaagacaggtgttctgcccggcaactacgtgtcccagagaatcgccatgtaccaggcctctgccgcctctaaagctagaggcgtggtgctgcccaaccggctgagagtgaaagcctacctgcagaacctcgtgggactgaactacatctgcaccacctgggccgctcctatgctgagagccgtgggcgacatcaagagcaagaacagcaacaactaccgcttcgtgggcgagagactggaacggcagcaagagatcgataacctgctggccgtgtccaacatcagaagcgcccaggccatcctgcagcagttcagggccaatgagagcaaccagttctacatcaagaagcggcacatcggcaagggcctgcctagcctgtacgacatgtgggatctgatggacgagaaagagggcatcgacaactacatccagagcctgaagggcgacaagaccgagaggctgccaatcagagagctgctgcagatcatctaccctcacagaaagagcgtgtccgccgagctgtttctgtctgccgccgaactgaccgacgtggaagatagacagaaccggtgcatggtgcaccctacagtgcggggctctctggtcatcaacttcggcaagagcagcaccatcttcggcgctatcacccctcctgacacactgatcaagttccggggcgaaatggtgcctgctggacagacaggcatgatctggttcacaatgcacctggtggacggcggcaaatgggtcaagcaccacattccttgccacagcagccggtacttcgaggaaatctacgcctggaagaaggacctgcctacactgccctttccacggcggagcctgtatggctatgccatcggcaacaagatcagcgacacccggaagatcgacctgcggagaaagaaggccagcaagcagtacctgcggaccctggaaaacatgacccacaacgtggaatttgaccccaccacacagttcatggtggaccaagagctgaacgtgaccatcaccgccagagtgaagaaaatccctcctgtgcgggatgtgcccgtgggcagcagaattatgggcctgaacaagaaccagaccatccgggactgctacagcatctgggagagagtggaagccaacaccagcggcagctttcagcatcccgtggtccaggatgtgtggctgagactggtggccgatggccacgtgacctctacagtgaatggccccaacggccagatcgaccagatgagctactctggccccgatgtggccaactgcggcaactggatgcaagagcggagcaacttcatcaccagcgtggacgacgccgaccagtctatcatgaagcactttctgtggaacaaccgcgtgaagctgtatgcctggaactgcgtgtacgccggcacactgatgaaggccatctctaagcagatgaccaccgccaaccggaacctgttcagaaacgagatcctgagcttcgttggcggcagattcggctgcagactgggatctctggcccaggtttcactggacctgctgcggaggatgaagtccgtgatcagctgctacttcagccggaacaacgccttcaccatcgaggaaagaagcgccttcgacaaagaactgatggaactgttcgagagcctggacaacaagatgaacaacaagcggaaagagaaagtcaaccggacactcagcagcatcttccaggtggccaagcagcacaatgttgtgcggctggtggtcaccaagaacctgcagacccctgatgccaatgtgcggagcgtgatgaatcagagatccgtggattggtgcgctcggaagattgaagagaagatcgtggacctgggcaacgtgatcggaatctatgtggatctggtggaagccctggatctgagccatctggaccccttcatctatatcgccaagggcgacgtgggcaaagagtgccagtttgacgaggtggaaagcagctccctgctgccaattcacaccagcatgtttcgcgactggcacggcctggttaacaagggcagaaccaccacacctatctaccacagcgccctgaggagcttcgccagccactacggcctgagattcgatgacctggccagaatcaaggccgctgagctggccaaaatgctgccagaccagaaggtgttcatcccacacagaggcggacggttcttcatgagcacataccccgtgaccagcaccagcagacccgtgtcttatgatggccggcagcggttcctgaacagcggcgatatggtggccccagtgaacaccatgctgcgcggattcagaagggccagatctggatcccatcatcatcaccatcaccctgctgctaagagagtgaaactggatgactacaaagaccatgacggtgattataaagatcatgatatcgattacaaggatgacgatgacaagggatccaaaagaactggaagcggagctactaacttcagcctgctgaagcaggctggagacgtggaggagaaccctggacctgttaacatggtgagcaagggcgaggaggataacatggccatcatcaaggagttcatgcgcttcaaggtgcacatggagggctccgtgaacggccacgagttcgagatcgagggcgagggcgagggccgcccctacgagggcacccagaccgccaagctgaaggtgaccaagggtggccccctgcccttcgcctgggacatcctgtcccctcagttcatgtacggctccaaggcctacgtgaagcaccccgccgacatccccgactacttgaagctgtccttccccgagggcttcaagtgggagcgcgtgatgaacttcgaggacggcggcgtggtgaccgtgacccaggactcctccctgcaggacggcgagttcatctacaaggtgaagctgcgcggcaccaacttcccctccgacggccccgtaatgcagaagaagaccatgggctgggaggcctcctccgagcggatgtaccccgaggacggcgccctgaagggcgagatcaagcagaggctgaagctgaaggacggcggccactacgacgctgaggtcaagaccacctacaaggccaagaagcccgtgcagctgcccggcgcctacaacgtcaacatcaagttggacatcacctcccacaacgaggactacaccatcgtggaacagtacgaacgcgccgagggccgccactccaccggcggcatggacgagctgtacaagtaagctcgagcctagagggcccgtttaaacccgctgatcagcctcgactgtgccttctagttgccagccatctgttgtttgcccctcccccgtgccttccttgaccctggaaggtgccactcccactgtcctttcctaataaaatgaggaaattgcatcgcattgtctgagtaggtgtcattctattctggggggtggggtggggcaggacagcaagggggaggattgggaagacaatagcaggcatgctggggatgcggtgggctctatggtaccgtcgacctctagctagagcttggcgtaatcatggtcatagctgtttcctgtgtgaaattgttatccgctcacaattccacacaacatacgagccggaagcataaagtgtaaagcctggggtgcctaatgagtgagctaactcacattaattgcgttgcgctcactgcccgctttccagtcgggaaacctgtcgtgccagctgcattaatgaatcggccaacgcgcggggagaggcggtttgcgtattgggcgctcttccgcttcctcgctcactgactcgctgcgctcggtcgttcggctgcggcgagcggtatcagctcactcaaaggcggtaatacggttatccacagaatcaggggataacgcaggaaagaacatg

SEQ ID NO: 115 - DNA, 7846 bp, synthetic construct
  misc_feature 1..7846: note = EpiCas059 gRNA plamid DNA
  source 1..7846: mol_type = other DNA
gaagatcctttgatcttttctacggggtctgacgctcagtggaacgaaaactcacgttaagggattttggtcatgagattatcaaaaaggatcttcacctagatccttttaaattaaaaatgaagttttaaatcaatctaaagtatatatgagtaaacttggtctgacagttaccaatgcttaatcagtgaggcacctatctcagcgatctgtctatttcgttcatccatagttgcctgactccccgtcgtgtagataactacgatacgggagggcttaccatctggccccagtgctgcaatgataccgcgagacccacgctcaccggctccagatttatcagcaataaaccagccagccggaagggccgagcgcagaagtggtcctgcaactttatccgcctccatccagtctattaattgttgccgggaagctagagtaagtagttcgccagttaatagtttgcgcaacgttgttgccattgctacaggcatcgtggtgtcacgctcgtcgtttggtatggcttcattcagctccggttcccaacgatcaaggcgagttacatgatcccccatgttgtgcaaaaaagcggttagctccttcggtcctccgatcgttgtcagaagtaagttggccgcagtgttatcactcatggttatggcagcactgcataattctcttactgtcatgccatccgtaagatgcttttctgtgactggtgagtactcaaccaagtcattctgagaatagtgtatgcggcgaccgagttgctcttgcccggcgtcaatacgggataataccgcgccacatagcagaactttaaaagtgctcatcattggaaaacgttcttcggggcgaaaactctcaaggatcttaccgctgttgagatccagttcgatgtaacccactcgtgcacccaactgatcttcagcatcttttactttcaccagcgtttctgggtgagcaaaaacaggaaggcaaaatgccgcaaaaaagggaataagggcgacacggaaatgttgaatactcatactcttcctttttcaatattattgaagcatttatcagggttattgtctcatgagcggatacatatttgaatgtatttagaaaaataaacaaataggggttccgcgcacatttccccgaaaagtgccacctgacgtcgacggatcgggagatctcccgatcccctatggtgcactctcagtacaatctgctctgatgccgcatagttaagccagtatctgctccctgcttgtgtgttggaggtcgctgagtagtgcgcgagcaaaatttaagctacaacaaggcaaggcttgaccgacaattgcatgaagaatctgcttagggttaggcgttttgcgctgcttcgcgatgtacgggccagatatacgcgttgacattgattattgactagttattaatagtaatcaattacggggtcattagttcatagcccatatatggagttccgcgttacataacttacggtaaatggcccgcctggctgaccgcccaacgacccccgcccattgacgtcaataatgacgtatgttcccatagtaacgccaatagggactttccattgacgtcaatgggtggagtatttacggtaaactgcccacttggcagtacatcaagtgtatcatatgccaagtacgccccctattgacgtcaatgacggtaaatggcccgcctggcattatgcccagtacatgaccttatgggactttcctacttggcagtacatctacgtattagtcatcgctattaccatggtgatgcggttttggcagtacatcaatgggcgtggatagcggtttgactcacggggatttccaagtctccaccccattgacgtcaatgggagtttgttttggcaccaaaatcaacgggactttccaaaatgtcgtaacaactccgccccattgacgcaaatgggcggtaggcgtgtacggtgggaggtctatataagcagcgcgttttgcctgtactgggtctctctggttagaccagatctgagcctgggagctctctggctaactagggaacccactgcttaagcctcaataaagcttgccttgagtgcttcaagtagtgtgtgcccgtctgttgtgtgactctggtaactagagatccctcagacccttttagtcagtgtggaaaatctctagcagtggcgcccgaacagggacttgaaagcgaaagggaaaccagaggagctctctcgacgcaggactcggcttgctgaagcgcgcacggcaagaggcgaggggcggcgactggtgagtacgccaaaaattttgactagcggaggctagaaggagagagatgggtgcgagagcgtcagtattaagcgggggagaattagatcgcgatgggaaaaaattcggttaaggccagggggaaagaaaaaatataaattaaaacatatagtatgggcaagcagggagctagaacgattcgcagttaatcctggcctgttagaaacatcagaaggctgtagacaaatactgggacagctacaaccatcccttcagacaggatcagaagaacttagatcattatataatacagtagcaaccctctattgtgtgcatcaaaggatagagataaaagacaccaaggaagctttagacaagatagaggaagagcaaaacaaaagtaagaccaccgcacagcaagcggccgctgatcttcagacctggaggaggagatatgagggacaattggagaagtgaattatataaatataaagtagtaaaaattgaaccattaggagtagcacccaccaaggcaaagagaagagtggtgcagagagaaaaaagagcagtgggaataggagctttgttccttgggttcttgggagcagcaggaagcactatgggcgcagcgtcaatgacgctgacggtacaggccagacaattattgtctggtatagtgcagcagcagaacaatttgctgagggctattgaggcgcaacagcatctgttgcaactcacagtctggggcatcaagcagctccaggcaagaatcctggctgtggaaagatacctaaaggatcaacagctcctggggatttggggttgctctggaaaactcatttgcaccactgctgtgccttggaatgctagttggagtaataaatctctggaacagatttggaatcacacgacctggatggagtgggacagagaaattaacaattacacaagcttaatacactccttaattgaagaatcgcaaaaccagcaagaaaagaatgaacaagaattattggaattagataaatgggcaagtttgtggaattggtttaacataacaaattggctgtggtatataaaattattcataatgatagtaggaggcttggtaggtttaagaatagtttttgctgtactttctatagtgaatagagttaggcagggatattcaccattatcgtttcagacccacctcccaaccccgaggggacccgacaggcccgaaggaatagaagaagaaggtggagagagagacagagacagatccattcgattagtgaacggatcggcactgcgtgcgccaattctgcagacaaatggcagtattcatccacaattttaaaagaaaaggggggattggggggtacagtgcaggggaaagaatagtagacataatagcaacagacatacaaactaaagaattacaaaaacaaattacaaaaattcaaaattttcgggtttattacaggggagggcctatttcccatgattccttcatatttgcatatacgatacaaggctgttagagagataattagaattaatttgactgtaaacacaaagatattagtacaaaatacgtgacgtagaaagtaataatttcttgggtagtttgcagttttaaaattatgttttaaaatggactatcatatgcttaccgtaacttgaaagtatttcgatttcttggctttatatatcttgtggaaaggacgaaacaccgagaaatccgtccttggttgacggaagtcccctcatccccacagtttttttaggcagctgtagatctaggtcttgaaaggagtgggaattggctccggtgcccgtcagtgggcagagcgcacatcgcccacagtccccgagaagttggggggaggggtcggcaattgatccggtgcctagagaaggtggcgcggggtaaactgggaaagtgatgtcgtgtactggctccgcctttttcccgagggtgggggagaaccgtatataagtgcagtagtcgccgtgaacgttctttttcgcaacgggtttgccgccagaacacaggaccggttctagagcgctgccaccatggcgcgtaaggtcgatctcacctcctgcgatcgcgagccgatccacatccccggcagcattcagccgtgcggctgcctgctagcctgcgacgcgcaggcggtgcggatcacgcgcattacggaaaatgccggcgcgttctttggacgcgaaactccgcgggtcggtgagctactcgccgattacttcggcgagaccgaagcccatgcgctgcgcaacgcactggcgcagtcctccgatccaaagcgaccggcgctgatcttcggttggcgcgacggcctgaccggccgcaccttcgacatctcactgcatcgccatgacggtacatcgatcatcgagttcgagcctgcggcggccgaacaggccgacaatccgctgcggctgacgcggcagatcatcgcgcgcaccaaagaactgaagtcgctcgaagagatggccgcacgggtgccgcgctatctgcaggcgatgctcggctatcaccgcgtgatgttgtaccgcttcgcggacgacggctccgggatggtgatcggcgaggcgaagcgcagcgacctggagagctttctcggtcagcactttccggcgtcgctggtcccgcagcaggcgcggctactgtacttgaagaacgcgatccgcgtggtctcggattcgcgcggcatcagcagccggatcgtgcccgagcacgacgcctccggcgccgcgctcgatctgtcgttcgcgcacctgcgcagcatctcgccctgccatctcgaatttctgcggaacatgggcgtcagcgcctcgatgtcgctgtcgatcatcattgacggcacgctatggggattgatcatctgtcatcattacgagccgcgtgccgtgccgatggcgcagcgcgtcgcggccgaaatgttcgccgacttcttatcgctgcacttcaccgccgcccaccaccaacgcggatccggcgagggcagaggtagcctgctgacctgcggcgacgtggaggagaaccccggccccaccgagtacaagcccacggtgcgcctcgccacccgcgacgacgtccccagggccgtacgcaccctcgccgccgcgttcgccgactaccccgccacgcgccacaccgtcgatccggaccgccacatcgagcgggtcaccgagctgcaagaactcttcctcacgcgcgtcgggctcgacatcggcaaggtgtgggtcgcggacgacggcgccgcggtggcggtctggaccacgccggagagcgtcgaagcgggggcggtgttcgccgagatcggcccgcgcatggccgagttgagcggttcccggctggccgcgcagcaacagatggaaggcctcctggcgccgcaccggcccaaggagcccgcgtggttcctggccaccgtcggagtctcgcccgaccaccagggcaagggtctgggcagcgccgtcgtgctccccggagtggaggcggccgagcgcgccggggtgcccgccttcctggagacctccgcgccccgcaacctccccttctacgagcggctcggcttcaccgtcaccgccgacgtcgaggtgcccgaaggaccgcgcacctggtgcatgacccgcaagcccggtgcctgaacgcgttaagtcgaccgatatcaagcttatcgataatcaacctctggattacaaaatttgtgaaagattgactggtattcttaactatgttgctccttttacgctatgtggatacgctgctttaatgcctttgtatcatgctattgcttcccgtatggctttcattttctcctccttgtataaatcctggttgctgtctctttatgaggagttgtggcccgttgtcaggcaacgtggcgtggtgtgcactgtgtttgctgacgcaacccccactggttggggcattgccaccacctgtcagctcctttccgggactttcgctttccccctccctattgccacggcggaactcatcgccgcctgccttgcccgctgctggacaggggctcggctgttgggcactgacaattccgtggtgttgtcggggaaatcatcgtcctttccttggctgctcgcctgtgttgccacctggattctgcgcgggacgtccttctgctacgtcccttcggccctcaatccagcggaccttccttcccgcggcctgctgccggctctgcggcctcttccgcgtcttcgccttcgccctcagacgagtcggatctccctttgggccgcctccccgcgtcgactttaagaccaatgacttacaaggcagctgtagatcttagccactttttaaaagaaaaggggggactggaagggctaattcactcccaacgaagacaagatctgctttttgcttgtactgggtctctctggttagaccagatctgagcctgggagctctctggctaactagggaacccactgcttaagcctcaataaagcttgccttgagtgcttcaagtagtgtgtgcccgtctgttgtgtgactctggtaactagagatccctcagacccttttagtcagtgtggaaaatctctagcagggcccgtttaaacccgctgatcagcctcgactgtgccttctagttgccagccatctgttgtttgcccctcccccgtgccttccttgaccctggaaggtgccactcccactgtcctttcctaataaaatgaggaaattgcatcgcattgtctgagtaggtgtcattctattctggggggtggggtggggcaggacagcaagggggaggattgggaagacaatagcaggcatgctggggatgcggtgggctctatggcttctgaggcggaaagaaccagcggtatcagctcactcaaaggcggtaatacggttatccacagaatcaggggataacgcaggaaagaacatgtgagcaaaaggccagcaaaaggccaggaaccgtaaaaaggccgcgttgctggcgtttttccataggctccgcccccctgacgagcatcacaaaaatcgacgctcaagtcagaggtggcgaaacccgacaggactataaagataccaggcgtttccccctggaagctccctcgtgcgctctcctgttccgaccctgccgcttaccggatacctgtccgcctttctcccttcgggaagcgtggcgctttctcatagctcacgctgtaggtatctcagttcggtgtaggtcgttcgctccaagctgggctgtgtgcacgaaccccccgttcagcccgaccgctgcgccttatccggtaactatcgtcttgagtccaacccggtaagacacgacttatcgccactggcagcagccactggtaacaggattagcagagcgaggtatgtaggcggtgctacagagttcttgaagtggtggcctaactacggctacactagaagaacagtatttggtatctgcgctctgctgaagccagttaccttcggaaaaagagttggtagctcttgatccggcaaacaaaccaccgctggtagcggtggtttttttgtttgcaagcagcagattacgcgcagaaaaaaaggatctcaa

SEQ ID NO: 116 - protein, 1546 aa, synthetic construct
  REGION 1..1546: note = dEpiCas059m46-CBE
  SITE 1546: note = misc_feature - Xaa =
MKRTADGSEFESPKKKRKVSSETGPVAVDPTLRRRIEPHEFEVFFDPRELRKETCLLYEINWGGRHSIWRHTSQNTNKHVEVNFIEKFTTERYFCPNTRCSITWFLSWSPCGECSRAITEFLSRYPHVTLFIYIARLYHHADPRNRQGLRDLISSGVTIQIMTEQESGYCWRNFVNYSPSNEAHWPRYPHLWVRLYVLELYCIILGLPPCLNILRRKQPQLTFFTIALQSCHYQRLPPHILWATGLKSGSETPGTSESATPESGSEETRTPEKIACQQDRSAFFKLGKLPQKTTSAIYHLMRCSKRYIDNVSETISNNIEKAAMTSDNHIFRSALKEEYKKIYREKFYPDVTGQPFPDKGPDNTHIVERTVENLCGQYISALKGVMKVRKPKWQDDIFEDESDKVIAKMLMASGNEADIHPKLEKKIASAKKKDKMDEWQKVLDRYYYIKSKTDIEWTYTTLLYDHIARECARSMFEDGNKPKFCYTNGNKFAKQVVDELWGSERVEYEYEKYLHCRTLEAYWNEENKYFFLENQKKSKKTYEARQIIDHFIENEDAVKAETEEYMAKVAKEFGENGGCKFRTENILYLVNSVSINKKQDEERCPIFKVTDIPQYAEAGIDRIGECKYVIKLKLFTVGERYGTTYMPEAFSGLYDRRTNQRYDLIDRACKGSYVYLPIYISDKDSRKWSDRLKNTFTMSAFSISERKTKKDGRVLCVNLPYKHIQHKPRNYFKVYPTYGVAINVKHSLFSTNATNLNGYIDVNGELIDFYNSIGRPDKLKNINLAVTLGDKCGTAGNHTNFLLVSDLGDWDDHGKKRNDRFVKREDGTYYSRPDLLADGLNFLKKKYSGDRKSYDYINTTIAFRNNQTRLRCIDKEWNDRKRAYDEEHGKPEKGERNGFYPTEDAERLTMERQALRREIAENTRQVIAYMLWLFQENGIKSIALAHLDCGSWKNFRDQLKPKWFCNNCKYWAEKYGIPYEATKYYRSNRKYFDIEDGELIPENVKLNALGEAENDKRYFQTSIAKAVGMSSIKQMFSIVSQNYDIQVNYTEQAYTSQTDSRNGTVDKDFRVSQECYIGSDGTKMNCAFNAAVNIADRISDDTLREEFNKELPMKEFVKYGATQIVSRNRRWNAENAERVTMAAFQKRKNADGGAHTAAVKPTSKTEESSLKLVAEPKKKRKVSGGSTNLSDIIEKETGKQLVIQESILMLPEEVEEVIGNKPESDILVHTAYDESTDENVMLLTSDAPEYKPWALVIQDSNGENKIKMLSGGSPKKKRKVGSKRTGSGATNFSLLKQAGDVEENPGPVNMVSKGEEDNMAIIKEFMRFKVHMEGSVNGHEFEIEGEGEGRPYEGTQTAKLKVTKGGPLPFAWDILSPQFMYGSKAYVKHPADIPDYLKLSFPEGFKWERVMNFEDGGVVTVTQDSSLQDGEFIYKVKLRGTNFPSDGPVMQKKTMGWEASSERMYPEDGALKGEIKQRLKLKDGGHYDAEVKTTYKAKKPVQLPGAYNVNIKLDITSHNEDYTIVEQYERAEGRHSTGGMDELYKX

SEQ ID NO: 117 - DNA, 8090 bp, synthetic construct
  misc_feature 1..8090: note = dEpiCas059m46-CBE plasmid DNA
  source 1..8090: mol_type = other DNA
tgagcaaaaggccagcaaaaggccaggaaccgtaaaaaggccgcgttgctggcgtttttccataggctccgcccccctgacgagcatcacaaaaatcgacgctcaagtcagaggtggcgaaacccgacaggactataaagataccaggcgtttccccctggaagctccctcgtgcgctctcctgttccgaccctgccgcttaccggatacctgtccgcctttctcccttcgggaagcgtggcgctttctcatagctcacgctgtaggtatctcagttcggtgtaggtcgttcgctccaagctgggctgtgtgcacgaaccccccgttcagcccgaccgctgcgccttatccggtaactatcgtcttgagtccaacccggtaagacacgacttatcgccactggcagcagccactggtaacaggattagcagagcgaggtatgtaggcggtgctacagagttcttgaagtggtggcctaactacggctacactagaagaacagtatttggtatctgcgctctgctgaagccagttaccttcggaaaaagagttggtagctcttgatccggcaaacaaaccaccgctggtagcggtttttttgtttgcaagcagcagattacgcgcagaaaaaaaggatctcaagaagatcctttgatcttttctacggggtctgacgctcagtggaacgaaaactcacgttaagggattttggtcatgagattatcaaaaaggatcttcacctagatccttttaaattaaaaatgaagttttaaatcaatctaaagtatatatgagtaaacttggtctgacagttaccaatgcttaatcagtgaggcacctatctcagcgatctgtctatttcgttcatccatagttgcctgactccccgtcgtgtagataactacgatacgggagggcttaccatctggccccagtgctgcaatgataccgcgagacccacgctcaccggctccagatttatcagcaataaaccagccagccggaagggccgagcgcagaagtggtcctgcaactttatccgcctccatccagtctattaattgttgccgggaagctagagtaagtagttcgccagttaatagtttgcgcaacgttgttgccattgctacaggcatcgtggtgtcacgctcgtcgtttggtatggcttcattcagctccggttcccaacgatcaaggcgagttacatgatcccccatgttgtgcaaaaaagcggttagctccttcggtcctccgatcgttgtcagaagtaagttggccgcagtgttatcactcatggttatggcagcactgcataattctcttactgtcatgccatccgtaagatgcttttctgtgactggtgagtactcaaccaagtcattctgagaatagtgtatgcggcgaccgagttgctcttgcccggcgtcaatacgggataataccgcgccacatagcagaactttaaaagtgctcatcattggaaaacgttcttcggggcgaaaactctcaaggatcttaccgctgttgagatccagttcgatgtaacccactcgtgcacccaactgatcttcagcatcttttactttcaccagcgtttctgggtgagcaaaaacaggaaggcaaaatgccgcaaaaaagggaataagggcgacacggaaatgttgaatactcatactcttcctttttcaatattattgaagcatttatcagggttattgtctcatgagcggatacatatttgaatgtatttagaaaaataaacaaataggggttccgcgcacatttccccgaaaagtgccacctgacgtcgacggatcgggagatctcccgatcccctatggtgcactctcagtacaatctgctctgatgccgcatagttaagccagtatctgctccctgcttgtgtgttggaggtcgctgagtagtgcgcgagcaaaatttaagctacaacaaggcaaggcttgaccgacaattgcataatacgactcactatagggcggccgccaaaaaacccctcaagacccgtttagaggccccaaggggttatgctagatctgcttagggttaggcgttttgcgctgcttcgcgatgtacgggccagatatacgcgttgacattgattattgactagttattaatagtaatcaattacggggtcattagttcatagcccatatatggagttccgcgttacataacttacggtaaatggcccgcctggctgaccgcccaacgacccccgcccattgacgtcaataatgacgtatgttcccatagtaacgccaatagggactttccattgacgtcaatgggtggagtatttacggtaaactgcccacttggcagtacatcaagtgtatcatatgccaagtacgccccctattgacgtcaatgacggtaaatggcccgcctggcattatgcccagtacatgaccttatgggactttcctacttggcagtacatctacgtattagtcatcgctattaccatggtgatgcggttttggcagtacatcaatgggcgtggatagcggtttgactcacggggatttccaagtctccaccccattgacgtcaatgggagtttgttttggcaccaaaatcaacgggactttccaaaatgtcgtaacaactccgccccattgacgcaaatgggcggtaggcgtgtacggtgggaggtctatataagcagagctctctggctaactagagaacccactgcttactggcttatcgaaattaatacgactcactatagggagacccaagctggctagcgtttaaacttaggagagccaccatgaaacggactgctgacggcagcgaatttgagagccccaagaagaagaggaaagtcagctcagagactggcccagtggctgtggaccccacattgagacggcggatcgagccccatgagtttgaggtattcttcgatccgagagagctccgcaaggaaacctgcctgctttacgaaattaattgggggggccggcactccatttggcgacatacatcacagaacactaacaagcacgtcgaagtcaacttcatcgagaagttcacgacagaaagatatttctgtccgaacacaaggtgcagcattacctggtttctcagctggagcccatgcggcgaatgtagtagggccatcactgagttcctgtcaaggtatccccacgtcactctgtttatttacatcgcaaggctgtaccaccacgctgacccccgcaatcgacaaggcctgcgggatttgatctcttcaggtgtgactatccaaattatgactgagcaggagtcaggatactgctggagaaactttgtgaattatagcccgagtaatgaagcccactggcctaggtatccccatctgtgggtacgactgtacgttcttgaactgtactgcatcatactgggcctgcctccttgtctcaacattctgagaaggaagcagccacagctgacattctttaccatcgctcttcagtcttgtcattaccagcgactgcccccacacattctctgggccaccgggttgaaatccggcagcgagacgccaggcacctccgagagcgctacgcctgaatccggatccgaagagacacggacccctgagaagatcgcctgccagcaggatagaagcgccttcttcaagctgggcaagctgccccagaaaaccaccagcgccatctaccacctgatgcggtgtagcaagcggtacatcgacaacgtgtccgagacaatcagcaacaacatcgagaaggccgccatgaccagcgacaaccacatcttcagaagcgccctgaaagaagagtacaagaagatctaccgcgagaagttctaccccgacgtgaccggccagccttttccagataagggccccgacaacacccacatcgtggaacggaccgtggaaaacctgtgcggccagtacatctctgccctgaagggcgtgatgaaagtgcggaagcccaagtggcaggacgacatcttcgaggacgagagcgacaaagtgatcgccaagatgctgatggccagcggcaacgaggccgacattcaccccaagctggaaaagaagattgccagcgccaagaaaaaggacaagatggacgagtggcagaaggtgctggacagatactactacatcaagagcaagaccgacatcgagtggacctacaccacactgctgtacgaccacattgcccgcgagtgcgccagatccatgttcgaggatggcaacaagcctaagttctgctacaccaacggcaacaagttcgccaaacaggtggtggacgagctgtggggctctgagagagtggaatacgagtacgagaagtacctgcactgcagaaccctggaagcctactggaacgaggaaaacaagtacttcttcctggaaaatcaaaagaagtccaagaaaacctacgaggcccggcagatcatcgaccacttcatcgagaacgaggacgccgtgaaggccgaaaccgaagagtatatggccaaggtggccaaagagttcggcgagaacggcggctgcaagttcagaaccgagaacatcctgtacctggtcaacagcgtgtccatcaacaagaagcaggacgaggaacggtgccccatcttcaaagtgaccgacattccccagtatgccgaggccggcatcgatagaatcggcgagtgcaaatacgtgatcaagctgaagctgttcaccgtgggcgagagatacggcaccacctatatgcctgaggccttcagcggcctgtacgacagaaggaccaaccagagatacgacctgatcgacagagcctgcaagggcagctacgtgtacctgcctatctacatcagcgacaaggacagccggaagtggagcgacagactgaagaacaccttcaccatgtccgccttcagcatcagcgagcgcaagaccaagaaagacggcagagtgctgtgcgtgaacctgccttacaaacacatccagcacaagccccggaactacttcaaggtgtaccccacctacggcgtggctatcaacgtgaagcacagcctgttcagcaccaacgccaccaacctgaacggctacatcgacgtgaacggcgagctgatcgacttctacaacagcatcggcagacccgataagctcaagaacatcaacctggccgtgacactgggcgacaaatgcggcacagctggcaaccacaccaactttctgctggtgtccgacctcggcgactgggatgatcacggcaagaagcggaacgacagattcgtgaagagagaggacggcacctactacagcagacctgacctgctggccgacggcctgaacttcctgaagaagaagtatagcggcgaccggaagtcctacgattatatcaacaccacaatcgccttccggaacaaccagaccagactgagatgcatcgacaaagagtggaacgatcggaagcgggcctacgatgaggaacacggcaagcctgagaagggcgaaagaaacggcttctaccctaccgaggatgccgagcggctgacaatggaaagacaggccctgcggagagagattgccgagaacaccagacaagtgattgcctacatgctgtggctgttccaagagaacggcatcaagtctatcgccctggctcacctggattgcggcagctggaagaacttccgggaccagctgaagccaaagtggttctgcaacaactgcaagtactgggccgagaagtatggcatcccttacgaggccaccaagtactacagaagcaaccggaagtactttgacatcgaggacggggagctgattcccgagaatgtgaagctgaacgccctgggcgaagccgagaacgacaagagatacttccagacctctatcgccaaggccgtgggcatgagcagcatcaagcagatgttcagcatcgtgtcccagaactacgacatccaagtgaactacaccgagcaggcctacaccagccagaccgacagcagaaatggcaccgtggacaaggacttcagagtgtcccaagagtgctacatcggcagcgacggcaccaagatgaactgcgcttttaacgccgccgtgaatatcgccgaccggatctccgatgacaccctgcgggaagagttcaacaaagaactgcccatgaaggaatttgtgaagtacggcgccacacagatcgtgtctcggaacagaagatggaacgccgaaaacgccgagagggtcacaatggccgccttccagaagagaaagaacgctgacggcggagcccataccgccgctgtgaagcctacatccaagaccgaggaaagcagcctgaagctggtggccgaacccaagaagaaacggaaagtgtccggcggcagcaccaacctgtccgacatcatcgagaaggagacgggcaagcaactcgtgatccaggagagcatcctcatgctgccagaggaggtggaggaggtcatcggcaacaagccagagtccgacatcctggtgcacaccgcctacgacgagtccaccgacgagaacgtcatgctcctgaccagcgacgccccagagtacaagccctgggccctcgtcatccaggacagcaacggggagaacaagatcaagatgctgtctggtggttctcccaagaagaagaggaaagtcggatccaaaagaactggaagcggagctactaacttcagcctgctgaagcaggctggagacgtggaggagaaccctggacctgttaacatggtgagcaagggcgaggaggataacatggccatcatcaaggagttcatgcgcttcaaggtgcacatggagggctccgtgaacggccacgagttcgagatcgagggcgagggcgagggccgcccctacgagggcacccagaccgccaagctgaaggtgaccaagggtggccccctgcccttcgcctgggacatcctgtcccctcagttcatgtacggctccaaggcctacgtgaagcaccccgccgacatccccgactacttgaagctgtccttccccgagggcttcaagtgggagcgcgtgatgaacttcgaggacggcggcgtggtgaccgtgacccaggactcctccctgcaggacggcgagttcatctacaaggtgaagctgcgcggcaccaacttcccctccgacggccccgtaatgcagaagaagaccatgggctgggaggcctcctccgagcggatgtaccccgaggacggcgccctgaagggcgagatcaagcagaggctgaagctgaaggacggcggccactacgacgctgaggtcaagaccacctacaaggccaagaagcccgtgcagctgcccggcgcctacaacgtcaacatcaagttggacatcacctcccacaacgaggactacaccatcgtggaacagtacgaacgcgccgagggccgccactccaccggcggcatggacgagctgtacaagtaagctcgagcctagagggcccgtttaaacccgctgatcagcctcgactgtgccttctagttgccagccatctgttgtttgcccctcccccgtgccttccttgaccctggaaggtgccactcccactgtcctttcctaataaaatgaggaaattgcatcgcattgtctgagtaggtgtcattctattctggggggtggggtggggcaggacagcaagggggaggattgggaagacaatagcaggcatgctggggatgcggtgggctctatggtaccgtcgacctctagctagagcttggcgtaatcatggtcatagctgtttcctgtgtgaaattgttatccgctcacaattccacacaacatacgagccggaagcataaagtgtaaagcctggggtgcctaatgagtgagctaactcacattaattgcgttgcgctcactgcccgctttccagtcgggaaacctgtcgtgccagctgcattaatgaatcggccaacgcgcggggagaggcggtttgcgtattgggcgctcttccgcttcctcgctcactgactcgctgcgctcggtcgttcggctgcggcgagcggtatcagctcactcaaaggcggtaatacggttatccacagaatcaggggataacgcaggaaagaacatg

SEQ ID NO: 118 - protein, 1863 aa, synthetic construct
  REGION 1..1863: note = dAsCas12a-CBE
  SITE 1863: note = misc_feature - Xaa =
MKRTADGSEFESPKKKRKVSSETGPVAVDPTLRRRIEPHEFEVFFDPRELRKETCLLYEINWGGRHSIWRHTSQNTNKHVEVNFIEKFTTERYFCPNTRCSITWFLSWSPCGECSRAITEFLSRYPHVTLFIYIARLYHHADPRNRQGLRDLISSGVTIQIMTEQESGYCWRNFVNYSPSNEAHWPRYPHLWVRLYVLELYCIILGLPPCLNILRRKQPQLTFFTIALQSCHYQRLPPHILWATGLKSGSETPGTSESATPESGSSKLEKFTNCYSLSKTLRFKAIPVGKTQENIDNKRLLVEDEKRAEDYKGVKKLLDRYYLSFINDVLHSIKLKNLNNYISLFRKKTRTEKENKELENLEINLRKEIAKAFKGNEGYKSLFKKDIIETILPEFLDDKDEIALVNSFNGFTTAFTGFFDNRENMFSEEAKSTSIAFRCINENLTRYISNMDIFEKVDAIFDKHEVQEIKEKILNSDYDVEDFFEGEFFNFVLTQEGIDVYNAIIGGFVTESGEKIKGLNEYINLYNQKTKQKLPKFKPLYKQVLSDRESLSFYGEGYTSDEEVLEVFRNTLNKNSEIFSSIKKLEKLFKNFDEYSSAGIFVKNGPAISTISKDIFGEWNVIRDKWNAEYDDIHLKKKAVVTEKYEDDRRKSFKKIGSFSLEQLQEYADADLSVVEKLKEIIIQKVDEIYKVYGSSEKLFDADFVLEKSLKKNDAVVAIMKDLLDSVKSFENYIKAFFGEGKETNRDESFYGDFVLAYDILLKVDHIYDAIRNYVTQKPYSKDKFKLYFQNPQFMGGWDKDKETDYRATILRYGSKYYLAIMDKKYAKCLQKIDKDDVNGNYEKINYKLLPGPNKMLPKVFFSKKWMAYYNPSEDIQKIYKNGTFKKGDMFNLNDCHKLIDFFKDSISRYPKWSNAYDFNFSETEKYKDIAGFYREVEEQGYKVSFESASKKEVDKLVEEGKLYMFQIYNKDFSDKSHGTPNLHTMYFKLLFDENNHGQIRLSGGAELFMRRASLKKEELVVHPANSPIANKNPDNPKKTTTLSYDVYKDKRFSEDQYELHIPIAINKCPKNIFKINTEVRVLLKHDDNPYVIGIARGERNLLYIVVVDGKGNIVEQYSLNEIINNFNGIRIKTDYHSLLDKKEKERFEARQNWTSIENIKELKAGYISQVVHKICELVEKYDAVIALADLNSGFKNSRVKVEKQVYQKFEKMLIDKLNYMVDKKSNPCATGGALKGYQITNKFESFKSMSTQNGFIFYIPAWLTSKIDPSTGFVNLLKTKYTSIADSKKFISSFDRIMYVPEEDLFEFALDYKNFSRTDADYIKKWKLYSYGNRIRIFRNPKKNNVFDWEEVCLTSAYKELFNKYGINYQQGDIRALLCEQSDKAFYSSFMALMSLMLQMRNSITGRTDVAFLISPVKNSDGIFYDSRNYEAQENAILPKNADANGAYNIARKVLWAIGQFKKAEDEKLDKVKIAISNKEWLEYAQTSVKHPKKKRKVSGGSTNLSDIIEKETGKQLVIQESILMLPEEVEEVIGNKPESDILVHTAYDESTDENVMLLTSDAPEYKPWALVIQDSNGENKIKMLSGGSPKKKRKVGSKRTGSGATNFSLLKQAGDVEENPGPVNMVSKGEEDNMAIIKEFMRFKVHMEGSVNGHEFEIEGEGEGRPYEGTQTAKLKVTKGGPLPFAWDILSPQFMYGSKAYVKHPADIPDYLKLSFPEGFKWERVMNFEDGGVVTVTQDSSLQDGEFIYKVKLRGTNFPSDGPVMQKKTMGWEASSERMYPEDGALKGEIKQRLKLKDGGHYDAEVKTTYKAKKPVQLPGAYNVNIKLDITSHNEDYTIVEQYERAEGRHSTGGMDELYKX

SEQ ID NO: 119 - DNA, 9041 bp, synthetic construct
  misc_feature 1..9041: note = dAsCas12a-CBE plasmid DNA
  source 1..9041: mol_type = other DNA
tgagcaaaaggccagcaaaaggccaggaaccgtaaaaaggccgcgttgctggcgtttttccataggctccgcccccctgacgagcatcacaaaaatcgacgctcaagtcagaggtggcgaaacccgacaggactataaagataccaggcgtttccccctggaagctccctcgtgcgctctcctgttccgaccctgccgcttaccggatacctgtccgcctttctcccttcgggaagcgtggcgctttctcatagctcacgctgtaggtatctcagttcggtgtaggtcgttcgctccaagctgggctgtgtgcacgaaccccccgttcagcccgaccgctgcgccttatccggtaactatcgtcttgagtccaacccggtaagacacgacttatcgccactggcagcagccactggtaacaggattagcagagcgaggtatgtaggcggtgctacagagttcttgaagtggtggcctaactacggctacactagaagaacagtatttggtatctgcgctctgctgaagccagttaccttcggaaaaagagttggtagctcttgatccggcaaacaaaccaccgctggtagcggtttttttgtttgcaagcagcagattacgcgcagaaaaaaaggatctcaagaagatcctttgatcttttctacggggtctgacgctcagtggaacgaaaactcacgttaagggattttggtcatgagattatcaaaaaggatcttcacctagatccttttaaattaaaaatgaagttttaaatcaatctaaagtatatatgagtaaacttggtctgacagttaccaatgcttaatcagtgaggcacctatctcagcgatctgtctatttcgttcatccatagttgcctgactccccgtcgtgtagataactacgatacgggagggcttaccatctggccccagtgctgcaatgataccgcgagacccacgctcaccggctccagatttatcagcaataaaccagccagccggaagggccgagcgcagaagtggtcctgcaactttatccgcctccatccagtctattaattgttgccgggaagctagagtaagtagttcgccagttaatagtttgcgcaacgttgttgccattgctacaggcatcgtggtgtcacgctcgtcgtttggtatggcttcattcagctccggttcccaacgatcaaggcgagttacatgatcccccatgttgtgcaaaaaagcggttagctccttcggtcctccgatcgttgtcagaagtaagttggccgcagtgttatcactcatggttatggcagcactgcataattctcttactgtcatgccatccgtaagatgcttttctgtgactggtgagtactcaaccaagtcattctgagaatagtgtatgcggcgaccgagttgctcttgcccggcgtcaatacgggataataccgcgccacatagcagaactttaaaagtgctcatcattggaaaacgttcttcggggcgaaaactctcaaggatcttaccgctgttgagatccagttcgatgtaacccactcgtgcacccaactgatcttcagcatcttttactttcaccagcgtttctgggtgagcaaaaacaggaaggcaaaatgccgcaaaaaagggaataagggcgacacggaaatgttgaatactcatactcttcctttttcaatattattgaagcatttatcagggttattgtctcatgagcggatacatatttgaatgtatttagaaaaataaacaaataggggttccgcgcacatttccccgaaaagtgccacctgacgtcgacggatcgggagatctcccgatcccctatggtgcactctcagtacaatctgctctgatgccgcatagttaagccagtatctgctccctgcttgtgtgttggaggtcgctgagtagtgcgcgagcaaaatttaagctacaacaaggcaaggcttgaccgacaattgcataatacgactcactatagggcggccgccaaaaaacccctcaagacccgtttagaggccccaaggggttatgctagatctgcttagggttaggcgttttgcgctgcttcgcgatgtacgggccagatatacgcgttgacattgattattgactagttattaatagtaatcaattacggggtcattagttcatagcccatatatggagttccgcgttacataacttacggtaaatggcccgcctggctgaccgcccaacgacccccgcccattgacgtcaataatgacgtatgttcccatagtaacgccaatagggactttccattgacgtcaatgggtggagtatttacggtaaactgcccacttggcagtacatcaagtgtatcatatgccaagtacgccccctattgacgtcaatgacggtaaatggcccgcctggcattatgcccagtacatgaccttatgggactttcctacttggcagtacatctacgtattagtcatcgctattaccatggtgatgcggttttggcagtacatcaatgggcgtggatagcggtttgactcacggggatttccaagtctccaccccattgacgtcaatgggagtttgttttggcaccaaaatcaacgggactttccaaaatgtcgtaacaactccgccccattgacgcaaatgggcggtaggcgtgtacggtgggaggtctatataagcagagctctctggctaactagagaacccactgcttactggcttatcgaaattaatacgactcactatagggagacccaagctggctagcgtttaaacttaggagagccaccatgaaacggactgctgacggcagcgaatttgagagccccaagaagaagaggaaagtcagctcagagactggcccagtggctgtggaccccacattgagacggcggatcgagccccatgagtttgaggtattcttcgatccgagagagctccgcaaggaaacctgcctgctttacgaaattaattgggggggccggcactccatttggcgacatacatcacagaacactaacaagcacgtcgaagtcaacttcatcgagaagttcacgacagaaagatatttctgtccgaacacaaggtgcagcattacctggtttctcagctggagcccatgcggcgaatgtagtagggccatcactgagttcctgtcaaggtatccccacgtcactctgtttatttacatcgcaaggctgtaccaccacgctgacccccgcaatcgacaaggcctgcgggatttgatctcttcaggtgtgactatccaaattatgactgagcaggagtcaggatactgctggagaaactttgtgaattatagcccgagtaatgaagcccactggcctaggtatccccatctgtgggtacgactgtacgttcttgaactgtactgcatcatactgggcctgcctccttgtctcaacattctgagaaggaagcagccacagctgacattctttaccatcgctcttcagtcttgtcattaccagcgactgcccccacacattctctgggccaccgggttgaaatccggcagcgagacgccaggcacctccgagagcgctacgcctgaatccggatcctcaaagctggagaaattcaccaactgttatagcctgtctaagaccctgcgcttcaaggcaatcccagtgggcaagacacaagagaacattgacaacaaacggctcctggtggaggatgagaagagggctgaagattacaagggcgttaagaagctgctggataggtactatctgtcattcatcaacgatgtcctccacagtatcaagctgaagaatctgaacaattacatttctctgttccggaagaagacacggaccgagaaggagaacaaagagctggagaatctggagatcaacctgaggaaagaaatagctaaggctttcaaagggaacgagggttacaagtccctgttcaagaaagacattatcgagactattctgcctgagttcctggacgataaagatgagatcgccctcgtcaattccttcaatgggtttaccacagcctttaccggcttcttcgacaatagagagaatatgttctctgaagaggccaaatccactagcatcgcctttcgctgcataaacgagaacctgactaggtacatcagcaatatggacatctttgagaaagtcgatgccatattcgacaaacatgaggtgcaggagattaaggagaagatcctgaactcagattacgatgtcgaagatttcttcgagggagagttcttcaacttcgtgctcacacaagagggcattgatgtgtacaatgcaatcattggagggttcgtgacagagagtggcgagaagataaagggcctgaacgagtatatcaacctctacaaccagaaaaccaagcagaaactgcctaagttcaagccactgtacaaacaagtgctctcagatagggaaagcctgagcttctacggtgaagggtatacatcagatgaagaagtgctcgaagtgttccgcaacaccctcaataagaacagtgaaatcttctcttcaatcaagaagctggagaaactgttcaagaatttcgatgagtactcctctgccggaatctttgtgaagaatggccctgcaatatccactattagcaaagacatctttggcgagtggaacgttatcagggataagtggaatgccgagtacgatgatattcatctcaagaagaaagccgtggttacagagaaatacgaggatgatagacgcaagagctttaagaagattggtagcttctctctcgaacagctgcaggagtacgccgacgctgacctgtcagtcgtggagaaactcaaggagatcataatccagaaggtggatgaaatctacaaagtgtatggaagctctgagaaactcttcgatgcagactttgttctggagaagagtctgaagaagaacgacgcagtggttgctatcatgaaggacctgctggattctgttaagtctttcgagaattacattaaggcattctttggtgaagggaaggagacaaatagggacgagagcttctatggcgactttgttctggcctacgacatcctcctcaaggttgaccacatctatgacgctatacggaattacgttacccagaagccctatagcaaagacaagttcaagctgtatttccagaatccacagtttatgggtgggtgggataaagacaaagaaacagattacagggccactatcctgcggtacggcagcaaatactatctggctatcatggataagaagtacgccaaatgcctccagaagatcgacaaggacgacgtgaacggtaactacgagaagatcaattacaagctcctgccaggacctaacaagatgctgcccaaggtgttcttctccaagaaatggatggcctactataacccaagcgaggacattcagaagatatacaagaatgggacattcaagaagggcgatatgttcaacctcaacgactgccacaagctgattgatttcttcaaggatagcatttctcgctatcccaagtggtctaatgcatacgatttcaacttcagcgagactgagaagtacaaagacatcgctggcttctaccgggaggtggaagagcaaggctataaggtgtcattcgaatccgcttctaagaaggaagtggataagctcgtggaagagggtaagctgtacatgttccagatatacaacaaagacttcagcgataagagccacggcactccaaacctccatactatgtatttcaagctgctgtttgacgagaacaaccacggacagattaggctgtcaggaggcgcagaactcttcatgcgcagagcttcactgaagaaggaggaactcgttgtccacccagccaatagccctatagccaataagaatccagacaatcctaagaaaaccactactctgtcttacgatgtgtataaggataagagattctctgaagatcagtacgaactgcacatacccattgccattaacaagtgccctaagaacatcttcaagattaacacagaggttagagtgctcctgaaacacgacgataacccttatgttataggcattgctcgcggagagagaaacctgctgtacatcgtcgtggtggacggcaaaggcaacatcgtggaacagtacagtctcaatgaaatcattaacaatttcaacggaatccgcattaagaccgactaccattctctcctcgacaagaaggagaaagaaaggttcgaagcaagacagaattggacaagtatagagaatatcaaagaactgaaggctgggtacatctctcaggttgtgcacaagatatgtgagctggtggagaagtacgacgctgttatcgccctcgcggacctgaatagcggcttcaagaactccagggtgaaggtggagaagcaggtgtatcagaagttcgagaagatgctgatcgacaagctcaactatatggtggacaagaaatccaatccttgcgctactggtggagccctgaagggctatcaaatcaccaataagttcgaatctttcaagtctatgagcacccagaatggcttcatcttctacatacccgcatggctgacatccaagattgatccctctaccggatttgttaatctgctcaagactaagtacacctctattgctgactcaaagaagttcatatcatcatttgaccgcatcatgtacgtgccagaagaggacctgttcgagtttgccctggattacaagaatttctctcggactgacgccgactacatcaagaagtggaagctctactcttatggtaatcggattcgcatattccgcaatcccaagaagaataacgtgttcgattgggaggaagtttgcctcaccagcgcttacaaggagctgttcaataagtatgggattaactaccagcagggcgacataagagccctgctgtgcgaacaatctgataaggcattctattcctctttcatggcactgatgtcactgatgctgcaaatgcgcaattccatcaccggaagaacagacgtggcctttctgatctctcctgtcaagaactcagatggcatcttctacgattcccgcaactatgaagcacaggagaatgctatcctgcctaagaatgccgatgcaaatggagcctataacatcgccagaaaggtcctctgggccataggacaattcaagaaagctgaagatgagaagctggacaaggtgaagatcgccatttcaaacaaagagtggctcgaatatgctcagacctcagtgaagcatcccaagaagaaacggaaagtgtccggcggcagcaccaacctgtccgacatcatcgagaaggagacgggcaagcaactcgtgatccaggagagcatcctcatgctgccagaggaggtggaggaggtcatcggcaacaagccagagtccgacatcctggtgcacaccgcctacgacgagtccaccgacgagaacgtcatgctcctgaccagcgacgccccagagtacaagccctgggccctcgtcatccaggacagcaacggggagaacaagatcaagatgctgtctggtggttctcccaagaagaagaggaaagtcggatccaaaagaactggaagcggagctactaacttcagcctgctgaagcaggctggtgacgtggaggagaaccctggacctgttaacatggtgagcaagggcgaggaggataacatggccatcatcaaggagttcatgcgcttcaaggtgcacatggagggctccgtgaacggccacgagttcgagatcgagggcgagggcgagggccgcccctacgagggcacccagaccgccaagctgaaggtgaccaagggtggccccctgcccttcgcctgggacatcctgtcccctcagttcatgtacggctccaaggcctacgtgaagcaccccgccgacatccccgactacttgaagctgtccttccccgagggcttcaagtgggagcgcgtgatgaacttcgaggacggcggcgtggtgaccgtgacccaggactcctccctgcaggacggcgagttcatctacaaggtgaagctgcgcggcaccaacttcccctccgacggccccgtaatgcagaagaagaccatgggctgggaggcctcctccgagcggatgtaccccgaggacggcgccctgaagggcgagatcaagcagaggctgaagctgaaggacggcggccactacgacgctgaggtcaagaccacctacaaggccaagaagcccgtgcagctgcccggcgcctacaacgtcaacatcaagttggacatcacctcccacaacgaggactacaccatcgtggaacagtacgaacgcgccgagggccgccactccaccggcggcatggacgagctgtacaagtaagctcgagcctagagggcccgtttaaacccgctgatcagcctcgactgtgccttctagttgccagccatctgttgtttgcccctcccccgtgccttccttgaccctggaaggtgccactcccactgtcctttcctaataaaatgaggaaattgcatcgcattgtctgagtaggtgtcattctattctggggggtggggtggggcaggacagcaagggggaggattgggaagacaatagcaggcatgctggggatgcggtgggctctatggtaccgtcgacctctagctagagcttggcgtaatcatggtcatagctgtttcctgtgtgaaattgttatccgctcacaattccacacaacatacgagccggaagcataaagtgtaaagcctggggtgcctaatgagtgagctaactcacattaattgcgttgcgctcactgcccgctttccagtcgggaaacctgtcgtgccagctgcattaatgaatcggccaacgcgcggggagaggcggtttgcgtattgggcgctcttccgcttcctcgctcactgactcgctgcgctcggtcgttcggctgcggcgagcggtatcagctcactcaaaggcggtaatacggttatccacagaatcaggggataacgcaggaaagaacatg

SEQ ID NO: 120 - DNA, 23 bp, synthetic construct
  misc_feature 1..23: note = Example7 CXCR4 Spacer-1
  source 1..23: mol_type = other DNA
gcaaggatggacgcgccacagag

SEQ ID NO: 121 - DNA, 23 bp, synthetic construct
  misc_feature 1..23: note = Example7 CXCR4 Spacer-2
  source 1..23: mol_type = other DNA
taaaagtccggccgcggccagaa

SEQ ID NO: 122 - DNA, 23 bp, synthetic construct
  misc_feature 1..23: note = Example7 CXCR4 Spacer-3
  source 1..23: mol_type = other DNA
agggaagcgggatgcgcctgaag

SEQ ID NO: 123 - DNA, 23 bp, synthetic construct
  misc_feature 1..23: note = Example7 CXCR4 Spacer-4
  source 1..23: mol_type = other DNA
cgggtggtcggtagtgagtccgg

SEQ ID NO: 124 - protein, 620 aa, synthetic construct
  REGION 1..620: note = Example7 scFV-P65-HSF1
  SITE 620: note = misc_feature - Xaa =
MGPDIVMTQSPSSLSASVGDRVTITCRSSTGAVTTSNYASWVQEKPGKLFKGLIGGTNNRAPGVPSRFSGSLIGDKATLTISSLQPEDFATYFCALWYSNHWVFGQGTKVELKRGGGGSGGGGSGGGGSSGGGSEVKLLESGGGLVQPGGSLKLSCAVSGFSLTDYGVNWVRQAPGRGLEWIGVIWGDGITDYNSALKDRFIISKDNGKNTVYLQMSKVRSDDTALYYCVTGLFDYWGQGTLVTVSSYPYDVPDYAGGGGGSGGGGSGGGGSGGGGSPKKKRKVAAAPSGQISNQALALAPSSAPVLAQTMVPSSAMVPLAQPPAPAPVLTPGPPQSLSAPVPKSTQAGEGTLSEALLHLQFDADEDLGALLGNSTDPGVFTDLASVDNSEFQQLLNQGVSMSHSTAEPMLMEYPEAITRLVTGSQRPPDPAPTPLGTSGLPNGLSGDEDFSSIADMDFSALLSQISSSGQGGGGSGFSVDTSALLDLFSPSVTVPDMSLPDLDSSLASIQELLSPQEPPRPPEAENSSPDSGKQLVHYTAQPLFLLDPGSVDTGSNDLPVLFELGEGSYFSEGDGFAEDPTISLLTGSEPPKAKDPTVSASEGRGSLLTCDYKDDDDKX

SEQ ID NO: 125 - protein, 1356 aa, synthetic construct
  REGION 1..1356: note = Example7 dEpiCas057-10xGCN4
  SITE 1356: note = misc_feature - Xaa =
MKRTADGSEFESPKKKRKVHRRRRVREGITMSDTTFRPYKSKLNPNERKMPMVVDTMNWCDNACSVFFDLFVGLYGGVKIGDVTNFLTEKQDTTTDADLLCAINWFRAMPVSNPDAVVGPEQLVVRFRDYSGHNPSPMASMYLSAPVNPRYTWVDCRFLYQQMCQTLGANLDVDISTLVQTGLLPIQKDTQLNAYSFCSNVFGEGVKEDPSAKVTSYTAAANALSGATNPIITYEDYRQILSSAITNRPSRKGAKDILAADLDSTKTGVLPGNYVSQRIAMYQASAASKARGVVLPNRLRVKAYLQNLVGLNYICTTWAAPMLRAVGDIKSKNSNNYRFVGERLERQQEIDNLLAVSNIRSAQAILQQFRANESNQFYIKKRHIGKGLPSLYDMWDLMDEKEGIDNYIQSLKGDKTERLPIRELLQIIYPHRKSVSAELFLSAAELTDVEDRQNRCMVHPTVRGSLVINFGKSSTIFGAITPPDTLIKFRGEMVPAGQTGMIWFTMHLVDGGKWVKHHIPCHSSRYFEEIYAWKKDLPTLPFPRRSLYGYAIGNKISDTRKIDLRRKKASKQYLRTLENMTHNVEFDPTTQFMVDQELNVTITARVKKIPPVRDVPVGSRIMGLNKNQTIRDCYSIWERVEANTSGSFQHPVVQDVWLRLVADGHVTSTVNGPNGQIDQMSYSGPDVANCGNWMQERSNFITSVDDADQSIMKHFLWNNRVKLYAWNCVYAGTLMKAISKQMTTANRNLFRNEILSFVGGRFGCRLGSLAQVSLDLLRRMKSVISCYFSRNNAFTIEERSAFDKELMELFESLDNKMNNKRKEKVNRTLSSIFQVAKQHNVVRLVVTKNLQTPDANVRSVMNQRSVDWCARKIEEKIVDLGNVIGIYVDLVEALDLSHLDPFIYIAKGDVGKECQFDEVESSSLLPIHTSMFRDWHGLVNKGRTTTPIYHSALRSFASHYGLRFDDLARIKAAELAKMLPDQKVFIPHRGGRFFMSTYPVTSTSRPVSYDGRQRFLNSGAMVAPVNTMLRGFRRARSHHHHHHPAAKRVKLDDYKDHDGDYKDHDIDYKDDDDKGSMEELLSKNYHLENEVARLKKGSGSGEELLSKNYHLENEVARLKKGSGSGEELLSKNYHLENEVARLKKGSGSGEELLSKNYHLENEVARLKKGSGSGEELLSKNYHLENEVARLKKGSGSGEELLSKNYHLENEVARLKKGSGSGEELLSKNYHLENEVARLKKGSGSGEELLSKNYHLENEVARLKKGSGSGEELLSKNYHLENEVARLKKGSGSGEELLSKNYHLENEVARLKKGSGSGTAVNIGGGTGPMDLQRPQGGGGPKKKRKVGSGVRLQRRX

SEQ ID NO: 126 - DNA, 15951 bp, synthetic construct
  misc_feature 1..15951: note = Example7 dEpiCas057-10xGCN4/scFV-P65-HSF1 plasmid DNA
  source 1..15951: mol_type = other DNA
cttccgcttcctcgctcactgactcgctgcgctcggtcgttcggctgcggcgagcggtatcagctcactcaaaggcggtaatacggttatccacagaatcaggggataacgcaggaaagaacatgtgagcaaaaggccagcaaaaggccaggaaccgtaaaaaggccgcgttgctggcgtttttccataggctccgcccccctgacgagcatcacaaaaatcgacgctcaagtcagaggtggcgaaacccgacaggactataaagataccaggcgtttccccctggaagctccctcgtgcgctctcctgttccgaccctgccgcttaccggatacctgtccgcctttctcccttcgggaagcgtggcgctttctcatagctcacgctgtaggtatctcagttcggtgtaggtcgttcgctccaagctgggctgtgtgcacgaaccccccgttcagcccgaccgctgcgccttatccggtaactatcgtcttgagtccaacccggtaagacacgacttatcgccactggcagcagccactggtaacaggattagcagagcgaggtatgtaggcggtgctacagagttcttgaagtggtggcctaactacggctacactagaagaacagtatttggtatctgcgctctgctgaagccagttaccttcggaaaaagagttggtagctcttgatccggcaaacaaaccaccgctggtagcggtggtttttttgtttgcaagcagcagattacgcgcagaaaaaaaggatctcaagaagatcctttgatcttttctacggggtctgacgctcagtggaacgaaaactcacgttaagggattttggtcatgagattatcaaaaaggatcttcacctagatccttttaaattaaaaatgaagttttaaatcaatctaaagtatatatgagtaaacttggtctgacagttaccaatgcttaatcagtgaggcacctatctcagcgatctgtctatttcgttcatccatagttgcctgactccccgtcgtgtagataactacgatacgggagggcttaccatctggccccagtgctgcaatgataccgcgagacccacgctcaccggctccagatttatcagcaataaaccagccagccggaagggccgagcgcagaagtggtcctgcaactttatccgcctccatccagtctattaattgttgccgggaagctagagtaagtagttcgccagttaatagtttgcgcaacgttgttgccattgctacaggcatcgtggtgtcacgctcgtcgtttggtatggcttcattcagctccggttcccaacgatcaaggcgagttacatgatcccccatgttgtgcaaaaaagcggttagctccttcggtcctccgatcgttgtcagaagtaagttggccgcagtgttatcactcatggttatggcagcactgcataattctcttactgtcatgccatccgtaagatgcttttctgtgactggtgagtactcaaccaagtcattctgagaatagtgtatgcggcgaccgagttgctcttgcccggcgtcaatacgggataataccgcgccacatagcagaactttaaaagtgctcatcattggaaaacgttcttcggggcgaaaactctcaaggatcttaccgctgttgagatccagttcgatgtaacccactcgtgcacccaactgatcttcagcatcttttactttcaccagcgtttctgggtgagcaaaaacaggaaggcaaaatgccgcaaaaaagggaataagggcgacacggaaatgttgaatactcatactcttcctttttcaattcagaagaactcgtcaagaaggcgatagaaggcgatgcgctgcgaatcgggagcggcgataccgtaaagcacgaggaagcggtcagcccattcgccgccaagctcttcagcaatatcacgggtagccaacgctatgtcctgatagcggtccgccacacccagccggccacagtcgatgaatccagaaaagcggccattttccaccatgatattcggcaagcaggcatcgccatgggtcacgacgagatcctcgccgtcgggcatgcgcgccttgagcctggcgaacagttcggctggcgcgagcccctgatgctcttcgtccagatcatcctgatcgacaagaccggcttccatccgagtacgtgctcgctcgatgcgatgtttcgcttggtggtcgaatgggcaggtagccggatcaagcgtatgcagccgccgcattgcatcagccatgatggatactttctcggcaggagcaaggtgggatgacaggagatcctgccccggcacttcgcccaatagcagccagtcccttcccgcttcagtgacaacgtcgagcacagctgcgcaaggaacgcccgtcgtggccagccacgatagccgcgctgcctcgtcctgcagttcattcagggcaccggacaggtcggtcttgacaaaaagaaccgggcgcccctgcgctgacagccggaacacggcggcatcagagcagccgattgtctgttgtgcccagtcatagccgaatagcctctccacccaagcggccggagaacctgcgtgcaatccatcttgttcaatcatgcgaaacgatcctcatcctgtctcttgatcagatcttgatcccctgcgccatcagatccttggcggcaagaaagccatccagtttactttgcagggcttcccaaccttaccagagggcgccccagctggcaattccggttcgcttgctgtccataaaaccgcccagtctagctatcgccatgtaagcccactgcaagctacctgctttctctttgcgcttgcgttttcccttgtccagatagcccagtagctgacattcatccggggtcagcaccgtttctgcggactggctttctacgtgttccgcttcctttagcagcccttgcgccctgaattttgttaaaattcgcgttaaatttttgttaaatcagctcattttttaaccaataggccgaaatcggcaaaatcccttataaatcaaaagaatagaccgagatagggttgagtgttgttccagtttggaacaagagtccactattaaagaacgtggactccaacgtcaaagggcgaaaaaccgtctatcagggcgatggcccactacgtgaaccatcaccctaatcaagttttttggggtcgaggtgccgtaaagcactaaatcggaaccctaaagggagcccccgatttagagcttgacggggaaagccggcgaacgtggcgagaaaggaagggaagaaagcgaaaggagcgggcgctagggcgctggcaagtgtagcggtcacgctgcgcgtaaccaccacacccgccgcgcttaatgcgccgctacagggcgcgtccattcgccattcaggctgcgcaactgttgggaagggcgatcggtgcgggcctcttcgctattacgccagctggcgaaagggggatgtgctgcaaggcgattaagttgggtaacgccagggttttcccagtcacgacgttgtaaaacgacggccagtgaattgtaatacgactcactatagggcgaattgggccctctagatgcatgctcgagcggccgccagtgtgatggatatctgcagaattcgcccttttggccggccttaaccctagaaagataatcatattgtgacgtacgttaaagataatcatgcgtaaaattgacgcatgtgttttatcggtctgtatatcgaggtttatttattaatttgaatagatattaagttttattatatttacacttacatactaataataaattcaacaaacaatttatttatgtttatttatttattaaaaaaaaacaaaaactcaaaatttcttctataaagtaacaaaacttttaggcgcgccggattcgacattgattattgactagttattaatagtaatcaattacggggtcattagttcatagcccatatatggagttccgcgttacataacttacggtaaatggcccgcctggctgaccgcccaacgacccccgcccattgacgtcaataatgacgtatgttcccatagtaacgccaatagggactttccattgacgtcaatgggtggagtatttacggtaaactgcccacttggcagtacatcaagtgtatcatatgccaagtacgccccctattgacgtcaatgacggtaaatggcccgcctggcattatgcccagtacatgaccttatgggactttcctacttggcagtacatctacgtattagtcatcgctattaccatggtcgaggtgagccccacgttctgcttcactctccccatctcccccccctccccacccccaattttgtatttatttattttttaattattttgtgcagcgatgggggcggggggggggggggggcgcgcgccaggcggggcggggcggggcgaggggcggggcggggcgaggcggagaggtgcggcggcagccaatcagagcggcgcgctccgaaagtttccttttatggcgaggcggcggcggcggcggccctataaaaagcgaagcgcgcggcgggcgggagtcgctgcgttgccttcgccccgtgccccgctccgcgccgcctcgcgccgcccgccccggctctgactgaccgcgttactcccacaggtgagcgggcgggacggcccttctcctccgggctgtaattagcgcttggtttaatgacggctcgtttcttttctgtggctgcgtgaaagccttaaagggctccgggagggccctttgtgcgggggggagcggctcggggggtgcgtgcgtgtgtgtgtgcgtggggagcgccgcgtgcggcccgcgctgcccggcggctgtgagcgctgcgggcgcggcgcggggctttgtgcgctccgcgtgtgcgcgaggggagcgcggccgggggcggtgccccgcggtgcgggggggctgcgaggggaacaaaggctgcgtgcggggtgtgtgcgtgggggggtgagcagggggtgtgggcgcggcggtcgggctgtaacccccccctgcacccccctccccgagttgctgagcacggcccggcttcgggtgcggggctccgtgcggggcgtggcgcggggctcgccgtgccgggcggggggtggcggcaggtgggggtgccgggcggggcggggccgcctcgggccggggagggctcgggggaggggcgcggcggccccggagcgccggcggctgtcgaggcgcggcgagccgcagccattgccttttatggtaatcgtgcgagagggcgcagggacttcctttgtcccaaatctggcggagccgaaatctgggaggcgccgccgcaccccctctagcgggcgcgggcgaagcggtgcggcgccggcaggaaggaaatgggcggggagggccttcgtgcgtcgccgcgccgccgtccccttctccatctccagcctcggggctgccgcagggggacggctgccttcgggggggacggggcagggcggggttcggcttctggcgtgtgaccggcggctctagagcctctgctaaccatgttcatgccttcttctttttcctacagatccttaatatgggccccgacatcgtgatgacccagagccccagcagcctgagcgccagcgtgggcgaccgcgtgaccatcacctgccgcagcagcaccggcgccgtgaccaccagcaactacgccagctgggtgcaggagaagcccggcaagctgttcaagggcctgatcggcggcaccaacaaccgcgcccccggcgtgcccagccgcttcagcggcagcctgatcggcgacaaggccaccctgaccatcagcagcctgcagcccgaggacttcgccacctacttctgcgccctgtggtacagcaaccactgggtgttcggccagggcaccaaggtggagctgaagcgcggcggcggcggcagcggcggcggcggcagcggcggcggcggcagcagcggcggcggcagcgaggtgaagctgctggagagcggcggcggcctggtgcagcccggcggcagcctgaagctgagctgcgccgtgagcggcttcagcctgaccgactacggcgtgaactgggtgcgccaggcccccggccgcggcctggagtggatcggcgtgatctggggcgacggcatcaccgactacaacagcgccctgaaggaccgcttcatcatcagcaaggacaacggcaagaacaccgtgtacctgcagatgagcaaggtgcgcagcgacgacaccgccctgtactactgcgtgaccggcctgttcgactactggggccagggcaccctggtgaccgtgagcagctacccatacgatgttccagattacgctggtggaggcggaggttctgggggaggaggtagtggcggtggtggttcaggaggcggcggaagccctaagaaaaagaggaaggtggcggccgctccttcagggcagatcagcaaccaggccctggctctggcccctagctccgctccagtgctggcccagactatggtgccctctagtgctatggtgcctctggcccagccacctgctccagcccctgtgctgaccccaggaccaccccagtcactgagcgctccagtgcccaagtctacacaggccggcgaggggactctgagtgaagctctgctgcacctgcagttcgacgctgatgaggacctgggagctctgctggggaacagcaccgatcccggagtgttcacagatctggcctccgtggacaactctgagtttcagcagctgctgaatcagggcgtgtccatgtctcatagtacagccgaaccaatgctgatggagtaccccgaagccattacccggctggtgaccggcagccagcggccccccgaccccgctccaactcccctgggaaccagcggcctgcctaatgggctgtccggagatgaagacttctcaagcatcgctgatatggactttagtgccctgctgtcacagatttcctctagtgggcagggaggaggtggaagcggcttcagcgtggacaccagtgccctgctggacctgttcagcccctcggtgaccgtgcccgacatgagcctgcctgaccttgacagcagcctggccagtatccaagagctcctgtctccccaggagccccccaggcctcccgaggcagagaacagcagcccggattcagggaagcagctggtgcactacacagcgcagccgctgttcctgctggaccccggctccgtggacaccgggagcaacgacctgccggtgctgtttgagctgggagagggctcctacttctccgaaggggacggcttcgccgaggaccccaccatctccctgctgacaggctcggagcctcccaaagccaaggaccccactgtctccgctagcgagggcagaggaagtctgctaacatgcgattacaaagacgatgacgataagtaaaatcaacctctggattacaaaatttgtgaaagattgactggtattcttaactatgttgctccttttacgctatgtggatacgctgctttaatgcctttgtatcatgctattgcttcccgtatggctttcattttctcctccttgtataaatcctggttgctgtctctttatgaggagttgtggcccgttgtcaggcaacgtggcgtggtgtgcactgtgtttgctgacgcaacccccactggttggggcattgccaccacctgtcagctcctttccgggactttcgctttccccctccctattgccacggcggaactcatcgccgcctgccttgcccgctgctggacaggggctcggctgttgggcactgacaattccgtggtgttgtcggggaaatcatcgtcctttccttggctgctcgcctgtgttgccacctggattctgcgcgggacgtccttctgctacgtcccttcggccctcaatccagcggaccttccttcccgcggcctgctgccggctctgcggcctcttccgcgtcttcgccttcgccctcagacgagtcggatctccctttgggccgcctccccgcatcgataccgtcgatcctgtgccttctagttgccagccatctgttgtttgcccctcccccgtgccttccttgaccctggaaggtgccactcccactgtcctttcctaataaaatgaggaaattgcatcgcattgtctgagtaggtgtcattctattctggggggtggggtggggcaggacagcaagggggaggattgggaagacaatagcaggcatgctggggatgcggtgggctctatgggaattccgttgacattgattattgactagttattaatagtaatcaattacggggtcattagttcatagcccatatatggagttccgcgttacataacttacggtaaatggcccgcctggctgaccgcccaacgacccccgcccattgacgtcaataatgacgtatgttcccatagtaacgccaatagggactttccattgacgtcaatgggtggagtatttacggtaaactgcccacttggcagtacatcaagtgtatcatatgccaagtacgccccctattgacgtcaatgacggtaaatggcccgcctggcattatgcccagtacatgaccttatgggactttcctacttggcagtacatctacgtattagtcatcgctattaccatggtgatgcggttttggcagtacatcaatgggcgtggatagcggtttgactcacggggatttccaagtctccaccccattgacgtcaatgggagtttgttttggcaccaaaatcaacgggactttccaaaatgtcgtaacaactccgccccattgacgcaaatgggcggtaggcgtgtacggtgggaggtctatataagcagagctctctggctaactagagaacccactgcttactggcttatcgaaattaatacgactcactatagggagacccaagctggctagcgtttaaacttaggagagccaccatgaaacggactgctgacggcagcgaatttgagagccccaagaagaagaggaaagtccaccggagacgacgcgttcgcgagggcatcaccatgagcgacaccaccttcagaccctacaagagcaagctgaaccccaacgagcggaagatgcctatggtggtggacaccatgaattggtgcgacaacgcctgcagcgtgttcttcgatctgttcgtgggcctgtacggcggcgtgaagatcggcgacgtgaccaatttcctgaccgagaagcaggacaccaccaccgatgccgatctgctgtgcgccatcaactggttcagagccatgcctgtgtctaaccccgatgccgttgtgggacctgagcagctggttgtgcggttcagagactacagcggccacaatccatctccaatggccagcatgtacctgagcgcccctgtgaaccctagatacacctgggtcgactgccggttcctgtaccagcagatgtgtcagaccctgggcgccaacctggatgtggacatctctaccctggtgcagaccggcctgctgcctatccagaaggatacacagctgaacgcctacagcttctgcagcaacgtgttcggcgagggcgtgaaagaagatcccagcgccaaagtgaccagctacacagccgctgccaatgctctgagcggcgccaccaatcctatcatcacctacgaggactaccggcagatcctgtccagcgccatcaccaacagacccagcagaaagggcgccaaggatattctggccgccgatctggatagcaccaagacaggtgttctgcccggcaactacgtgtcccagagaatcgccatgtaccaggcctctgccgcctctaaagctagaggcgtggtgctgcccaaccggctgagagtgaaagcctacctgcagaacctcgtgggactgaactacatctgcaccacctgggccgctcctatgctgagagccgtgggcgacatcaagagcaagaacagcaacaactaccgcttcgtgggcgagagactggaacggcagcaagagatcgataacctgctggccgtgtccaacatcagaagcgcccaggccatcctgcagcagttcagggccaatgagagcaaccagttctacatcaagaagcggcacatcggcaagggcctgcctagcctgtacgacatgtgggatctgatggacgagaaagagggcatcgacaactacatccagagcctgaagggcgacaagaccgagaggctgccaatcagagagctgctgcagatcatctaccctcacagaaagagcgtgtccgccgagctgtttctgtctgccgccgaactgaccgacgtggaagatagacagaaccggtgcatggtgcaccctacagtgcggggctctctggtcatcaacttcggcaagagcagcaccatcttcggcgctatcacccctcctgacacactgatcaagttccggggcgaaatggtgcctgctggacagacaggcatgatctggttcacaatgcacctggtggacggcggcaaatgggtcaagcaccacattccttgccacagcagccggtacttcgaggaaatctacgcctggaagaaggacctgcctacactgccctttccacggcggagcctgtatggctatgccatcggcaacaagatcagcgacacccggaagatcgacctgcggagaaagaaggccagcaagcagtacctgcggaccctggaaaacatgacccacaacgtggaatttgaccccaccacacagttcatggtggaccaagagctgaacgtgaccatcaccgccagagtgaagaaaatccctcctgtgcgggatgtgcccgtgggcagcagaattatgggcctgaacaagaaccagaccatccgggactgctacagcatctgggagagagtggaagccaacaccagcggcagctttcagcatcccgtggtccaggatgtgtggctgagactggtggccgatggccacgtgacctctacagtgaatggccccaacggccagatcgaccagatgagctactctggccccgatgtggccaactgcggcaactggatgcaagagcggagcaacttcatcaccagcgtggacgacgccgaccagtctatcatgaagcactttctgtggaacaaccgcgtgaagctgtatgcctggaactgcgtgtacgccggcacactgatgaaggccatctctaagcagatgaccaccgccaaccggaacctgttcagaaacgagatcctgagcttcgttggcggcagattcggctgcagactgggatctctggcccaggtttcactggacctgctgcggaggatgaagtccgtgatcagctgctacttcagccggaacaacgccttcaccatcgaggaaagaagcgccttcgacaaagaactgatggaactgttcgagagcctggacaacaagatgaacaacaagcggaaagagaaagtcaaccggacactcagcagcatcttccaggtggccaagcagcacaatgttgtgcggctggtggtcaccaagaacctgcagacccctgatgccaatgtgcggagcgtgatgaatcagagatccgtggattggtgcgctcggaagattgaagagaagatcgtggacctgggcaacgtgatcggaatctatgtggatctggtggaagccctggatctgagccatctggaccccttcatctatatcgccaagggcgacgtgggcaaagagtgccagtttgacgaggtggaaagcagctccctgctgccaattcacaccagcatgtttcgcgactggcacggcctggttaacaagggcagaaccaccacacctatctaccacagcgccctgaggagcttcgccagccactacggcctgagattcgatgacctggccagaatcaaggccgctgagctggccaaaatgctgccagaccagaaggtgttcatcccacacagaggcggacggttcttcatgagcacataccccgtgaccagcaccagcagacccgtgtcttatgatggccggcagcggttcctgaacagcggcgccatggtggccccagtgaacaccatgctgcgcggattcagaagggccagatctcatcatcatcaccatcaccctgctgctaagagagtgaaactggatgactacaaagaccatgacggtgattataaagatcatgatatcgattacaaggatgacgatgacaagggatccatggaagaacttttgagcaagaattatcatcttgagaacgaagtggctcgtcttaagaaaggttctggcagtggagaagaactgctttcaaagaattaccacctggaaaatgaggtagctagactgaaaaaggggagcggaagtggggaggagttgctgagcaaaaattatcatttggagaacgaagtagcacgactaaagaaagggtccggatcgggtgaggagttactctcgaaaaattatcatctcgaaaacgaagtggctcggctaaaaaagggcagtggttctggagaagagctattatctaaaaactaccacctcgaaaatgaggtggcacgcttaaaaaagggaagtggcagtggtgaagagctactatccaagaattatcatcttgagaacgaggtagcgcgtttgaagaagggttccggctcaggagaggaactgctctcgaagaactatcatcttgaaaatgaggtcgctcgattaaaaaagggatcgggcagtggtgaggaactactttcaaagaattaccacctcgaaaacgaagtagctcgattaaagaaaggttcagggtcgggtgaagaattactgagtaaaaattatcatctggaaaatgaggtagcgagactaaaaaaggggagtggttctggcgaggaattgctatcgaaaaattatcatcttgagaacgaagttgctaggctcaaaaagggctcaggctcaggcaccgcggtaaacataggtggtggaaccggtccgatggatctacagcggccgcaaggtggaggtggacccaagaagaagcgcaaggtgggaagcggagtaagattacaaagacgatgacgataagtaaaatcaacctctggattacaaaatttgtgaaagattgactggtattcttaactatgttgctccttttacgctatgtggatacgctgctttaatgcctttgtatcatgctattgcttcccgtatggctttcattttctcctccttgtataaatcctggttgctgtctctttatgaggagttgtggcccgttgtcaggcaacgtggcgtggtgtgcactgtgtttgctgacgcaacccccactggttggggcattgccaccacctgtcagctcctttccgggactttcgctttccccctccctattgccacggcggaactcatcgccgcctgccttgcccgctgctggacaggggctcggctgttgggcactgacaattccgtggtgttgtcggggaaatcatcgtcctttccttggctgctcgcctgtgttgccacctggattctgcgcgggacgtccttctgctacgtcccttcggccctcaatccagcggaccttccttcccgcggcctgctgccggctctgcggcctcttccgcgtcttcgccttcgccctcagacgagtcggatctccctttgggccgcctccccgcatcgataccgtcgatcctgtgccttctagttgccagccatctgttgtttgcccctcccccgtgccttccttgaccctggaaggtgccactcccactgtcctttcctaataaaatgaggaaattgcatcgcattgtctgagtaggtgtcattctattctggggggtggggtggggcaggacagcaagggggaggattgggaagacaatagcaggcatgctggggatgcggtgggctctatgggaattccgaagttcctattctctagaaagtataggaacttcaggtctgaagaggagtttacgtccagcgcgatgggtaggggaggcgcttttcccaaggcagtctggagcatgcgctttagcagccccgctgggcacttggcgctacacaagtggcctctggcctcgcacacattccacatccaccggtaggcgccaaccggctccgttctttggtggccccttcgcgccaccttctactcctcccctagtcaggaagttcccccccgccccgcagctcgcgtcgtgcaggacgtgacaaatggaagtagcacgtctcactagtctcgtgcagatggacagcaccgctgagcaatggaagcgggtaggcctttggggcagcggccaatagcagctttgctccttcgctttctgggctcagaggctgggaaggggtgggtccgggggcgggctcaggggcgggctcaggggcggggcgggcgcccgaaggtcctccggaggcccggcattctgcacgcttcaaaagcgcacgtctgccgcgctgttctcctcttcctcatctccgggcctttcgacctgcagcctgttgacaattaatcatcggcatagtatatcggcatagtataatacgacaaggtgaggaactaaaccatgaccgagtacaagcccacggtgcgcctcgccacccgcgacgacgtccccagggccgtacgcaccctcgccgccgcgttcgccgactaccccgccacgcgccacaccgtcgatccggaccgccacatcgagcgggtcaccgagctgcaagaactcttcctcacgcgcgtcgggctcgacatcggcaaggtgtgggtcgcggacgacggcgccgcggtggcggtctggaccacgccggagagcgtcgaagcgggggcggtgttcgccgagatcggcccgcgcatggccgagttgagcggttcccggctggccgcgcagcaacagatggaaggcctcctggcgccgcaccggcccaaggagcccgcgtggttcctggccaccgtcggcgtctcgcccgaccaccagggcaagggtctgggcagcgccgtcgtgctccccggagtggaggcggccgagcgcgccggggtgcccgccttcctggaaacctccgcgccccgcaacctccccttctacgagcggctcggcttcaccgtcaccgccgacgtcgaggtgcccgaaggaccgcgcacctggtgcatgacccgcaagcccggtgcctgaaaacccgctgatcagcctcgactgtgccttctagttgccagccatctgttgtttgcccctcccccgtgccttccttgaccctggaaggtgccactcccactgtcctttcctaataaaatgaggaaattgcatcgcattgtctgagtaggtgtcattctattctggggggtggggtggggcaggacagcaagggggaggattgggaagacaatagcaggcatgctggggatgcggtgggctctatggcggcgcgccatcgatattaatgatatctataacaagaaaatatatatataataagttatcacgtaagtagaacatgaaataacaatataattatcgtatgagttaaatcttaaaagtcacgtaaaagataatcatgcgtcattttgactcacgcggtcgttatagttcaaaatcagtgacacttaccgcattgacaagcacgcctcacgggagctccaagcggcgactgagatgtcctaaatgcacagcgacggattcgcgctatttagaaagagagagcaatatttcaagaatgcatgcgtcaattttacgcagactatctttctagggttaaggtaccaagcttggcgtaatcatggtcatagctgtttcctgtgtgaaattgttatccgctcacaattccacacaacatacgagccggaagcataaagtgtaaagcctggggtgcctaatgagtgagctaactcacattaattgcgttgcgctcactgcccgctttccagtcgggaaacctgtcgtgccagctgcattaatgaatcggccaacgcgcggggagaggcggtttgcgtattgggcgct

SEQ ID NO: 127 - protein, 1307 aa, synthetic construct
  REGION 1..1307: note = AsCas12a
MTQFEGFTNLYQVSKTLRFELIPQGKTLKHIQEQGFIEEDKARNDHYKELKPIIDRIYKTYADQCLQLVQLDWENLSAAIDSYRKEKTEETRNALIEEQATYRNAIHDYFIGRTDNLTDAINKRHAEIYKGLFKAELFNGKVLKQLGTVTTTEHENALLRSFDKFTTYFSGFYENRKNVFSAEDISTAIPHRIVQDNFPKFKENCHIFTRLITAVPSLREHFENVKKAIGIFVSTSIEEVFSFPFYNQLLTQTQIDLYNQLLGGISREAGTEKIKGLNEVLNLAIQKNDETAHIIASLPHRFIPLFKQILSDRNTLSFILEEFKSDEEVIQSFCKYKTLLRNENVLETAEALFNELNSIDLTHIFISHKKLETISSALCDHWDTLRNALYERRISELTGKITKSAKEKVQRSLKHEDINLQEIISAAGKELSEAFKQKTSEILSHAHAALDQPLPTTLKKQEEKEILKSQLDSLLGLYHLLDWFAVDESNEVDPEFSARLTGIKLEMEPSLSFYNKARNYATKKPYSVEKFKLNFQMPTLASGWDVNKEKNNGAILFVKNGLYYLGIMPKQKGRYKALSFEPTEKTSEGFDKMYYDYFPDAAKMIPKCSTQLKAVTAHFQTHTTPILLSNNFIEPLEITKEIYDLNNPEKEPKKFQTAYAKKTGDQKGYREALCKWIDFTRDFLSKYTKTTSIDLSSLRPSSQYKDLGEYYAELNPLLYHISFQRIAEKEIMDAVETGKLYLFQIYNKDFAKGHHGKPNLHTLYWTGLFSPENLAKTSIKLNGQAELFYRPKSRMKRMAHRLGEKMLNKKLKDQKTPIPDTLYQELYDYVNHRLSHDLSDEARALLPNVITKEVSHEIIKDRRFTSDKFFFHVPITLNYQAANSPSKFNQRVNAYLKEHPETPIIGIDRGERNLIYITVIDSTGKILEQRSLNTIQQFDYQKKLDNREKERVAARQAWSVVGTIKDLKQGYLSQVIHEIVDLMIHYQAVVVLENLNFGFKSKRTGIAEKAVYQQFEKMLIDKLNCLVLKDYPAEKVGGVLNPYQLTDQFTSFAKMGTQSGFLFYVPAPYTSKIDPLTGFVDPFVWKTIKNHESRKHFLEGFDFLHYDVKTGDFILHFKMNRNLSFQRGLPGFMPAWDIVFEKNETQFDAKGTPFIAGKRIVPVIENHRFTGRYRDLYPANELIALLEEKGIVFRDGSNILPKLLENDDSHAIDTMVALIRSVLQMRNSNAATGEDYINSPVRDLNGVCFDSRFQNPEWPMDADANGAYHIALKGQLLLNHLKESKDLKLQNGISNQDWLAYIQELRN